European Patent Specification EP 3 878 973 B1, published July 10, 2024. Title: METHODS FOR DETERMINING FRACTION OF FETAL NUCLEIC ACIDS IN MATERNAL SAMPLES. Applicant: VERINATA HEALTH, INC. Application PCT/US2010/058606. The sequence listing filed with the application follows.

SEQUENCE LISTING (427 sequences)

SEQ ID NO: 1 - DNA, 111 bp, Homo sapiens
cacatgcacagccagcaaccctgtcagcaggagttcccaccagtttctttctgagaacatctgttcaggtttctctccatctctatttactcaggtcacaggaccttgggg

SEQ ID NO: 2 - DNA, 111 bp, Homo sapiens
cacatgcacagccagcaaccctgtcagcaggagttcccaccagtttctttctgagaacatctgttcaggtttctctccatctctgtttactcaggtcacaggaccttgggg

SEQ ID NO: 3 - DNA, 126 bp, Homo sapiens
tgaggaagtgaggctcagagggtaagaaactttgtcacagagctggtggtgagggtggagattttacactccctgcctcccacaccagtttctccagagtggaaagactttcatctcgcactggca

SEQ ID NO: 4 - DNA, 126 bp, Homo sapiens
tgaggaagtgaggctcagagggtaagaaactttgtcacagagctggtggtgagggtggagattttacactccctgcctcccacaccagtttctccggagtggaaagactttcatctcgcactggca

SEQ ID NO: 5 - DNA, 121 bp, Homo sapiens
gtgccttcagaacctttgagatctgattctatttttaaagcttcttagaagagagattgcaaagtgggttgtttctctagccagacagggcaggcaaataggggtggctggtgggatggga

SEQ ID NO: 6 - DNA, 121 bp, Homo sapiens
gtgccttcagaacctttgagatctgattctatttttaaagcttcttagaagagagattgcaaagtgggttgtttctctagccagacagggcaggtaaataggggtggctggtgggatggga

SEQ ID NO: 7 - DNA, 111 bp, Homo sapiens
aggtgtgtctctcttttgtgaggggaggggtcccttctggcctagtagagggcctggcctgcagtgagcattcaaatcctcaaggaacagggtggggaggtgggacaaagg

SEQ ID NO: 8 - DNA, 111 bp, Homo sapiens
aggtgtgtctctcttttgtgaggggaggggtcccttctggcctagtagagggcctggcctgcagtgagcattcaaatcctcgaggaacagggtggggaggtgggacaaagg

SEQ ID NO: 9 - DNA, 139 bp, Homo sapiens
cctcgcctactgtgctgtttctaaccatcatgcttttccctgaatctcttgagtctttttctgctgtggactgaaacttgatcctgagattcacctctagtccctctgagcagcctcctggaatactcagctgggatgg

SEQ ID NO: 10 - DNA, 139 bp, Homo sapiens
cctcgcctactgtgctgtttctaaccatcatgcttttccctgaatctcttgagtctttttctgctgtggactgaaacttgatcctgagattcacctctagtccctctgggcagcctcctggaatactcagctgggatgg

SEQ ID NO: 11 - DNA, 117 bp, Homo sapiens
aattgcaatggtgagaggttgatggtaaaatcaaacggaacttgttattttgtcattctgatggactggaactgaggattttcaatttcctctccaacccaagacacttctcactgg

SEQ ID NO: 12 - DNA, 117 bp, Homo sapiens
aattgcaatggtgagaggttgatggtaaaatcaaacggaacttgttattttgtcattctgatggactggaactgaggattttcaatttcctttccaacccaagacacttctcactgg

SEQ ID NO: 13 - DNA, 114 bp, Homo sapiens
gaaatgccttctcaggtaatggaaggttatccaaatatttttcgtaagtatttcaaatagcaatggctcgtctatggttagtctcacagccacattctcagaactgctcaaacc

SEQ ID NO: 14 - DNA, 114 bp, Homo sapiens
gaaatgccttctcaggtaatggaaggttatccaaatatttttcgtaagtatttcaaatagcaatggctcgtctatggttagtctcgcagccacattctcagaactgctcaaacc

SEQ ID NO: 15 - DNA, 128 bp, Homo sapiens
acccaaaacactggaggggcctcttctcattttcggtagactgcaagtgttagccgtcgggaccagcttctgtctggaagttcgtcaaattgcagttaagtccaagtatgccacatagcagataaggg

SEQ ID NO: 16 - DNA, 128 bp, Homo sapiens
acccaaaacactggaggggcctcttctcattttcggtagactgcaagtgttagccgtcgggaccagcttctgtctggaagttcgtcaaattgcagttaggtccaagtatgccacatagcagataaggg

SEQ ID NO: 17 - DNA, 110 bp, Homo sapiens
gcaccagaatttaaacaacgctgacaataaatatgcagtcgatgatgacttcccagagctccagaagcaactccagcacacagagaggcgctgatgtgcctgtcaggtgc

SEQ ID NO: 18 - DNA, 110 bp, Homo sapiens
gcaccagaatttaaacaacgctgacaataaatatgcagtcgatgatgacttcccagagctccagaagcaactccagcacacggagaggcgctgatgtgcctgtcaggtgc

SEQ ID NO: 19 - DNA, 116 bp, Homo sapiens
tgactgtataccccaggtgcacccttgggtcatctctatcatagaacttatctcacagagtataagagctgatttctgtgtctgcctctcacactagacttccacatccttagtgc

SEQ ID NO: 20 - DNA, 116 bp, Homo sapiens
tgactgtataccccaggtgcacccttgggtcatctctatcatagaacttatctcacagagtataagagctgatttctgtgtctgcctgtcacactagacttccacatccttagtgc

SEQ ID NO: 21 - DNA, 110 bp, Homo sapiens
tgtacgtggtcaccaggggacgcctggcgctgcgagggaggccccgagcctcgtgcccccgtgaagcttcagctcccctccccggctgtccttgaggctcttctcacact

SEQ ID NO: 22 - DNA, 110 bp, Homo sapiens
tgtacgtggtcaccaggggacgcctggcgctgcgagggaggccccgagcctcgtgcccccgtgaagcttcagctcccctccctggctgtccttgaggctcttctcacact

SEQ ID NO: 23 - DNA, 114 bp, Homo sapiens
cagtggaccctgctgcacctttcctcccctcccatcaacctcttttgtgcctccccctccgtgtaccaccttctctgtcaccaaccctggcctcacaactctctcctttgccac

SEQ ID NO: 24 - DNA, 114 bp, Homo sapiens
cagtggaccctgctgcacctttcctcccctcccatcaacctcttttgtgcctccccctccgtgtaccaccttctctgtcaccacccctggcctcacaactctctcctttgccac

SEQ ID NO: 25 - DNA, 110 bp, Homo sapiens
cagtggcatagtagtccaggggctcctcctcagcacctccagcaccttccaggaggcagcagcgcaggcagagaacccgctggaagaatcggcggaagttgtcggagagg

SEQ ID NO: 26 - DNA, 110 bp, Homo sapiens
cagtggcatagtagtccaggggctcctcctcagcacctccagcaccttccaggaggcagcagcgcaggcagagaacccgctggaaggatcggcggaagttgtcggagagg

SEQ ID NO: 27 - DNA, 129 bp, Homo sapiens
aggtctgggggccgctgaatgccaagctgggaatcttaaatgttaaggaacaaggtcatacaatgaatggtgtgatgtaaaagcttgggaggtgatttctgagggtaggtgctgggtttaatgggagga

SEQ ID NO: 28 - DNA, 129 bp, Homo sapiens
aggtctgggggccgctgaatgccaagctgggaatcttaaatgttaaggaacaaggtcatacaatgaatggtgtgatgtaaaagcttgggaggtgatttttgagggtaggtgctgggtttaatgggagga

SEQ ID NO: 29 - DNA, 107 bp, Homo sapiens
acggttctgtcctgtaggggagaaaagtcctcgttgttcctctgggatgcaacatgagagagcagcacactgaggctttatggattgccctgccacaagtgaacagg

SEQ ID NO: 30 - DNA, 107 bp, Homo sapiens
acggttctgtcctgtaggggagaaaagtcctcgttgttcctctgggatgcaacatgagagagcagcacactgaggctttatgggttgccctgccacaagtgaacagg

SEQ ID NO: 31 - DNA, 127 bp, Homo sapiens
gcgcagtcagatgggcgtgctggcgtctgtcttctctctctcctgctctctggcttcatttttctctccttctgtctcaccttctttcgtgtgcctgtgcacacacacgtttgggacaagggctgga

SEQ ID NO: 32 - DNA, 127 bp, Homo sapiens
gcgcagtcagatgggcgtgctggcgtctgtcttctctctctcctgctctctggcttcatttttctctccttctgtctcaccttctttcgtgtgcctgtgcatacacacgtttgggacaagggctgga

SEQ ID NO: 33 - DNA, 130 bp, Homo sapiens
gccggacctgcgaaatcccaaaatgccaaacattcccgcctcacatgatcccagagagaggggacccagtgttcccagcttgcagctgaggagcccgaggttgccgtcagatcagagccccagttgcccg

SEQ ID NO: 34 - DNA, 130 bp, Homo sapiens
gccggacctgcgaaatcccaaaatgccaaacattcccgcctcacatgatcccagagagaggggacccagtgttcccagcttgcagctgaggagcccgagtttgccgtcagatcagagccccagttgcccg

SEQ ID NO: 35 - DNA, 121 bp, Homo sapiens
agcagcctccctcgactagctcacactacgataaggaaaattcatgagctggtgtccaaggagggctgggtgactcgtggctcagtcagcatcaagattcctttcgtctttcccctctgcc

SEQ ID NO: 36 - DNA, 121 bp, Homo sapiens
agcagcctccctcgactagctcacactacgataaggaaaattcatgagctggtgtccaaggagggctgggtgactcgtggctcagtcagcgtcaagattcctttcgtctttcccctctgcc

SEQ ID NO: 37 - DNA, 138 bp, Homo sapiens
tggcattgcctgtaatatacatagccatggttttttataggcaatttaagatgaatagcttctaaactatagataagtttcattaccccaggaagctgaactatagctactttacccaaaatcattagaatggtgctt

SEQ ID NO: 38 - DNA, 138 bp, Homo sapiens
tggcattgcctgtaatatacatagccatggttttttataggcaatttaagatgaatagcttctaaactatagataagtttcattaccccaggaagctgaactatagctactttccccaaaatcattagaatggtgctt

SEQ ID NO: 39 - DNA, 136 bp, Homo sapiens
atgaagccttccaccaactgcctgtatgactcatctggggacttctgctctatactcaaagtggcttagtcactgccaatgtatttccatatgagggacgatgattactaaggaaatatagaaacaacaactgatc

SEQ ID NO: 40 - DNA, 136 bp, Homo sapiens
atgaagccttccaccaactgcctgtatgactcatctggggacttctgctctatactcaaagtggcttagtcactgccaatgtatttccatatgagggacggtgattactaaggaaatatagaaacaacaactgatc

SEQ ID NO: 41 - DNA, 118 bp, Homo sapiens
acaacagaatcaggtgattggagaaaagatcacaggcctaggcacccaaggcttgaaggatgaaagaatgaaagatggacggaacaaaattaggaccttaattctttgttcagttcag

SEQ ID NO: 42 - DNA, 118 bp, Homo sapiens
acaacagaatcaggtgattggagaaaagatcacaggcctaggcacccaaggcttgaaggatgaaagaatgaaagatggacggaagaaaattaggaccttaattctttgttcagttcag

SEQ ID NO: 43 - DNA, 150 bp, Homo sapiens
ttggggtaaattttcattgtcatatgtggaatttaaatataccatcatctacaaagaattccacagagttaaatatcttaagttaaacacttaaaataagtgtttgcgtgatattttgatgacagataaacagagtctaattcccacccc

SEQ ID NO: 44 - DNA, 150 bp, Homo sapiens
ttggggtaaattttcattgtcatatgtggaatttaaatataccatcatctacaaagaattccacagagttaaatatcttaagttaaacacttaaaataagtgtttgcgtgatattttgatgatagataaacagagtctaattcccacccc

SEQ ID NO: 45 - DNA, 145 bp, Homo sapiens
tgcaattcaaatcaggaagtatgaccaaaagacagagatcttttttggatgatccctagcctagcaatgcctggcagccatgcaggtgcaatgtcaaccttaaataatgtattgcaaactcagagctgacaaacctcgatgttgc

SEQ ID NO: 46 - DNA, 145 bp, Homo sapiens
tgcaattcaaatcaggaagtatgaccaaaagacagagatcttttttggatgatccctagcctagcaatgcctggcagccatgcaggtgcaatgtcaaccttaaataatgtattgcaaattcagagctgacaaacctcgatgttgc

SEQ ID NO: 47 - DNA, 124 bp, Homo sapiens
ctgtgctctgcgaatagctgcagaagtaacttggggacccaaaataaagcagaatgctaatgtcaagtcctgagaaccaagccctgggactctggtgccatttcggattctccatgagcatggt

SEQ ID NO: 48 - DNA, 124 bp, Homo sapiens
ctgtgctctgcgaatagctgcagaagtaacttggggacccaaaataaagcagaatgctaatgtcaagtcctgagaaccaagccctgggactctggtgccattttggattctccatgagcatggt

SEQ ID NO: 49 - DNA, 118 bp, Homo sapiens
tttttccagccaactcaaggccaaaaaaaatttcttaatatagttattatgcgaggggaggggaagcaaaggagcacaggtagtccacagaataagacacaagaaacctcaagctgtg

SEQ ID NO: 50 - DNA, 118 bp, Homo sapiens
tttttccagccaactcaaggccaaaaaaaatttcttaatatagttattatgcgaggggaggggaagcaaaggagcacaggtagtccacagaataggacacaagaaacctcaagctgtg

SEQ ID NO: 51 - DNA, 110 bp, Homo sapiens
tcttctcgtcccctaagcaaacaacatccgcttgcttctgtctgtgtaaccacagtgaatgggtgtgcacgcttgatgggcctctgagcccctgttgcacaaaccagaaa

SEQ ID NO: 52 - DNA, 110 bp, Homo sapiens
tcttctcgtcccctaagcaaacaacatccgcttgcttctgtctgtgtaaccacagtgaatgggtgtgcacgcttggtgggcctctgagcccctgttgcacaaaccagaaa

SEQ ID NO: 53 - DNA, 110 bp, Homo sapiens
cacatgggggcattaagaatcgcccagggaggaggagggagaacgcgtgcttttcacatttgcatttgaattttcgagttcccaggatgtgtttttgtgctcatcgatgt

SEQ ID NO: 54 - DNA, 110 bp, Homo sapiens
cacatgggggcattaagaatcgcccagggaggaggagggagaacgcgtgcttttcacatttgcatttgaatttttgagttcccaggatgtgtttttgtgctcatcgatgt

SEQ ID NO: 55 - DNA, 128 bp, Homo sapiens
gggctctgaggtgtgtgaaataaaaacaaatgtccatgtctgtccttttatggcattttgggactttacatttcaaacatttcagacatgtatcacaacacgaaggaataacagttccagggatatct

SEQ ID NO: 56 - DNA, 128 bp, Homo sapiens
gggctctgaggtgtgtgaaataaaaacaaatgtccatgtctgtccttttatggcattttgggactttacatttcaaacatttcagacatgtatcacaacacgagggaataacagttccagggatatct

SEQ ID NO: 57 - DNA, 21 bp, Artificial Sequence
  Description of Artificial Sequence: Synthetic primer
cacatgcacagccagcaaccc

SEQ ID NO: 58 - DNA, 23 bp, Artificial Sequence
  Description of Artificial Sequence: Synthetic primer
ccccaaggtcctgtgacctgagt

SEQ ID NO: 59 - DNA, 23 bp, Artificial Sequence
  Description of Artificial Sequence: Synthetic primer
tgaggaagtgaggctcagagggt

SEQ ID NO: 60 - DNA, 24 bp, Artificial Sequence
  Description of Artificial Sequence: Synthetic primer
tgccagtgcgagatgaaagtcttt

SEQ ID NO: 61 - DNA, 27 bp, Artificial Sequence
  Description of Artificial Sequence: Synthetic primer
gtgccttcagaacctttgagatctgat

SEQ ID NO: 62 - DNA, 20 bp, Artificial Sequence
  Description of Artificial Sequence: Synthetic primer
tcccatcccaccagccaccc

SEQ ID NO: 63 - DNA, 25 bp, Artificial Sequence
  Description of Artificial Sequence: Synthetic primer
aggtgtgtctctcttttgtgagggg

SEQ ID NO: 64 - DNA, 21 bp, Artificial Sequence
  Description of Artificial Sequence: Synthetic primer
cctttgtcccacctccccacc

SEQ ID NO: 65 - DNA, 26 bp, Artificial Sequence
  Description of Artificial Sequence: Synthetic primer
cctcgcctactgtgctgtttctaacc

SEQ ID NO: 66 - DNA, 25 bp, Artificial Sequence
  Description of Artificial Sequence: Synthetic primer
ccatcccagctgagtattccaggag

SEQ ID NO: 67 - DNA, 26 bp, Artificial Sequence
  Description of Artificial Sequence: Synthetic primer
aattgcaatggtgagaggttgatggt

SEQ ID NO: 68 - DNA, 24 bp, Artificial Sequence
  Description of Artificial Sequence: Synthetic primer
ccagtgagaagtgtcttgggttgg

SEQ ID NO: 69 - DNA, 27 bp, Artificial Sequence
  Description of Artificial Sequence: Synthetic primer
gaaatgccttctcaggtaatggaaggt

SEQ ID NO: 70 - DNA, 27 bp, Artificial Sequence
  Description of Artificial Sequence: Synthetic primer
ggtttgagcagttctgagaatgtggct

SEQ ID NO: 71 - DNA, 22 bp, Artificial Sequence
  Description of Artificial Sequence: Synthetic primer
acccaaaacactggaggggcct

SEQ ID NO: 72 - DNA, 27 bp, Artificial Sequence
  Description of Artificial Sequence: Synthetic primer
cccttatctgctatgtggcatacttgg

SEQ ID NO: 73 - DNA, 27 bp, Artificial Sequence
  Description of Artificial Sequence: Synthetic primer
gcaccagaatttaaacaacgctgacaa

SEQ ID NO: 74 - DNA, 22 bp, Artificial Sequence
  Description of Artificial Sequence: Synthetic primer
gcacctgacaggcacatcagcg

SEQ ID NO: 75 - DNA, 24 bp, Artificial Sequence
  Description of Artificial Sequence: Synthetic primer
tgactgtataccccaggtgcaccc

SEQ ID NO: 76 - DNA, 27 bp, Artificial Sequence
  Description of Artificial Sequence: Synthetic primer
gcactaaggatgtggaagtctagtgtg

SEQ ID NO: 77 - DNA, 22 bp, Artificial Sequence
  Description of Artificial Sequence: Synthetic primer
tgtacgtggtcaccaggggacg

SEQ ID NO: 78 - DNA, 26 bp, Artificial Sequence
  Description of Artificial Sequence: Synthetic primer
agtgtgagaagagcctcaaggacagc

SEQ ID NO: 79 - DNA, 21 bp, Artificial Sequence
  Description of Artificial Sequence: Synthetic primer
cagtggaccctgctgcacctt

SEQ ID NO: 80 - DNA, 24 bp, Artificial Sequence
  Description of Artificial Sequence: Synthetic primer
gtggcaaaggagagagttgtgagg

SEQ ID NO: 81 - DNA, 24 bp, Artificial Sequence
  Description of Artificial Sequence: Synthetic primer
cagtggcatagtagtccaggggct

SEQ ID NO: 82 - DNA, 21 bp, Artificial Sequence
  Description of Artificial Sequence: Synthetic primer
cctctccgacaacttccgccg

SEQ ID NO: 83 - DNA, 20 bp, Artificial Sequence
  Description of Artificial Sequence: Synthetic primer
aggtctgggggccgctgaat

SEQ ID NO: 84 - DNA, 23 bp, Artificial Sequence
  Description of Artificial Sequence: Synthetic primer
tcctcccattaaacccagcacct

SEQ ID NO: 85 - DNA, 23 bp, Artificial Sequence
  Description of Artificial Sequence: Synthetic primer
acggttctgtcctgtaggggaga

SEQ ID NO: 86 - DNA, 22 bp, Artificial Sequence
  Description of Artificial Sequence: Synthetic primer
cctgttcacttgtggcagggca

SEQ ID NO: 87 - DNA, 20 bp, Artificial Sequence
  Description of Artificial Sequence: Synthetic primer
gcgcagtcagatgggcgtgc

SEQ ID NO: 88 - DNA, 23 bp, Artificial Sequence
  Description of Artificial Sequence: Synthetic primer
tccagcccttgtcccaaacgtgt

SEQ ID NO: 89 - DNA, 21 bp, Artificial Sequence
  Description of Artificial Sequence: Synthetic primer
gccggacctgcgaaatcccaa

SEQ ID NO: 90 - DNA, 21 bp, Artificial Sequence
  Description of Artificial Sequence: Synthetic primer
cgggcaactggggctctgatc

SEQ ID NO: 91 - DNA, 21 bp, Artificial Sequence
  Description of Artificial Sequence: Synthetic primer
agcagcctccctcgactagct

SEQ ID NO: 92 - DNA, 23 bp, Artificial Sequence
  Description of Artificial Sequence: Synthetic primer
ggcagaggggaaagacgaaagga

SEQ ID NO: 93 - DNA, 24 bp, Artificial Sequence
  Description of Artificial Sequence: Synthetic primer
tggcattgcctgtaatatacatag

SEQ ID NO: 94 - DNA, 23 bp, Artificial Sequence
  Description of Artificial Sequence: Synthetic primer
aagcaccattctaatgattttgg

SEQ ID NO: 95 - DNA, 20 bp, Artificial Sequence
  Description of Artificial Sequence: Synthetic primer
atgaagccttccaccaactg

SEQ ID NO: 96 - DNA, 27 bp, Artificial Sequence
  Description of Artificial Sequence: Synthetic primer
gatcagttgttgtttctatatttcctt

SEQ ID NO: 97 - DNA, 22 bp, Artificial Sequence
  Description of Artificial Sequence: Synthetic primer
acaacagaatcaggtgattgga

SEQ ID NO: 98 - DNA, 25 bp, Artificial Sequence
  Description of Artificial Sequence: Synthetic primer
ctgaactgaacaaagaattaaggtc

SEQ ID NO: 99 - DNA, 22 bp, Artificial Sequence
  Description of Artificial Sequence: Synthetic primer
ttggggtaaattttcattgtca

SEQ ID NO: 100 - DNA, 20 bp, Artificial Sequence
  Description of Artificial Sequence: Synthetic primer
ggggtgggaattagactctg

SEQ ID NO: 101 - DNA, 23 bp, Artificial Sequence
  Description of Artificial Sequence: Synthetic primer
tgcaattcaaatcaggaagtatg

SEQ ID NO: 102 - DNA, 20 bp, Artificial Sequence
  Description of Artificial Sequence: Synthetic primer
gcaacatcgaggtttgtcag

SEQ ID NO: 103 - DNA, 20 bp, Artificial Sequence
  Description of Artificial Sequence: Synthetic primer
ctgtgctctgcgaatagctg

SEQ ID NO: 104 - DNA, 20 bp, Artificial Sequence
  Description of Artificial Sequence: Synthetic primer
accatgctcatggagaatcc

SEQ ID NO: 105 - DNA, 20 bp, Artificial Sequence
  Description of Artificial Sequence: Synthetic primer
tttttccagccaactcaagg

SEQ ID NO: 106 - DNA, 21 bp, Artificial Sequence
  Description of Artificial Sequence: Synthetic primer
cacagcttgaggtttcttgtg

SEQ ID NO: 107 - DNA, 20 bp, Artificial Sequence
  Description of Artificial Sequence: Synthetic primer
tcttctcgtcccctaagcaa

SEQ ID NO: 108 - DNA, 20 bp, Artificial Sequence
  Description of Artificial Sequence: Synthetic primer
tttctggtttgtgcaacagg

SEQ ID NO: 109 - DNA, 20 bp, Artificial Sequence
  Description of Artificial Sequence: Synthetic primer
cacatgggggcattaagaat

SEQ ID NO: 110 - DNA, 22 bp, Artificial Sequence
  Description of Artificial Sequence: Synthetic primer
acatcgatgagcacaaaaacac

SEQ ID NO: 111 - DNA, 20 bp, Artificial Sequence
  Description of Artificial Sequence: Synthetic primer
gggctctgaggtgtgtgaaa

SEQ ID NO: 112 - DNA, 24 bp, Artificial Sequence
  Description of Artificial Sequence: Synthetic primer
agatatccctggaactgttattcc

SEQ ID NO: 113 - DNA, 23 bp, Artificial Sequence
  Description of Artificial Sequence: Synthetic primer
acagtaactgccttcatagatag

SEQ ID NO: 114 - DNA, 22 bp, Artificial Sequence
  Description of Artificial Sequence: Synthetic primer
gtgtcagaccctgttctaagta

SEQ ID NO: 115 - DNA, 26 bp, Artificial Sequence
  Description of Artificial Sequence: Synthetic primer
aaataaaattaggcatatttacaagc

SEQ ID NO: 116 - DNA, 23 bp, Artificial Sequence
  Description of Artificial Sequence: Synthetic primer
gctgagtgatttgtctgtaattg

SEQ ID NO: 117 - DNA, 21 bp, Artificial Sequence
  Description of Artificial Sequence: Synthetic primer
cctgttcctcccttatttccc

SEQ ID NO: 118 - DNA, 21 bp, Artificial Sequence
  Description of Artificial Sequence: Synthetic primer
gggaacacagactccatggtg

SEQ ID NO: 119 - DNA, 22 bp, Artificial Sequence
  Description of Artificial Sequence: Synthetic primer
cttagggaaccctcactgaatg

SEQ ID NO: 120 - DNA, 22 bp, Artificial Sequence
  Description of Artificial Sequence: Synthetic primer
gtccttgtcagcgtttatttgc

SEQ ID NO: 121 - DNA, 26 bp, Artificial Sequence
  Description of Artificial Sequence: Synthetic primer
aataatcagtatgtgacttggattga

SEQ ID NO: 122 - DNA, 22 bp, Artificial Sequence
  Description of Artificial Sequence: Synthetic primer
ataggatggatggatagatgga

SEQ ID NO: 123 - DNA, 21 bp, Artificial Sequence
  Description of Artificial Sequence: Synthetic primer
cagagcaagaccctgtctcat

SEQ ID NO: 124 - DNA, 21 bp, Artificial Sequence
  Description of Artificial Sequence: Synthetic primer
tcaacagaggcttgcatgtat

SEQ ID NO: 125 - DNA, 20 bp, Artificial Sequence
  Description of Artificial Sequence: Synthetic primer
gggtgattttcctctttggt

SEQ ID NO: 126 - DNA, 33 bp, Artificial Sequence
  Description of Artificial Sequence: Synthetic primer
aacatttgtatctttatctgtatccttatttat

SEQ ID NO: 127 - DNA, 27 bp, Artificial Sequence
  Description of Artificial Sequence: Synthetic primer
gaacacttgtcatagtttagaacgaac

SEQ ID NO: 128 - DNA, 20 bp, Artificial Sequence
  Description of Artificial Sequence: Synthetic primer
tcattgacagaattgcacca

SEQ ID NO: 129 - DNA, 27 bp, Artificial Sequence
  Description of Artificial Sequence: Synthetic primer
tttgtatttcatgtgtacattcgtatc

SEQ ID NO: 130 - DNA, 28 bp, Artificial Sequence
  Description of Artificial Sequence: Synthetic primer
acctatcctgtagattattttcactgtg

SEQ ID NO: 131 - DNA, 20 bp, Artificial Sequence
  Description of Artificial Sequence: Synthetic primer
tctgacccatctaacgccta

SEQ ID NO: 132 - DNA, 27 bp, Artificial Sequence
  Description of Artificial Sequence: Synthetic primer
cagacagaaagatagatagatgattga

SEQ ID NO: 133 - DNA, 21 bp, Artificial Sequence
  Description of Artificial Sequence: Synthetic primer
atacagacagacagacaggtg

SEQ ID NO: 134 - DNA, 23 bp, Artificial Sequence
  Description of Artificial Sequence: Synthetic primer
gcatgtatctatcatccatctct

SEQ ID NO: 135 - DNA, 21 bp, Artificial Sequence
  Description of Artificial Sequence: Synthetic primer
tgagtgacaaattgagacctt

SEQ ID NO: 136 - DNA, 26 bp, Artificial Sequence
  Description of Artificial Sequence: Synthetic primer
gtcttacaataacagttgctactatt

SEQ ID NO: 137 - DNA, 18 bp, Artificial Sequence
  Description of Artificial Sequence: Synthetic primer
attccccaagtgaattgc

SEQ ID NO: 138 - DNA, 26 bp, Artificial Sequence
  Description of Artificial Sequence: Synthetic primer
ggtagatagactggatagatagacga

SEQ ID NO: 139 - DNA, 20 bp, Artificial Sequence
  Description of Artificial Sequence: Synthetic primer
tggaaacagaaatggcttgg

SEQ ID NO: 140 - DNA, 20 bp, Artificial Sequence
  Description of Artificial Sequence: Synthetic primer
gattgcaggagggaaggaag

SEQ ID NO: 141 - DNA, 22 bp, Artificial Sequence
  Description of Artificial Sequence: Synthetic primer
gagcaagacaccatctcaagaa

SEQ ID NO: 142 - DNA, 30 bp, Artificial Sequence
  Description of Artificial Sequence: Synthetic primer
gaaattttacatttatgtttatgattctct

SEQ ID NO: 143 - DNA, 18 bp, Artificial Sequence
  Description of Artificial Sequence: Synthetic primer
ggcgactgagcaagactc

SEQ ID NO: 144 - DNA, 27 bp, Artificial Sequence
  Description of Artificial Sequence: Synthetic primer
ggttattaattgagaaaactccttaca

SEQ ID NO: 145 - DNA, 23 bp, Artificial Sequence
  Description of Artificial Sequence: Synthetic primer
attttccccgatgatagtagtct

SEQ ID NO: 146 - DNA, 26 bp, Artificial Sequence
  Description of Artificial Sequence: Synthetic primer
gcgaatgtatgattggcaatattttt

SEQ ID NO: 147 - DNA, 27 bp, Artificial Sequence
  Description of Artificial Sequence: Synthetic primer
acatgtatcccagaacttaaagtaaac

SEQ ID NO: 148 - DNA, 22 bp, Artificial Sequence
  Description of Artificial Sequence: Synthetic primer
gcagaagggaaaattgaagctg

SEQ ID NO: 149 - DNA, 22 bp, Artificial Sequence
  Description of Artificial Sequence: Synthetic primer
cagagacaccgaaccaataaga

SEQ ID NO: 150 - DNA, 27 bp, Artificial Sequence
  Description of Artificial Sequence: Synthetic primer
gccacatgaatcaattcctataataaa

SEQ ID NO: 151 - DNA, 25 bp, Artificial Sequence
  Description of Artificial Sequence: Synthetic primer
gcacatgtaccctaaaacttaaaat

SEQ ID NO: 152 - DNA, 26 bp, Artificial Sequence
  Description of Artificial Sequence: Synthetic primer
gtcaaccaaaactcaacaagtagtaa

SEQ ID NO: 153 - DNA, 25 bp, Artificial Sequence
  Description of Artificial Sequence: Synthetic primer
aagatgaaattgccatgtaaaaata

SEQ ID NO: 154 - DNA, 27 bp, Artificial Sequence
  Description of Artificial Sequence: Synthetic primer
gtgtgtataacaaaattcctatgatgg

SEQ ID NO: 155 - DNA, 22 bp, Artificial Sequence
  Description of Artificial Sequence: Synthetic primer
gcacccaaaactgaatgtcata

SEQ ID NO: 156 - DNA, 20 bp, Artificial Sequence
  Description of Artificial Sequence: Synthetic primer
ggtgagagtgagaccctgtc

SEQ ID NO: 157 - DNA, 27 bp, Artificial Sequence
  Description of Artificial Sequence: Synthetic primer
tgtaataactctacgactgtctgtctg

SEQ ID NO: 158 - DNA, 21 bp, Artificial Sequence
  Description of Artificial Sequence: Synthetic primer
gaataggaggtggatggatgg

SEQ ID NO: 159 - DNA, 20 bp, Artificial Sequence
  Description of Artificial Sequence: Synthetic primer
gagcgagaccctgtctcaag

SEQ ID NO: 160 - DNA, 24 bp, Artificial Sequence
  Description of Artificial Sequence: Synthetic primer
ggaaaagacataggatagcaattt

SEQ ID NO: 161 - DNA, 21 bp, Artificial Sequence
  Description of Artificial Sequence: Synthetic primer
tctggattgatctgtctgtcc

SEQ ID NO: 162 - DNA, 26 bp, Artificial Sequence
  Description of Artificial Sequence: Synthetic primer
gaattaaataccatctgagcactgaa

SEQ ID NO: 163 - DNA, 27 bp, Artificial Sequence
  Description of Artificial Sequence: Synthetic primer
tgttataatgcattgagttttattctg

SEQ ID NO: 164 - DNA, 28 bp, Artificial Sequence
  Description of Artificial Sequence: Synthetic primer
gcctgtctcaaaaataaagagatagaca

SEQ ID NO: 165 - DNA, 25 bp, Artificial Sequence
  Description of Artificial Sequence: Synthetic primer
ttaatgaattgaacaaatgagtgag

SEQ ID NO: 166 - DNA, 25 bp, Artificial Sequence
  Description of Artificial Sequence: Synthetic primer
gcaactctggttgtattgtcttcat

SEQ ID NO: 167 - DNA, 21 bp, Artificial Sequence
  Description of Artificial Sequence: Synthetic primer
caaagcgagactctgtctcaa

SEQ ID NO: 168 - DNA, 27 bp, Artificial Sequence
  Description of Artificial Sequence: Synthetic primer
gaaaatgctatcctctttggtataaat

SEQ ID NO: 169 - DNA, 27 bp, Artificial Sequence
  Description of Artificial Sequence: Synthetic primer
gggtatttcaagataactgtagatagg

SEQ ID NO: 170 - DNA, 24 bp, Artificial Sequence
  Description of Artificial Sequence: Synthetic primer
gcttctgaaagcttctagtttacc

SEQ ID NO: 171 - DNA, 19 bp, Artificial Sequence
  Description of Artificial Sequence: Synthetic primer
tccacatcctcaccaacac

SEQ ID NO: 172 - DNA, 21 bp, Artificial Sequence
  Description of Artificial Sequence: Synthetic primer
gcctaggaaggctactgtcaa

SEQ ID NO: 173 - DNA, 18 bp, Artificial Sequence
  Description of Artificial Sequence: Synthetic primer
ccacccgtccatttaggc

SEQ ID NO: 174 - DNA, 27 bp, Artificial Sequence
  Description of Artificial Sequence: Synthetic primer
gtgaaaaagtagatataatggttggtg

SEQ ID NO: 175 - DNA, 25 bp, Artificial Sequence
  Description of Artificial Sequence: Synthetic primer
ggttttccaagagatagaccaatta

SEQ ID NO: 176 - DNA, 27 bp, Artificial Sequence
  Description of Artificial Sequence: Synthetic primer
gtcctctcataaatccctactcatatc

SEQ ID NO: 177 - DNA, 27 bp, Artificial Sequence
  Description of Artificial Sequence: Synthetic primer
ctgttggtacataataggtaggtaggt

SEQ ID NO: 178 - DNA, 19 bp, Artificial Sequence
  Description of Artificial Sequence: Synthetic primer
gtcgtgggccccataaatc

SEQ ID NO: 179 - DNA, 27 bp, Artificial Sequence
  Description of Artificial Sequence: Synthetic primer
aaggtacataacagttcaatagaaagc

SEQ ID NO: 180 - DNA, 26 bp, Artificial Sequence
  Description of Artificial Sequence: Synthetic primer
gtgaaatgactgaaaaatagtaacca

SEQ ID NO: 181 - DNA, 24 bp, Artificial Sequence
  Description of Artificial Sequence: Synthetic primer
ctaggagatcatgtgggtatgatt

SEQ ID NO: 182 - DNA, 24 bp, Artificial Sequence
  Description of Artificial Sequence: Synthetic primer
gcagtgaataaatgaacgaatgga

SEQ ID NO: 183 - DNA, 21 bp, Artificial Sequence
  Description of Artificial Sequence: Synthetic primer
cccaaaattacttgagccaat

SEQ ID NO: 184 - DNA, 24 bp, Artificial Sequence
  Description of Artificial Sequence: Synthetic primer
gagacaaaatgaagaaacagacag

SEQ ID NO: 185 - DNA, 25 bp, Artificial Sequence
  Description of Artificial Sequence: Synthetic primer
tctttgctctcatgaatagatcagt

SEQ ID NO: 186 - DNA, 24 bp, Artificial Sequence
  Description of Artificial Sequence: Synthetic primer
gtttgtgataatgaacccactcag

SEQ ID NO: 187 - DNA, 27 bp, Artificial Sequence
  Description of Artificial Sequence: Synthetic primer
tgaacacagatgttaagtgtgtatatg

SEQ ID NO: 188 - DNA, 23 bp, Artificial Sequence
  Description of Artificial Sequence: Synthetic primer
gtctgaggtggacagttatgaaa

SEQ ID NO: 189 - DNA, 23 bp, Artificial Sequence
  Description of Artificial Sequence: Synthetic primer
ctgtggctcatctatgaaaactt

SEQ ID NO: 190 - DNA, 22 bp, Artificial Sequence
  Description of Artificial Sequence: Synthetic primer
gaagtggctgtggtgttatgat

SEQ ID NO: 191 - DNA, 24 bp, Artificial Sequence
  Description of Artificial Sequence: Synthetic primer
ttctgttggtatagagcagtgttt

SEQ ID NO: 192 - DNA, 20 bp, Artificial Sequence
  Description of Artificial Sequence: Synthetic primer
gtgacaggaaggacggaatg

SEQ ID NO: 193 - DNA, 27 bp, Artificial Sequence
  Description of Artificial Sequence: Synthetic primer
catgaggtttgcaaatactatcttaac

SEQ ID NO: 194 - DNA, 24 bp, Artificial Sequence
  Description of Artificial Sequence: Synthetic primer
gttttaattttctccaaatctcca

SEQ ID NO: 195 - DNA, 27 bp, Artificial Sequence
  Description of Artificial Sequence: Synthetic primer
tcttagcctagatagatacttgcttcc

SEQ ID NO: 196 - DNA, 23 bp, Artificial Sequence
  Description of Artificial Sequence: Synthetic primer
gtcaacctttgaggctataggaa

SEQ ID NO: 197 - DNA, 19 bp, Artificial Sequence
  Description of Artificial Sequence: Synthetic primer
tcctggaaacaaaagtatt

SEQ ID NO: 198 - DNA, 21 bp, Artificial Sequence
  Description of Artificial Sequence: Synthetic primer
aaccttacaacaaagctagaa

SEQ ID NO: 199 - DNA, 20 bp, Artificial Sequence
  Description of Artificial Sequence: Synthetic primer
actaagccttggggatccag

SEQ ID NO: 200 - DNA, 21 bp, Artificial Sequence
  Description of Artificial Sequence: Synthetic primer
tgctgtggaaatactaaaagg

SEQ ID NO: 201 - DNA, 20 bp, Artificial Sequence
  Description of Artificial Sequence: Synthetic primer
ctccagaggtaatcctgtga

SEQ ID NO: 202 - DNA, 21 bp, Artificial Sequence
  Description of Artificial Sequence: Synthetic primer
tggtgtgagatggtatctagg

SEQ ID NO: 203 - DNA, 22 bp, Artificial Sequence
  Description of Artificial Sequence: Synthetic primer
gtataatccatgaatcttgttt

SEQ ID NO: 204 - DNA, 22 bp, Artificial Sequence
  Description of Artificial Sequence: Synthetic primer
ttcaaattgtatataagagagt

SEQ ID NO: 205 - DNA, 20 bp, Artificial Sequence
  Description of Artificial Sequence: Synthetic primer
gcaggaaagttatttttaat

SEQ ID NO: 206 - DNA, 21 bp, Artificial Sequence
  Description of Artificial Sequence: Synthetic primer
tgcttgagaaagctaacactt

SEQ ID NO: 207 - DNA, 20 bp, Artificial Sequence
  Description of Artificial Sequence: Synthetic primer
cagtgtttggaaattgtctg

SEQ ID NO: 208 - DNA, 20 bp, Artificial Sequence
  Description of Artificial Sequence: Synthetic primer
ggcactgggagattattgta

SEQ ID NO: 209 - DNA, 20 bp, Artificial Sequence
  Description of Artificial Sequence: Synthetic primer
tcctgttgttaagtacacat

SEQ ID NO: 210 - DNA, 18 bp, Artificial Sequence
  Description of Artificial Sequence: Synthetic primer
gggccgtaattacttttg

SEQ ID NO: 211 - DNA, 21 bp, Artificial Sequence
  Description of Artificial Sequence: Synthetic primer
actcagtaggcactttgtgtc

SEQ ID NO: 212 - DNA, 18 bp, Artificial Sequence
  Description of Artificial Sequence: Synthetic primer
tcttccaccacaccaatc

SEQ ID NO: 213 - DNA, 19 bp, Artificial Sequence
  Description of Artificial Sequence: Synthetic primer
tggcttttcaaaggtaaaa

SEQ ID NO: 214 - DNA, 21 bp, Artificial Sequence
  Description of Artificial Sequence: Synthetic primer
gcaacgttaacatctgaattt

SEQ ID NO: 215 - skipped

SEQ ID NO: 216 - DNA, 22 bp, Artificial Sequence
  Description of Artificial Sequence: Synthetic primer
attttatatgtcatgatctaag

SEQ ID NO: 217 - DNA, 19 bp, Artificial Sequence
  Description of Artificial Sequence: Synthetic primer
agagattacaggtgtgagc

SEQ ID NO: 218 - DNA, 19 bp, Artificial Sequence
  Description of Artificial Sequence: Synthetic primer
atgatcctcaactgcctct

SEQ ID NO: 219 - DNA, 20 bp, Artificial Sequence
  Description of Artificial Sequence: Synthetic primer
tgaaactcaaaagagaaaag

SEQ ID NO: 220 - DNA, 20 bp, Artificial Sequence
  Description of Artificial Sequence: Synthetic primer
acagatttctacttaaaatt

SEQ ID NO: 221 - DNA, 20 bp, Artificial Sequence
  Description of Artificial Sequence: Synthetic primer
tgaaactcaaaagagaaaag

SEQ ID NO: 222 - DNA, 20 bp, Artificial Sequence
  Description of Artificial Sequence: Synthetic primer
acagatttctacttaaaatt

SEQ ID NO: 223 - DNA, 20 bp, Artificial Sequence
  Description of Artificial Sequence: Synthetic primer
gcaaaggggtactctatgta

SEQ ID NO: 224 - DNA, 20 bp, Artificial Sequence
  Description of Artificial Sequence: Synthetic primer
tatcgggtcatcttgttaaa

SEQ ID NO: 225 - DNA, 22 bp, Artificial Sequence
  Description of Artificial Sequence: Synthetic primer
tctaacaaagctctgtccaaaa

SEQ ID NO: 226 - DNA, 21 bp, Artificial Sequence
  Description of Artificial Sequence: Synthetic primer
ccacactgaataactggaaca

SEQ ID NO: 227 - DNA, 21 bp, Artificial Sequence
  Description of Artificial Sequence: Synthetic primer
gcaagcaagctctctaccttc

SEQ ID NO: 228 - DNA, 22 bp, Artificial Sequence
  Description of Artificial Sequence: Synthetic primer
tgttcttccaaaattcacatgc

SEQ ID NO: 229 - DNA, 21 bp, Artificial Sequence
  Description of Artificial Sequence: Synthetic primer
atttcactattccttcatttt

SEQ ID NO: 230 - DNA, 22 bp, Artificial Sequence
  Description of Artificial Sequence: Synthetic primer
taattgttgcacactaaattac

SEQ ID NO: 231 - DNA, 21 bp, Artificial Sequence
  Description of Artificial Sequence: Synthetic primer
aaaaagccacagaaatcagtc

SEQ ID NO: 232 - DNA, 22 bp, Artificial Sequence
  Description of Artificial Sequence: Synthetic primer
ttcttatatctcactgggcatt

SEQ ID NO: 233 - DNA, 22 bp, Artificial Sequence
  Description of Artificial Sequence: Synthetic primer
ggatggtagaagagaagaaagg

SEQ ID NO: 234 - DNA, 22 bp, Artificial Sequence
  Description of Artificial Sequence: Synthetic primer
ggatggtagaagagaagaaagg

SEQ ID NO: 235 - DNA, 20 bp, Artificial Sequence
  Description of Artificial Sequence: Synthetic primer
tgcaaagatgcagaaccaac

SEQ ID NO: 236 - DNA, 22 bp, Artificial Sequence
  Description of Artificial Sequence: Synthetic primer
ttttgttccttgtcctggctga

SEQ ID NO: 237 - DNA, 20 bp, Artificial Sequence
  Description of Artificial Sequence: Synthetic primer
tgcaaagatgcagaaccaac

SEQ ID NO: 238 - DNA, 21 bp, Artificial Sequence
  Description of Artificial Sequence: Synthetic primer
gcctccagctctatccaagtt

SEQ ID NO: 239 - DNA, 22 bp, Artificial Sequence
  Description of Artificial Sequence: Synthetic primer
ccttaatatcttcccatgtcca

SEQ ID NO: 240 - DNA, 22 bp, Artificial Sequence
  Description of Artificial Sequence: Synthetic primer
attgttagtgcctcttctgctt

SEQ ID NO: 241 - DNA, 20 bp, Artificial Sequence
  Description of Artificial Sequence: Synthetic primer
gagaagtgaggtcagcagct

SEQ ID NO: 242 - DNA, 22 bp, Artificial Sequence
  Description of Artificial Sequence: Synthetic primer
tttctaaatttccattgaacag

SEQ ID NO: 243 - DNA, 20 bp, Artificial Sequence
  Description of Artificial Sequence: Synthetic primer
gaaattggcaatctgattct

SEQ ID NO: 244 - DNA, 21 bp, Artificial Sequence
  Description of Artificial Sequence: Synthetic primer
caacttgtcctttattgatgt

SEQ ID NO: 245 - DNA, 22 bp, Artificial Sequence
  Description of Artificial Sequence: Synthetic primer
ctatgttgataaaacattgaaa

SEQ ID NO: 246 - DNA, 20 bp, Artificial Sequence
  Description of Artificial Sequence: Synthetic primer
gcctgtctggaatatagttt

SEQ ID NO: 247 - DNA, 22 bp, Artificial Sequence
  Description of Artificial Sequence: Synthetic primer
cagggcatataatctaagctgt

SEQ ID NO: 248 - DNA, 21 bp, Artificial Sequence
  Description of Artificial Sequence: Synthetic primer
caatgactctgagttgagcac

SEQ ID NO: 249 - DNA, 18 bp, Artificial Sequence
  Description of Artificial Sequence: Synthetic primer
actctctccctcccctct

SEQ ID NO: 250 - DNA, 20 bp, Artificial Sequence
  Description of Artificial Sequence: Synthetic primer
tatggccccaaaactattct

SEQ ID NO: 251 - DNA, 20 bp, Artificial Sequence
  Description of Artificial Sequence: Synthetic primer
acaagtactgggcagattga

SEQ ID NO: 252 - DNA, 20 bp, Artificial Sequence
  Description of Artificial Sequence: Synthetic primer
gccaggtttagctttcaagt

SEQ ID NO: 253 - DNA, 22 bp, Artificial Sequence
  Description of Artificial Sequence: Synthetic primer
ttttatatcaggagaaacactg

SEQ ID NO: 254 - DNA, 21 bp, Artificial Sequence
  Description of Artificial Sequence: Synthetic primer
ccagaattttggaggtttaat

SEQ ID NO: 255 - DNA, 22 bp, Artificial Sequence
  Description of Artificial Sequence: Synthetic primer
tgtcattcctcctttatctcca

SEQ ID NO: 256 - DNA, 20 bp, Artificial Sequence
  Description of Artificial Sequence: Synthetic primer
ttcttttgcctctcccaaag

SEQ ID NO: 257 - DNA, 20 bp, Artificial Sequence
  Description of Artificial Sequence: Synthetic primer
accctggcacagtgttgact

SEQ ID NO: 258 - DNA, 20 bp, Artificial Sequence
  Description of Artificial Sequence: Synthetic primer
tgggcctgagttgagaagat

SEQ ID NO: 259 - DNA, 21 bp, Artificial Sequence
  Description of Artificial Sequence: Synthetic primer
aatttgtaagtatgtgcaacg

SEQ ID NO: 260 - DNA, 20 bp, Artificial Sequence
  Description of Artificial Sequence: Synthetic primer
tttttcccatttccaactct

SEQ ID NO: 261 - DNA, 20 bp, Artificial Sequence
  Description of Artificial Sequence: Synthetic primer
aaaagatgagacaggcaggt

SEQ ID NO: 262 - DNA, 20 bp, Artificial Sequence
  Description of Artificial Sequence: Synthetic primer
acccctgtgaatctcaaaat

SEQ ID NO: 263 - DNA, 21 bp, Artificial Sequence
  Description of Artificial Sequence: Synthetic primer
gcacttgcttctattgtttgt

SEQ ID NO: 264 - DNA, 20 bp, Artificial Sequence
  Description of Artificial Sequence: Synthetic primer
cccttcctctcttccattct

SEQ ID NO: 265 - DNA, 13 bp, Artificial Sequence
  Description of Artificial Sequence: Synthetic primer
agcactgcaggta

SEQ ID NO: 266 - DNA, 21 bp, Artificial Sequence
  Description of Artificial Sequence: Synthetic primer
acagataccaaagaactgcaa

SEQ ID NO: 267 - DNA, 20 bp, Artificial Sequence
  Description of Artificial Sequence: Synthetic primer
tggacacctttcaacttaga

SEQ ID NO: 268 - DNA, 22 bp, Artificial Sequence
  Description of Artificial Sequence: Synthetic primer
gaacagtaatgttgaacttttt

SEQ ID NO: 269 - DNA, 21 bp, Artificial Sequence
  Description of Artificial Sequence: Synthetic primer
tcttgcaaaaagcttagcaca

SEQ ID NO: 270 - DNA, 21 bp, Artificial Sequence
  Description of Artificial Sequence: Synthetic primer
aaaaagatctcaaagggtcca

SEQ ID NO: 271 - DNA, 20 bp, Artificial Sequence
  Description of Artificial Sequence: Synthetic primer
gcttttgctgaacatcaagt

SEQ ID NO: 272 - DNA, 19 bp, Artificial Sequence
  Description of Artificial Sequence: Synthetic primer
ccttccagcagcatagtct

SEQ ID NO: 273 - DNA, 18 bp, Artificial Sequence
  Description of Artificial Sequence: Synthetic primer
aaatccaggatgtgcagt

SEQ ID NO: 274 - DNA, 19 bp, Artificial Sequence
  Description of Artificial Sequence: Synthetic primer
atgatgaggtcagtggtgt

SEQ ID NO: 275 - DNA, 22 bp, Artificial Sequence
  Description of Artificial Sequence: Synthetic primer
catcacagatcatagtaaatgg

SEQ ID NO: 276 - DNA, 21 bp, Artificial Sequence
  Description of Artificial Sequence: Synthetic primer
aattattattttgcaggcaat

SEQ ID NO: 277 - DNA, 20 bp, Artificial Sequence
  Description of Artificial Sequence: Synthetic primer
catgaggcaaacacctttcc

SEQ ID NO: 278 - DNA, 22 bp, Artificial Sequence
  Description of Artificial Sequence: Synthetic primer
gctggactcaggataaagaaca

SEQ ID NO: 279 - DNA, 20 bp, Artificial Sequence
  Description of Artificial Sequence: Synthetic primer
tggaagcctgagctgactaa

SEQ ID NO: 280 - DNA, 20 bp, Artificial Sequence
  Description of Artificial Sequence: Synthetic primer
ccttcttttcccccagaatc

SEQ ID NO: 281 - DNA, 21 bp, Artificial Sequence
  Description of Artificial Sequence: Synthetic primer
taggagaacagaagatcagag

SEQ ID NO: 282 - DNA, 22 bp, Artificial Sequence
  Description of Artificial Sequence: Synthetic primer
aaagactattgctaaatgcttg

SEQ ID NO: 283 - DNA, 20 bp, Artificial Sequence
  Description of Artificial Sequence: Synthetic primer
taagcgtagggctgtgtgtg

SEQ ID NO: 284 - DNA, 21 bp, Artificial Sequence
  Description of Artificial Sequence: Synthetic primer
ggacggatagactccagaagg

SEQ ID NO: 285 - DNA, 23 bp, Artificial Sequence
  Description of Artificial Sequence: Synthetic primer
gaatgaccttggcacttttatca

SEQ ID NO: 286 - DNA, 27 bp, Artificial Sequence
  Description of Artificial Sequence: Synthetic primer
aaggatagagatatacagatgaatgga

SEQ ID NO: 287 - DNA, 18 bp, Artificial Sequence
  Description of Artificial Sequence: Synthetic primer
catgcaccgcgcaaatac

SEQ ID NO: 288 - DNA, 19 bp, Artificial Sequence
  Description of Artificial Sequence: Synthetic primer
atgcctcacccacaaacac

SEQ ID NO: 289 - DNA, 20 bp, Artificial Sequence
  Description of Artificial Sequence: Synthetic primer
tccaagcccttctcactcac

SEQ ID NO: 290 - DNA, 20 bp, Artificial Sequence
  Description of Artificial Sequence: Synthetic primer
ctgggacggtgacattttct

SEQ ID NO: 291 - DNA, 21 bp, Artificial Sequence
  Description of Artificial Sequence: Synthetic primer
cccaggaagagtggaaagatt

SEQ ID NO: 292 - DNA, 21 bp, Artificial Sequence
  Description of Artificial Sequence: Synthetic primer
ttagcttgcatgtacctgtgt

SEQ ID NO: 293 - DNA, 20 bp, Artificial Sequence
  Description of Artificial Sequence: Synthetic primer
agctagatggggtgaatttt

SEQ ID NO: 294 - DNA, 18 bp, Artificial Sequence
  Description of Artificial Sequence: Synthetic primer
tgggctgaggggagattc

SEQ ID NO: 295 - DNA, 22 bp, Artificial Sequence
  Description of Artificial Sequence: Synthetic primer
atcaagctaattaatgttatct

SEQ ID NO: 296 - DNA, 20 bp, Artificial Sequence
  Description of Artificial Sequence: Synthetic primer
aatgaataaggtcctcagag

SEQ ID NO: 297 - DNA, 21 bp, Artificial Sequence
  Description of Artificial Sequence: Synthetic primer
tttaatctgatcattgcccta

SEQ ID NO: 298 - DNA, 18 bp, Artificial Sequence
  Description of Artificial Sequence: Synthetic primer
agctgtgggtgaccttga

SEQ ID NO: 299 - DNA, 20 bp, Artificial Sequence
  Description of Artificial Sequence: Synthetic primer
tgtcccaccattgtgtatta

SEQ ID NO: 300 - DNA, 20 bp, Artificial Sequence
  Description of Artificial Sequence: Synthetic primer
tcagacttgaagtccaggat

SEQ ID NO: 301 - DNA, 20 bp, Artificial Sequence
  Description of Artificial Sequence: Synthetic primer
gcttcaggggtgttagtttt

SEQ ID NO: 302 - DNA, 20 bp, Artificial Sequence
  Description of Artificial Sequence: Synthetic primer
ctttgtgaaaagtcgtccag

SEQ ID NO: 303 - DNA, 18 bp, Artificial Sequence
  Description of Artificial Sequence: Synthetic primer
ccatcatggaaagcatgg

SEQ ID NO: 304 - DNA, 20 bp, Artificial Sequence
  Description of Artificial Sequence: Synthetic primer
tcatctccatgactgcacta

SEQ ID NO: 305 - DNA, 20 bp, Artificial Sequence
  Description of Artificial Sequence: Synthetic primer
gagatgacggagtagctcat

SEQ ID NO: 306 - DNA, 18 bp, Artificial Sequence
  Description of Artificial Sequence: Synthetic primer
cccagctgcactgtctac

SEQ ID NO: 307 - DNA, 20 bp, Artificial Sequence
  Description of Artificial Sequence: Synthetic primer
tcttgttccaatcacaggac

SEQ ID NO: 308 - DNA, 20 bp, Artificial Sequence
  Description of Artificial Sequence: Synthetic primer
atgctgttagctgaagctct

SEQ ID NO: 309 - DNA, 20 bp, Artificial Sequence
  Description of Artificial Sequence: Synthetic primer
tgaaagctcctaaagcagag

SEQ ID NO: 310 - DNA, 20 bp, Artificial Sequence
  Description of Artificial Sequence: Synthetic primer
ttgaagagatgtgctatcat

SEQ ID NO: 311 - DNA, 54 bp, Artificial Sequence
  Description of Artificial Sequence: Synthetic primer
gccgcctgcagcccgcgccccccgtgcccccgccccgccgccggcccgggcgcc

SEQ ID NO: 312 - DNA, 601 bp, Homo sapiens
catagtgacaggtatatgcccaactaactgtggaaaacagttctttctttcaaccttactcatcaccctcacggtctgtttatgaggctctcctccaccagccagaaaggatgacgtgccatacctgcaaaacttatacagcatcaacagaatgaatctttccaacaagccgaaacattgagtattgtggcacagaatatgccccacccattactcaatctagatatccttttattccaccgtctcatgattttctttttcctggaaaacaaaagtatttctttcatagcccagctagcaygataaatcagcgagtcagaattctagctttgttgtaaggttttgcgaatatctgatcctcttattttgtacttttctatttcctaggcaaatctgagtatttcacccagttttccttaactaggcattgaaaactcagtttttttcttacaaaccttcatgtcttcctgctcatttgcacagtcttatcttgcacctcctataaaatggagaaacttgacattaaaacgtaatttttattacattttgagggattcccagagaatttttccccaatctccttaggtagggacttctttac

SEQ ID NO: 313 - DNA, 601 bp, Homo sapiens
gtgggaactatagtaaagaagtccctacctaaggagattggggaaaaattctctgggaatccctcaaaatgtaataaaaattacgttttaatgtcaagtttctccattttataggaggtgcaagataagactgtgcaaatgagcaggaagacatgaaggtttgtaagaaaaaaactgagttttcaatgcctagttaaggaaaactgggtgaaatactcagatttgcctaggaaatagaaaagtacaaaataagaggatcagatattcgcaaaaccttacaacaaagctagaattctgactygctgatttatcgtgctagctgggctatgaaagaaatacttttgttttccaggaaaaagaaaatcatgagacggtggaataaaaggatatctagattgagtaatgggtggggcatattctgtgccacaatactcaatgtttcggcttgttggaaagattcattctgttgatgctgtataagttttgcaggtatggcacgtcatcctttctggctggtggaggagagcctcataaacagaccgtgagggtgatgagtaaggttgaaagaaagaactgttttccacagttagttgggcatata

SEQ ID NO: 314 - DNA, 650 bp, Homo sapiens
tttattggtcctgactggtacaaatactgataaaaaggattttaagatcatattcatacttttggggaatgagagccacaattaattaacaatgtctgccatgagattggatgcaagagtatggcactcatactattcctacttctgtctaattacactatttgtttctgtgtgcaaaaatctttggtaggtggtggatgtgcccaagacacagggaagaaaaagaagtaaacagggaagtacaacacagactctgaaatggggcatcatggaagacggagctttgtcgtcttggtctttgctgtatattcacttcctacaacagtgctaaataccttgtggatgcttaaatatattaaatgaatgcataaatgaaaagagtaaataaagagtgtatatgaaagtatgtagataaaattcttcactaagccttggggatccagctgcttmaggactaagaccgtatctagctccttttagtatttccacagcatgccatggagatacatgtttctgattatatatgatacatggaaattatatgttgttgaatgagtgattgagtaaatgtgtactagggcagctaatcataaatatttctactattgctaaaatgactggatttatccattccttctgagagtttatac

SEQ ID NO: 315 - DNA, 626 bp, Homo sapiens
ctgcttaaggactaagaccrtatctagctccttttagtatttccacagcatgccatggagatacatgtttctgattatatatgatacatggaaattatatgttgttgaatgagtgattgagtaaatgtgtactagggcagctaatcataaatatttctactattgctaaaatgactggatttatccattccttctgagagtttatactgattgcttatattgtatcaaataccgtaactgagggcaatgtttactcaaactaatagcaccattcaaatttatgcaaacaataacactatatctttaaaatgttttcactaaaagctgcataaagagtgtattcaacaacaatagaataattttacaatcttttttcttgcttaatggccatttgtgccttctgacatgctgctagccattcaaaggtcacactaccttgaagttgaagatcaagacaaatgattagactcataaaagacaaatcacgtctttctggacaggtgattattaataattaattagcatttaaacatgtattatttaagttctttttaagttataaagtctttgatttgctaaacagtttaaataatgaataaaacataaaataataatagttaccattt

SEQ ID NO: 316 - DNA, 1113 bp, Homo sapiens
caagagctgcatctcactccaatttttcttctccctataaccttatctagattcccagttgagggaaccgatgacctaattcctctcagtttaaatgcaacacaggagcaaattccaaatatctatgctggtcttgctgggattgcagaaccccagggtggttatcctcctccagaggtaatcctgtgatcagcactaacrccacataccagccctttcatcagcttgttggagaagcatctttacttcccaccaagcagtgacctagataccatctcacaccagttagaatcaggatcattaaaaagtcaagaaaaaacagatgctgaagaggatgtggagaaataggaatgcttttacactgttagtgggaatgtaaattagttcaaccattgtcaaagacagtgtggcgatccctcacagatctagaaccagaaataccatttgacccagcaatcccattactgggtctatacccaaaggattataaattactctactataaagacacatgcacacatatgtttattgcagcaccattcacaatagcaaagaattgcaaccaaccctaatgcccatcaatgacagactggataaagaaaatctggcacatatacaccatggaatactacgcagccataaaaaaggatgagtttatgtcctttacagggacatggatgaagctggaaaccatcattctcagcaaactaacacaggaacagaaaaccaaacacatgttctcactcacaagtgggagttgaacaatgagaacacatggacacagggaggggaacatcacacaccactgcttgtcagggggtggggggctaggggaaggatagcattaggagaaatacctaatgtagatgaagggttgatgggtgcagcaaaccaccatggcatgtgtatacctgtgtaacaaacctccatgttctgcacgtgtatcccagaacttaaagtacaatacaaaaaaaaaaaaaagtgtaatccagtttacattttcaaggtcaaagtgggtacaatgctatctatcttgggctaagaagagaaaaggaaaaattcttgctttaaatcttagaagtctggtttttttccctgttttgtaccccatcc

SEQ ID NO: 317 - DNA, 1113 bp, Homo sapiens
ttcccagttgagggaaccgatgacctaattcctctcagtttaaatgcaacacaggagcaaattccaaatatctatgctggtcttgctgggattgcagaaccccagggtggttatcctcctccagaggtaatcctgtgatcagcactaacgccacataccagccctttcatcagcttgttggagaagcatctttacttcccrccaagcagtgacctagataccatctcacaccagttagaatcaggatcattaaaaagtcaagaaaaaacagatgctgaagaggatgtggagaaataggaatgcttttacactgttagtgggaatgtaaattagttcaaccattgtcaaagacagtgtggcgatccctcacagatctagaaccagaaataccatttgacccagcaatcccattactgggtctatacccaaaggattataaattactctactataaagacacatgcacacatatgtttattgcagcaccattcacaatagcaaagaattgcaaccaaccctaatgcccatcaatgacagactggataaagaaaatctggcacatatacaccatggaatactacgcagccataaaaaaggatgagtttatgtcctttacagggacatggatgaagctggaaaccatcattctcagcaaactaacacaggaacagaaaaccaaacacatgttctcactcacaagtgggagttgaacaatgagaacacatggacacagggaggggaacatcacacaccactgcttgtcagggggtggggggctaggggaaggatagcattaggagaaatacctaatgtagatgaagggttgatgggtgcagcaaaccaccatggcatgtgtatacctgtgtaacaaacctccatgttctgcacgtgtatcccagaacttaaagtacaatacaaaaaaaaaaaaaagtgtaatccagtttacattttcaaggtcaaagtgggtacaatgctatctatcttgggctaagaagagaaaaggaaaaattcttgctttaaatcttagaagtctggtttttttccctgttttgtaccccatcctcttggtctctctagatatatttaagactcacataggacttgtcttttcta

SEQ ID NO: 318 - DNA, 1001 bp, Homo sapiens
tcatcaactaaatagttgatgaggggaaattgttctgtatatgttcatacttcagctaatcaattaaaaatgatgaaataataagattaccattttgcaaacccctaatgcaatgttggatccaggcaatgatcatcaatggccactaaaatcacacaaaaggagataaccagaatatgtgctttgtgatggaagcattaaatacaactaatgagatattgtttataagaaagaaaggaagcaagaaagcaatcacaccaagctctgtatctagctaccacatttaaggaaaaaaagagacagaagagcatgttaaatgttaccaagaagatacagtcagtcggaaaaaatacagacaagaaaatacagagcaaaacaacccagcttcttcagcaaatcaatataaaaaaattttaagaaagagttaaagtataaactgagagacttcagaaacatattatccaagtataatccatgaatcttgtttaaatatagatcaartaaaccactataccaaaaacatcaaaagacaactgggtaaattttttaaatgactagctatttgatgttaaggaagtaatgttactctcttatatacaatttgaaataatctagcgaggagcagcaaatgtgcggctatgaggaagaaacacaattggccattcttgaatcattagctggatggtggctatatgggggtagattttactactctctaattttacatatatttaaaatgttccataataaattgttgagttatcaaaagaaatatttctatataatagctaaaattatttataaaagttagtggtctcataactttatttatttatttacttattttgagaccgagtctccctctgttatgcaggctggagtgcagtggctccatctcggctcactgcaaacttcacctcctggattgaagcgattctcctgcctcagcccccccgagtagctgggattacaggcttgcacccccacgcccagctaatttt

SEQ ID NO: 319 - DNA, 601 bp, Homo sapiens
agctaccacatttaaggaaaaaaagagacagaagagcatgttaaatgttaccaagaagatacagtcagtcggaaaaaatacagacaagaaaatacagagcaaaacaacccagcttcttcagcaaatcaatataaaaaaattttaagaaagagttaaagtataaactgagagacttcagaaacatattatccaagtataatccatgaatcttgtttaaatatagatcaaataaaccactataccaaaaacatcaaaagacaactgggtaaattttttaaatgactagctatttgatgttaargaagtaatgttactctcttatatacaatttgaaataatctagcgaggagcagcaaatgtgcggctatgaggaagaaacacaattggccattcttgaatcattagctggatggtggctatatgggggtagattttactactctctaattttacatatatttaaaatgttccataataaattgttgagttatcaaaagaaatatttctatataatagctaaaattatttataaaagttagtggtctcataactttatttatttatttacttattttgagaccgagtctccctctgttatgca

SEQ ID NO: 320 - DNA, 601 bp, Homo sapiens
ccaactgatctaattagataaacttagtcaatatatttgaatcccacattccagcagctattttctccatttgcttttattgctgtttgtggtgagtttgatatataattttaaggtgttaacatccctaacttatgtatgggtacagctcataaatacgaacctgtgtcatgcaactcatatatgactgtgttcaaaataatgtgtattagactgtaaaacgattttaatattttaaataactttcctgcatttgtcggtttcagcaggaaagttatttttaataacttccctgtatttsttggtttcagtattaattaatctcattaatgctaaactttgtgatcctaggttaaaaaacatattcaagatagcttcagaatgtttggtatacaaataggtctggctaaatataagtgttagctttctcaagcatctaaatgctggcgggcttttaaaaaaccagggctttaaggagaaaacacctgctctgtggttttgtagcagatatgaagtattcaaatttcttaataaatagaaaaagaaatatataacagaaacaggttgcacttgtctttctcattaagcaggtggttagtac

SEQ ID NO: 321 - DNA, 501 bp, Homo sapiens
agctcataaatacgaacctgtgtcatgcaactcatatatgactgtgttcaaaataatgtgtattagactgtaaaacgattttaatattttaaataactttcctgcatttgtcggtttcagcaggaaagttatttttaataacttccctgtatttgttggtttcagtattaattaatctcattaatgctaaactttgtgatcctaggttaaaaaacatattcaagatagcttcagaatgtttggtatacaartaggtctggctaaatataagtgttagctttctcaagcatctaaatgctggcgggcttttaaaaaaccagggctttaaggagaaaacacctgctctgtggttttgtagcagatatgaagtattcaaatttcttaataaatagaaaaagaaatatataacagaaacaggttgcacttgtctttctcattaagcaggtggttagtaccattatttgcattctcatagccttaatatacattttccttctctag

SEQ ID NO: 322 - DNA, 601 bp, Homo sapiens
ttttgagtttctactttagtgtcttagtgctttctcgatatgggagaattcatgtcctccattcagaagtatgcactaagtaagaggtatcatgtctggttcttgattaggtactaatcttgaaatattatcctacaataggttagagcacgtatatctcctgataatatattgaatatgatagatttaaataattggttaactaaatactaaagcaaattgctgcacgtatcatttattattcattgtgtagaaagtgcctgactcagtgtttggaaattgtctgacttttcctcatatrtagtgtggtttcatgttattgtatataagacctgacatgaactctgtttacaataatctcccagtgccataaagaccataataaataatataaccaattggtttctttatgctgtcatttattagggcatatggcattagtggaggattaccttgtattacccatagtgcttagagtatgaatcacacatgcaccttgaaggaaaagaggtgcaatgtaataagaaaccagatattgaaaatgcaagttttgttatgttattctgggtatgttaacctttattcctgccctccatatgca

SEQ ID NO: 323 - DNA, 501 bp, Homo sapiens
aagaggtatcatgtctggttcttgattaggtactaatcttgaaatactatcctacagtaggttagagcacgtatatctcctgataatatattgaatatgatagatttaaataattggttaactaaatactaaagcaaattgctgcacgtatcatttattattcattgtgtagaaagtgcctgactcagtgtttggaaattgtctgacttttcctcatatatagtgtggtttcatgttattgtatataagamctgacatgaaccctgtttacaataatctcccagtgccataaagaccataataaataatataaccaattggtttctttatgctgtcatttattagggcatatggcattagtggaggattaccttgtattacccatagtgcttagagtatgaatcacacatgcaccttgaaggaaaagaggtgcaatgtaataagaaaccagatattgaaaatgcaagttttgttatgttattctgggtatgttaaccttta

SEQ ID NO: 324 - DNA, 854 bp, Homo sapiens
tttcagcactgagagccagagtggaattgtctccttcattgccactgccttcacgttttgtgtgtcgtatctgttttgtgatcactgagacccaagaacccccgacttgccgacatactatgtggccccgagagaggacttgagctctctgggtttcatcattaccatcaattaaataaacaggacagtagcttcttccttggattgttaatttaaggctctggataatacatgtaaccgccttatgatagagcagaattgtaagtaggctcatggtagaatcgttcaatgacatttccctttcctttgggagaaacagaaattcacaggtctaattcttttcctattaatagttcctgrccattattccagaactgtcctaaaggaattctttctccttaaggacaccacctcccaggagggtatttaaagatttgcacaggccgggcacggtggctcatgcttgtaatcccagcagtttgggaggccaaggcgggtggatcacttgtgctcaggggttcaagaccggcctggccaacatggtgaaaccctatctctactaaaaacacaaaagttagctgggcctggctatgcatgcctgtaattccagctactcgggaggctgaggctggagaatagcttgaaccagggaggtggagataacagtgagctgagatgccactatgacactccagcctgggtgacagagcaagactctctctcaaaaaaaaaaaaagatttttatagtccagtattcaacgttcatagtacacctttcttatcctagtaaatcttcttttatcaaggtatatgatcccatatagtagttaactcttactcttactttatgacaa

SEQ ID NO: 325 - DNA, 501 bp, Homo sapiens
aaatacttactattaaatatgagaaactgtggtgtttatcggtaagatccacgaaggaagaagttttaaagaaaaatactttaaccgtggaaaaaaaaaactttaatgtctattatcgaataggggccgtaattacttttgcaaaataaaaaaacaaacaagactagctatagtgtaaatgtaatctgtatgctttttaatgaaacaattaagtaggttgcccatttacaattagcctgattttctcctgygtggtattatgtgtacttaacaacaggacccagtggaaattcactcatttaacaaagtctgcctacatggtttcaaatatgggcctaacttgaaaattcagtcataattaaatctaaggactaaaacaaatctgtataaaaagattctgctaaataagggaaaattcaagtctagggctacattctgaaagatattgaagtagaacctctgcagcaagactaggcttggaaagtgcggggaggagggaaa

SEQ ID NO: 326 - DNA, 601 bp, Homo sapiens
ccacatcagaaacatgaggaaattctacatggtaaaaacagcaacaaccaaaaaatacttaaagtcaacaaaccaggaaaagacatctctgaatataggaatgccaaacctttaacacaataaaacacagattatatttcagaaggctatattatatgtgtataccaacatcaatatgtccagagtagctgcacagagttccatattttagtctttataagttcccctcctcaccctactcagtaggcactttgtgtctagaaacttctgtgtcaacagttttccctctctctggaattcmtcaggacagaagtgattggtgtggtggaagagggttgtgctaagagtgaagttatatgaaagtaggatggaggttagcaagtagttaaagtccagaaaggcaataaggtgttaaggaagaacttttccattttacaggtctgagcaagcaggaaatcaactctacaaactttgaaacttggtaaatatgaaaacattctcaataccatttgtcatttaataaatacaaattatactattttactgcttgcatctagaagtttgtcaaagatctcgtcttaattattcattgtgtcggcga

SEQ ID NO: 327 - DNA, 601 bp, Homo sapiens
gacgagatctttgacaaacttctagatgcaagcagtaaaatagtataatttgtatttattaaatgacaaatggtattgagaatgttttcatatttaccaagtttcaaagtttgtagagttgatttcctgcttgctcagacctgtaaaatggaaaagttcttccttaacaccttattgcctttctggactttaactacttgctaacctccatcctactttcatataacttcactcttagcacaaccctcttccaccacaccaatcacttctgtcctgatgaattccagagagagggaaaacygttgacacagaagtttctagacacaaagtgcctactgagtagggtgaggaggggaacttataaagactaaaatatggaactctgtgcagctactctggacatattgatgttggtatacacatataatatagccttctgaaatataatctgtgttttattgtgttaaaggtttggcattcctatattcagagatgtcttttcctggtttgttgactttaagtattttttggttgttgctgtttttaccatgtagaatttcctcatgtttctgatgtggaaagtataagaatatcagccaga

SEQ ID NO: 328 - DNA, 811 bp, Homo sapiens
taaataatctctaattagtataatgggtgttcttagtgcagtgggtacttttaaagtgctttgtggcttttgatgaaaattgtcttagtatttaaaactttttcttacccaattttttgttcccatcgaattagcaatgctgtaaagaaaggcatcttattccattttttgttgctataaaggaatacttgaggctgggtaatttataaagatgaaaagtttatttggctcgcaattctggatggctggaaggttaagtactgggccacagcatctggtgggggcctcgagctgcttctagtcataatggaaggtgaagggtgtaaagatcatgtgacaagggaggaaagaagagaaggaaggaggtgctggttctttctatcaaccaattcgcaagagaactaatagagaaagaactcacttagccctgtgggaacacattaatctattcataagggatctggctgtatgatacaaacacctcccattaggccccacctccaaattgtatcccattggggatcaaatttcaaaaagagatttggaaggaacaaacaaaccatatctaagccatagtaaaaggaatggcttttcaaaggtaaaatttactragtgtattaatattttaccaatttccagccaggagagtatgaatgttgcattattacattgctttgaaacaaagcattagtcttaattcagaagtttaaattcagatgttaacgttgcatatttaataatgcacaaccagtactaaaatcctcattgaaatgacaaataattttatttcgaatcccttatagaggttcac

SEQ ID NO: 329 - DNA, 811 bp, Homo sapiens
tgtcttagtatttaaaactttttcttacccaattttttgttcccatcgaattagcaatgctgtaaagaaaggcatcttattccattttttgttgctataaaggaatacttgaggctgggtaatttataaagatgaaaagtttatttggctcgcaattctggatggctggaaggttaagtactgggccacagcatctggtgggggcctcgagctgcttctagtcataatggaaggtgaagggtgtaaagatcatgtgacaagggaggaaagaagagaaggaaggaggtgctggttctttctatcaaccaattcgcaagagaactaatagagaaagaactcacttagccctgtgggaacacattaatctattcataagggatctggctgtatgatacaaacacctcccattaggccccacctccaaattgtatcccattggggatcaaatttcaaaaagagatttggaaggaacaaacaaaccatatctaagccatagtaaaaggaatggcttttcaaaggtaaaatttactaagtgtattaatattttaccaatttccagccaggagagtatgaatgttgcattattacattgctttgaaacaaagcattaktcttaattcagaagtttaaattcagatgttaacgttgcatatttaataatgcacaaccagtactaaaatcctcattgaaatgacaaataattttatttcgaatcccttatagaggttcacaatgttttaacaatgtagttttgactaaatagaagtagtcaaaacctgtcagattggaaatagtatttataaaacataaa

SEQ ID NO: 330 - DNA, 601 bp, Homo sapiens
gctcatcaattttgacttaagaaaattctagcaacatttatagattttgccaaaattcagcttcttcccaaatcaatctataagaaggctcttccttaaacataatttttatatctatgaactgcactagcatttactatatatttttatcactctcaccattactggataataaataaaagctcattaaaagagttaacaaaacatatttattttaggcatcctgaaaaaaagattcaattttattatcatttctacaataagtattgaagaaaggagaatttaaattacttcatatacstgataaaggaaaacatatgcaaggcaaataaacatcttagatcatgacatataaaataatagattattactaaagattaaaatactttcttaagaattaaagcaattctaaaagcaatagtaaataacattctttctagtgatcagacactggatactatgtttgagatagacagtgaattgggaatgttgttttacagaagctcctaccttgcaaggacaggcaagtttaaatgtcagctagaaaactatcttgagttttcagtaatgtaagattttcctattcaatttcacactttaa

SEQ ID NO: 331 - DNA, 601 bp, Homo sapiens
agaaaattctagcaacatttatagattttgccaaaattcagcttcttcccaaatcaatctataagaaggctcttccttaaacataatttttatatctatgaactgcactagcatttactatatatttttatcactctcaccattactggataataaataaaagctcattaaaagagttaacaaaacatatttattttaggcatcctgaaaaaaagattcaattttattatcatttctacaataagtattgaagaaaggagaatttaaattacttcatatacctgataaaggaaaacatatrcaaggcaaataaacatcttagatcatgacatataaaataatagattattactaaagattaaaatactttcttaagaattaaagcaattctaaaagcaatagtaaataacattctttctagtgatcagacactggatactatgtttgagatagacagtgaattgggaatgttgttttacagaagctcctaccttgcaaggacaggcaagtttaaatgtcagctagaaaactatcttgagttttcagtaatgtaagattttcctattcaatttcacactttaaattttatatatatataaaa

SEQ ID NO: 332 - DNA, 1110 bp, Homo sapiens
tgtagaagttcttatcacttcctggccttttggctaagatcaagtgtgaaatgtagaagttcctctaagctttacttccctcaaaaactagttttatcttgtcagcaggattcacttaaaaagacaaattcagattatgaatttttttcttttttacagggtctgctctgttgcccaggctggagtgcagaggcacaatctcggctcactgcagcctccgcctcctgggttcaagcaattctcttgcctcagcctcccgagtaactgggattacaggcatgtgccaccacccagctaatttttgtatttttagtagagatggggtttcaccacattggtcaggctggtctcgaactgctggcctcaagtgatccacttgcctcggcctcccaaagtgcagagattacaggtgtgagccaccgtgcccagcctcataaccgtttcaactactttttcacttgacaagcagatgtgaagttaacaaagtcacccatatttgaaataaagatagtatattcctggggyaggcagaggcagttgaggatcatgaaataactatgttggcatagttatttaggtgttgatactgttattatgccattgaaagttaaacagagaaccctctgggtacatgttttataccaatgcacactatcttattagtccctctcataatgtgcagtcatcattactgttacgggttgaggtgtccccatcctctatgggacacctctatgttgaagtctcagattccctagaatctcagaatgtgaccttgtttggaaacagatttgctacagacgcaattagttgagatgcgcttatatgggtaggtcctaattcagtgactggtgtccttaaaaaaatggaaatgtacacacggtggtagacatgcatagagggaagagagatggagaaaatggtcacctacaagccaaagacaggggtctggagcagatccttccctcacagccctcagaaggaaccaatcttgccaataccttgattttggacttccacctccagaactataacacatttctgttcttcaagcaatttgtagccatttgttacagctaatacaatcacacatagaaatgacttgtaaat

SEQ ID NO: 333 - DNA, 691 bp, Homo sapiens
taaaacatgtacccagagggttctctgtttaactttcaatggcataataacagtatcaacacctaaataactatgccaacatagttatttcatgatcctcaactgcctctgcctaccccaggaatatactatctttatttcaaatatgggtgactttgttaacttcacatctgcttgtcaagtgaaaaagtagttgaaacrgttatgaggctgggcacggtggctcacacctgtaatctctgcactttgggaggccgaggcaagtggatcacttgaggccagcagttcgagaccagcctgaccaatgtggtgaaaccccatctctactaaaaatacaaaaattagctgggtggtggcacatgcctgtaatcccagttactcgggaggctgaggcaagagaattgcttgaacccaggaggcggaggctgcagtgagccgagattgtgcctctgcactccagcctgggcaacagagcagaccctgtaaaaaagaaaaaaattcataatctgaatttgtctttttaagtgaatcctgctgacaagataaaactagtttttgagggaagtaaagcttagaggaacttctacatttcacacttgatcttagccaaaaggccaggaagtgataagaacttctacattttaagttattcacaagataactattaatgaacctgaaatagtttgtaaag

SEQ ID NO: 334 - DNA, 640 bp, Homo sapiens
aaacctttttcctgttttactattactaaaggtggcacaacagcaacctcaacaactttgcaccatgccaacactgatgtttacacccagcacagcatttttggtctctatttttattctcctctgaatgtaatgaggattcctagatggctagccaattcgaatatttaaggcaactgaaagttagaatgtttctgaaacatagtgttgttgccagagagtacgaaagttttcaagaatatcgggcaattctgaaagtacaaagaagccagattaaatgaaataacactggcgaagttttagcaaggtgactctcatataatgatcattatcattaccacagttaaaagaaaagagttgtttatgaaaggccatgtgtctgcaatgaaactcaaaagagaaaagttaacaggtgcaaraggtagttttattataaaaggagggtaggcaacaagaatatgtttaatttttcttccttttcatgagtaaggacaagagtttcatatatgtgaatatttttatttaattttaagtagaaatctgtttttaaaatatgggtatatgcttatttgtgtaagtgtaagaaacagaagtaagtacagcaaaccagaaataggccaaacactcctgagcataattt

SEQ ID NO: 335 - DNA, 919 bp, Homo sapiens
tacacccagcacagcatttttggtctctatttttattctcctctgaatgtaatgaggattcctagatggctagccaattcgaatatttaaggcaactgaaagttagaatgtttctgaaacatagtgttgttgccagagagtacgaaagttttcaagaatatcgggcaattctgaaagtacaaagaagccagattaaatgaaataacactggcgaagttttagcaaggtgactctcatataatgatcattatcattaccacagttaaaagaaaagagttgtttatgaaaggccatgtgtctgcaatgaaactcaaaagagaaaagttaacaggtgcaaaaggtagttttattataaaaggagggtaggcaacaagaatatgtttaatttttcttccttttcatgagtaaggacaagagtktcatatatgtgaatatttttatttaattttaagtagaaatctgtttttaaaatatgggtatatgcttatttgtgtaagtgtaagaaacagaagtaagtacagcaaaccagaaataggccaaacactcctgagcataattttacttggtagattattcctgaaacttaaggaatcatctttgaactcttttcctcacttgacttccaggattcaccatgcacttgtgattttcctttcatttcactctccgttcctcctcagtctttttttctcccccaggtcttttttgttcatcttaaactctaaattttagaatatcccaggggtctgccttcggccttctcttttatatctacactggcctcatacataatcttaaccaagtcattattttaaatacctacaatatactgaaaacttctaaatttgtattttaattcttgacttcttccatacagtctagatttgtatgtccataggctgacatcattggctgatac

SEQ ID NO: 336 - DNA, 1001 bp, Homo sapiens
ttactaaatattctccaacaaatatatacttagtatatactattagtgatgcatgctttcaaatatttggactatatcaatgaatgaaacaaaaaattatttgcccttaaggagcttagattctaacagatggattcagatgatttttatgccttatttcgtaggtttaaaagagcaatggggaaaagggaagaagagagggattgaaaatattgagaaggttgggagacttagcaattttaagtaaggtagtgagggtaggttttattggcaaagtgatttttcagcagagactgggaaagatgaacgtggtatcctggaggaaagcctcccaggcagagttaagctgctaacaaaagtgcccttaggctggagtgggcttgtttgattaaggaacaaagaggtcagcatggttgcactagagagaaaaaatcagatggcgtaaggagatgaaatcagaaagatacgaggctaggcaaaggggtactctatgtaatgaayatgacctggcagtactgacatctcctgagggactgttagaagtgcagactcttgtatcttttctcaagtctatgaaatctagacttcattttaacaagatgacccgatatttacatacacattaaagttccagaagcactgatataacacattgtaagatcgcacaggacttcaattctttttctggtttttagaggcagtcctttggggtgttttgtgtagagtataatgacctgaaatatctaggatcactctagctactatcttgaggaaagagtgcaataaggcggaacagttcagaggcaatggtggtcttctaaatgaaagacacacagcactcaaaccaggcagttgaggagggatgggaagaagttgtcaaattctagacatattttaaaggtagtgtccagagaatttccttagatgcgtaggaacatggaggataggacatagggtggaaataaacgaaataaagaaactgaagctgattctgacatttt

SEQ ID NO: 337 - DNA, 1576 bp, Homo sapiens
ataccttttaagtgacatcctagtgaatctccatttgtcacgagacctcaagctttccagttctggcacaaagtgattactcataccatcacttcaaaatgatgattatcttcatttattttagttatattgaacaaaatatacatttaaaaaatctaattactaaatattctccaacaaatatatacttagtatatactattagtgatgcatgctttcaaatatttggactatatcaatgaatgaaacaaaaaattatttgcccttaaggagcttagattctaacagatggattcagatgatttttatgccttatttcgtaggtttaaaagagcaatggggaaaagggaagaagagagggattgaaaatattgagaaggttgggagacttagcaattttaagtaaggtagtgagggtaggttttattggcaaagtgatttttcagcagagactgggaaagatgaacgtggtatcctggaggaaagcctcccaggcagagttaagctgctaacaaaagtgcccttaggctggagtgggcttgtttgattaaggaacaaagaggtcagcatggttgcactagagagaaaaaatcagatggcgtaaggagatgaaatcagaaagatacgaggctaggcaaaggggtactctatgtaatgaacatgacctggcagtactgacatctcctgagggactgttagaagtgcagactcttgtatcttttctcaartctatgaaatctagacttcattttaacaagatgacccgatatttacatacacattaaagttccagaagcactgatataacacattgtaagatcgcacaggacttcaattctttttctggtttttagaggcagtcctttggggtgttttgtgtagagtataatgacctgaaatatctaggatcactctagctactatcttgaggaaagagtgcaataaggcggaacagttcagaggcaatggtggtcttctaaatgaaagacacacagcactcaaaccaggcagttgaggagggatgggaagaagttgtcaaattctagacatattttaaaggtagtgtccagagaatttccttagatgcgtaggaacatggaggataggacatagggtggaaataaacgaaataaagaaactgaagctgattctgacattttagacctaaaatctcaactaaaagttgccaagatgggaaaaactaggtgcatcttgtttggtgagtggaaatcagccttgtgaattaagacttaaactgatgtctttaatcccgtagaaataccatgaaggcagtagaagatggctaaagagaggtctagactgtaggtacaaatttaaaagtcacttgcatttggatgcttaaagtcaggatattgtgaagtcaacagaggaataaataaatgcagagaggggaaagaaaaggcccatagactgagccattgtctggtttatttacatattagtatatattttcttaaagatgtttgctatataataatgagttacctaaagtgtgacttttctaaatttatggggaattttctacattgtgttatggcactactaaaaataataa

SEQ ID NO: 338 - DNA, 1275 bp, Homo sapiens
gtaaaactaattataattaaaatcaaaatatttactgaacctacttactcctataatttgcgttgctggttaaaacccagctataaaaattttgatcaaaaatttttattttgtaaatgatctgacacagcataaatgttaatcacatttctttattttatttgcagattaatttgagtaatttgaaaaattattaatgttacttaattactctcaacaccttacagtgtctcctgtaagcactattggtgatactgaatttaagttacatttaacaactatcagaaaatagtttttaaagtaaaaattatgatttggagtttaccaactaaatcttgttagctttcactgcctctattgagaagagcagcagttcttatcttcctcctttttcttctttaattaacaagagattatttgtatcatagccataaaatcagttcaggtattacatgaacgacacccctgactgcaatggtgtagtttattgtattagtccattttcatgctgctgataaagacatacataagactgggtaatttataaagaaatagaagtttaacggactcacagttccatgtggctggggaagcctcacaatcatgatcgaaggcaaaaggcacatcttacatggcaacaggcaagagagaatgagagccaagtgaaaggagaaaccccttataaaaccttcagacctcatgagacttattcactaccacaagaacagtatgtgagaaacagtcccatgatccagttatctcccactgggtccctcccaccacacaagggaattatgggaactgcaattcaagatgaaatgtgggtggaagcacaacggaactatatcatgatcaaagcattattgttttctctgataagctgatctagaaagtgctgcttgtgatcagctttggtgaccatgatcagtgaaatggttaaggaaatctacagattttgtaggtttgtgccttgacagacgaccggtatctgtttctcttttcatgatgaagtatctaacaaagctctgtccaaaattttgaatttctcgttaaawgcatcatgattatagaacagaggttacaatcaattattcagtcacacaatcactctcatcagtcattaaggtgcatacctggtgttccagttattcagtgtggtataacaaactacctggaacttaatggcttgaaatagtcaccattacattatgattgtccattctctgcatcaataattaggatttggcaaagagggaatggtttgtttacagacag

SEQ ID NO: 339 - DNA, 1275 bp, Homo sapiens
gtaaaactaattataattaaaatcaaaatatttactgaacctacttactcctataatttgcgttgctggttaaaacccagctataaaaattttgatcaaaaatttttattttgtaaatgatctgacacagcataaatgttaatcacatttctttattttatttgcagattaatttgagtaatttgaaaaattattaatgttacttaattactctcaacaccttacagtgtctcctgtaagcactattggtgatactgaatttaagttacatttaacaactatcagaaaatagtttttaaagtaaaaattatgatttggagtttaccaactaaatcttgttagctttcactgcctctattgagaagagcagcagttcttatcttcctcctttttcttctttaattaacaagagattatttgtatcatagccataaaatcagttcaggtattacatgaacgacacccctgactgcaatggtgtagtttattgtattagtccattttcatgctgctgataaagacatacataagactgggtaatttataaagaaatagaagtttaacggactcacagttccatgtggctggggaagcctcacaatcatgatcgaaggcaaaaggcacatcttacatggcaacaggcaagagagaatgagagccaagtgaaaggagaaaccccttataaaaccttcagacctcatgagacttattcactaccacaagaacagtatgtgagaaacagtcccatgatccagttatctcccactgggtccctcccaccacacaagggaattatgggaactgcaattcaagatgaaatgtgggtggaagcacaacggaactatatcatgatcaaagcattattgttttctctgataagctgatctagaaagtgctgcttgtgatcagctttggtgaccatgatcagtgaaatggttaaggaaatctacagattttgtaggtttgtgccttgacagacgaccggtatctgtttctcttttcatgatgaagtatctaacaaagctctgtccaaaattttgaatttctcgttaaatgcatcatgattatagaacagaggttacaatcaattattcagtcacacaatcactctcatcagtcattaaggtgcrtacctggtgttccagttattcagtgtggtataacaaactacctggaacttaatggcttgaaatagtcaccattacattatgattgtccattctctgcatcaataattaggatttggcaaagagggaatggtttgtttacagacag

SEQ ID NO: 340 - DNA, 1001 bp, Homo sapiens
gaaacaaaaaattgctttttatatattgatatttttgcacggatttcttaggattttctatgtacatgaccatgtcatctgcaaatgaaatagttttatttctttatcaatccggatgaatttattaaaattatcttgcctaatttcccaaatagggcctccatgttgaacataagtggtggcaagggtgatctgttgctaatctcagtggatgatattcagtgttttacaatgatcttcgacagctctggctgttaaattatcatagtctgtatggcctaaacaaacaaaatacttatgattatgggggaggctgggatatccaagatcaagttgctggcaggtctagcaacctgccactgggaagccctgcttcccagttttcagatggccaccttcttatagtatcttcaccaaagatagggcagagagagcaagcaagctctctaccttctcatataagggcactaatcccaccatgaaggcgccactgtcatgacstgattatgtcacaaagaccccggggcaaatattaccactgtgaggagtacagttttagcatgtgaattttggaagaacacaaacatttagtacagagtgactattaagtatgttattaactatggagtttttgtaggcattttttaacacattgagaaagtttcctctattcctacttttgttgagaagtttttatgatgacaaggcattacattttatccaatgacttttctgtgtgtattgagatgactgatttgttctgccaatttaaatccattgttgattctctctaggattttttttatttcagttattaaatttttcaacaggagaattactgtcttgttcttttttttgtaatttctgtccccttactggtattccatatttaataaggcatcataatagtactcttctttagtttcttaaagatggttttctttagtttttaacatatttatgtctatttagaagtctttgttaagtctgacatctgagct

SEQ ID NO: 341 - DNA, 1001 bp, Homo sapiens
ggatttcttaggattttctatgtacatgaccatgtcatctgcaaatgaaatagttttatttctttatcaatccggatgaatttattaaaattatcttgcctaatttcccaaatagggcctccatgttgaacataagtggtggcaagggtgatctgttgctaatctcagtggatgatattcagtgttttacaatgatcttcgacagctctggctgttaaattatcatagtctgtatggcctaaacaaacaaaatacttatgattatgggggaggctgggatatccaagatcaagttgctggcaggtctagcaacctgccactgggaagccctgcttcccagttttcagatggccaccttcttatagtatcttcaccaaagatagggcagagagagcaagcaagctctctaccttctcatataagggcactaatcccaccatgaaggcgccactgtcatgacctgattatgtcacaaagaccccggggcaaatattaccactstgaggagtacagttttagcatgtgaattttggaagaacacaaacatttagtacagagtgactattaagtatgttattaactatggagtttttgtaggcattttttaacacattgagaaagtttcctctattcctacttttgttgagaagtttttatgatgacaaggcattacattttatccaatgacttttctgtgtgtattgagatgactgatttgttctgccaatttaaatccattgttgattctctctaggattttttttatttcagttattaaatttttcaacaggagaattactgtcttgttcttttttttgtaatttctgtccccttactggtattccatatttaataaggcatcataatagtactcttctttagtttcttaaagatggttttctttagtttttaacatatttatgtctatttagaagtctttgttaagtctgacatctgagctctctcaaagtttctgctgattttttttttcctatgtttgg

SEQ ID NO: 342 - DNA, 701 bp, Homo sapiens
ggaaaccctggcctcttgatcacactttcctggagtttagtcccctctgcaatatgtacctgggagtcataagaaatgccagttacaaaaacttcctgtacagatatcctagcactcaactggaaaccggggagagtcacaattctgtctttccagccatatgtaactgaaatggagatcttttcaccctgagccaggggtgatgggaaagggagctggtcatggctcaatgtttagccttttcttggtcttcaagatttcatagacattcttaaatacatgtttctttcaatgaagtttgcccttaggacaattcacagctacattaggtactttttaaataatacttttgaccatccgtggttatttcattgaagaaaatctatagagcacctcagccatcattccagaagtgactatcctcctcagtaatggttcttattctaattttaaatatcattgatgtagaacattctatttcactattccttcattttattrttatgggaaattatatacagttctccagatttttaaagccttgctaacatgttttaagtcacacaaatattcttctgtgggaaaatgacagtaatttagtgtgcaacaattatatagaactatttttcaaacttataaacgaagtgaaattctaaataaaatcatttatcaaacacaaaaatttgagccagaataaggaa

SEQ ID NO: 343 - DNA, 701 bp, Homo sapiens
aatgccagttacaaaaacttcctgtacagatatcctagcactcaactggaaaccggggagagtcacaattctgtctttccagccatatgtaactgaaatggagatcttttcaccctgagccaggggtgatgggaaagggagctggtcatggctcaatgtttagccttttcttggtcttcaagatttcatagacattcttaaatacatgtttctttcaatgaagtttgcccttaggacaattcacagctacattaggtactttttaaataatacttttgaccatccgtggttatttcattgaagaaaatctatagagcacctcagccatcattccagaagtgactatcctcctcagtaatggttcttattctaattttaaatatcattgatgtagaacattctatttcactattccttcattttattattatgggaaattatatacagttctccagatttttaaagccttgctaacatgttttaagtcacacaaatattctyctgtgggaaaatgacagtaatttagtgtgcaacaattatatagaactatttttcaaacttataaacgaagtgaaattctaaataaaatcatttatcaaacacaaaaatttgagccagaataaggaatgtaaattacaatttaaacacagattataaactatcttacttttaaaatgttaaaattcctaacttgtttgaaa

SEQ ID NO: 344 - DNA, 768 bp, Homo sapiens
ctaaaatctaccattatatgatatccttcccaatacataaattaaaaaaaaaaacactgtagaggaaaaagcaatattttgaaatgatatgcttttctttgtttgtcttcaaacaattacatcttcatcataatggttgtattagtctgtttttacactgctataaagaattgcctgagactgagtaacatataaagaaaaaagttttaattgaccacagtttcacaggcttaataggaagcatgactgggaaacttagaatcatggcagaagaggaaggggaagcaaggatcttcttcacatggtagcaggagagagagcacaaagggggacacgctacacactttcaaacaacgagatctcctgagaactctatcgggagaacagcaagagggaagttcacccctatgattcaatcagctcccaccgggcttctcccctgacacatgaggaattacaattggatgagagatttgggtggggacacacagacaaaccatatcaactgtcatggacttaaacaattgtctttgaattgtcttttttcatacttttatttgcatctttycactaaaaagatgacacaaagtaatcctagtttacattttttaccatgtaattccatattactttttcctgaaagttacttatttttaaatctcaaagctcttcatacttatggtttgatctgcacttacaactggatctcagaaagattgaattctcccatcataccaagttcatgtctctcactcttaatatttgttc

SEQ ID NO: 345 - DNA, 701 bp, Homo sapiens
aaatgatatgcttttctttgtttgtcttcaaacaattacatcttcatcataatggttgtattagtctgtttttacactgctataaagaattgcctgagactgagtaacatataaagaaaaaagttttaattgaccacagtttcacaggcttaataggaagcatgactgggaaacttagaatcatggcagaagaggaaggggaagcaaggatcttcttcacatggtagcaggagagagagcacaaagggggacacgctacacactttcaaacaacgagatctcctgagaactctatcgggagaacagcaagagggaagttcacccctatgattcaatcagctcccaccgggcttctcccctgacacatgaggaattacaattggatgagagatttgggtggggacacacagacaaaccatatcaactgtcatggacttaaacaattgtctttgaattgtcttttttcatacttttatttgcatcttttcactaaaaagatgrcacaaagtaatcctagtttacattttttaccatgtaattccatattactttttcctgaaagttacttatttttaaatctcaaagctcttcatacttatggtttgatctgcacttacaactggatctcagaaagattgaattctcccatcataccaagttcatgtctctcactcttaatatttgttcccaagacaacaatt

SEQ ID NO: 346 - DNA, 6758 bp, Homo sapiens
agagtgggccattgttctgactagtctggggctccccaaagaactggtatctgtctcacctgactcagaacaatgataaggctgtagatctttttggaagtctatgaaaacaggcacaatgaaggcagcatgttagagatataattccacaggaagatgccaggtaaaacaaaagagaaaaagcaggaacaagctgattaggaaatttgtgatgactaaaagtatatacacaagcccaaataagatactccaaagatgtttgataggttctagatctctagatatactgctcaatgaaagtgtccccctgaacaaagccagtctgcaaagactgggtgagatgattttttttaaatgtcaagtctcagcaacaacaaaaatgacaagacatgcacagaagcaagaaaatataacacaatcaaagaaaaaaaagccacagaaatcagtcctagagaaaacygatctatgagctgcctgacaataattataaaataactatcataaaaatgcccagtgagatataagaaaacacagacaactaaatgaatcaggaaaatgatgcatgaacaaaatgggcatatcaacagagatggaaatgacaaagataaacaaacagaaattttggagcttaaaaatacagtaagtaaagtgaataattcactaaaaatattcaatagcagactagatcaggcagaagaaaatatcaatgaacttgaagacagatcatcaagtcagaggaacaacagcaacaaaaaagaatgaaaaaagtgaagacagcctaagggacttaggagtcagtaccaaggaaatcaatatatacgttatagatgtatcagaagaaaaagggagaaaaatgaaaagaaagcatatttgaaaaaataatagctgaagaattctcaatttcaaagagagaaattgatatacaaattcaagaagttcaaaagactctagccataataaatctaaagagactcacactaagacatattatcatcaaactgtcaaaatcaaagacaaagaattgtgaaatctgccaaggaaaagtgactcatcacacataagagatataacataagattgtcacaggatttctgaacagacactttgcaggtcagagggaagtagggtgacatattccaggtgctgaaagaagaaaacaccctgccaaccaagaatatggcatccagaaaaactttcctagaagaatgaaggagaaatttagactttcccaaataaacaaaagctgagggagttcattactaccagacctgctctgcaaaatgctaaagagaaaccttcaggtgaaacaaaaagatgctagacagtaacacaaaaccactcataaataacttcttcagtaaaaataatacatcgacaaatatggtaacctgtattaatactggtgcacaaattcactttcaaattttataaataagaatttaaaggatgaaaacatctaaaactaactataaatctatataatgaatatacaatatataaaaaaatttgtgatcacaataacataaaatgggggaggtagagctgtataggggtagagcttttgtatgcaattgaaattaccatcagtttaaactgaactgttataacattaagatgttttatgtaattgcaatggtaactatattctatagaatatattaaaaagaaaaagaaaataggaagggaatcaaagcatgtccttgtaaaaaagtcaatgaaagcaaaagaaaggcagaaagagtgaaaaggaggaataaaaagttataagacataaaaaaaatgaaaatagtaatagtcctgccatatcagtaattacattaaatataaatggattaaactccctaatcaaatcatagattggtttgcaagaactaactttacaattaaagacacacagctgacggtgaagggagaaaaaaaacttccatgcagtgaccaaaatagaggagggtggctgtattactgtcagacaaaataaaatttaagtcaaaaactgttacaagagtaaaagaagggcattatacagttaaaaaagtaaattcgccaggcagacacaacaattataaatatcaatacataaaaataagagctcctaaatatatgcagcaaacagacataattgaagaaagaaataaatagctaaaatggtagaagactttaatacccccacttacaataatgtataaaataacaagacagaatgtaaataaaaatgtagagaatttgagcaacactgtagaccaattggacctaataaatatactcagaataatccatccaaccaaagcagaaacagaatatacattcttttcaagtacacatttgacattctctgggattaactacatgttatgcaacaaacaagtctcaacaatgtttaaaagtctgatattacacaaagtattgtttctgatgacgatggaaagaacctagaagccaatagcaaaaagaaaatagaaaatccacacatatgtggaaattaaactacatgcaattaagcaaagggccaaagaagaagaagaaaaaagaaaacaccgtgaaacaaataaaaacaaaaatacagcatatgaaaatgcatgggatgcagcaaaagtgatggtaagagaaatgtttatagttataaatgcaaaccttaaaaaagaagaaagaaaacaaaaatactcaaattaacaactttacaagtcaagaaggtagagaaaaaagaacaaactataccaaaagctaacacagaaagaaaagaataaagattaaaaacaaaaacaatttaaaaaatagcagaactaaaagttggttctttgaaaagatcaacagaattgacaatttcttagctacattaagaaaaatacaagactcaaataacacaaatcagtggtgaaagggggtattataactgatgccacagaaatacaaaaggatcataagggactactacaaattgtatgacaacaaattgagtaacctaggataccttgataaattccaaaaaatgcacaatatactgaatcatgaatacatgacccttataaatcaagactaaatcataaagaaatagaaaatatcaacagaccaataattagtaaggagaataaactagtaatcagaaacctcccaacaaagaaaagcttaggaccaaatggctttactggagaattctaccaaccattaaaaggataattaagaccaatcttcctcaaacttttaaaacaaatgttaaagaggaggaaactctttcaatctcattcataaggtcagcattatccttataccaaaaccagacaaagacactattaaaaaaacttagaccaatatccctgatgaatttcgatgcaagaatcctcagcaaaatactatcaaacaattcaacagcatacttaaatgattatatgctgtaatcaagatgcatttattctttgaatgcaagtgtaattcaacacataaaattcaatcaatgtaatacaccacattaacagaatgagagacaaaaaccacataattatatcaactgatgcagaaaaaaatctgacacagttcaacaccttttgtgataaaaacactcaacaaactaggaaaagaaggaaacaactttaacacatcatatgctcactgatgaaaatctacaagttctttataaaagatcaggaacaagacaataatctgcattgttaccacttctattatacgtagtattggaagttctaatcagagcaaattaggcaagaaaaataaataaaaggcatccaaagtggaaaggaagtaaaataatctctttttacagatgatataaccttagaattagaaaatcctaaaaatttcacataccaagaaaaagcgtgttaaaattaataagtaaattcagcaagttgactgatacaaaatcaacacagaaagctcagttgtgtgtctgtgtgtctcatacactaacaatgaacaatctgaaaaggagattaagaaaacaatttcatttacaatagcatcaggaaaaaaaataaatacttaggaacaaacttaaccaaggggttggaattcctgtatactgaaaactacaaatattgccaaaagaaaataaaggagacacaaataagtgatatgtttttaatatgtccacccaaagtgatcttcagattcaatgaaatccctatcaaagttataatggcatttttctgcaggaatgtaaaaatttatcctaaaattcatatagaatctctaggtaccctgagggccaaacaattttgagaaaaaaaaaagaacaaaattggaggactcacacttccagattacaagaatatttacaaattacatatttacaaaaaaaattacaaagccacaataatcaaaacaacgtgggatttgcataaaggcagatatatagaccagtggaatagtattgagagtccagaaataaacccttaggtatatcatcaaatgacatttgacaaagtgctggtaccactcaatgggaatgggacaatttgttcaacaaatagagcaaagaaaactaaacatccatgtgcaaaagaataaatctggacccttatattacactatagacaaaattaattcaaaatggattaaagatctaaatgaaagatctaaaactataaaactcctaggagaaaacagaggaaaaatttcatgctaatttggcaacattttgtgatgtgacaccaaaagcagagtcaataaaagcaaaaattagacagatggaaatccatcatagtttataacttttggtcattaaagaacagtcaacagagtgaaaaggcaatctataaaatgggggaaaaacagaaaatatgtgcaaatcacagatatctgataggggattcatatccagaataaataaagaactcctatatctcaacaacaaaaaatctaatccaatcaaaaaatgggccaagggagtgaagatacatttctccaaagatgttatacaaatggccaggaagcatatgaaaagatgttcaatgtcactaatcatcagagaaatgcaaatcaaaaccacagtgcaatatcacttcacattcattagaatggcttctgtcatgaacaacagaaaataacaagtgttgatgagtgtgtagagaaattgagacctttatataattttggcagaaattcaaaatggtgcaaccactataaaaaatgatatggaggtcctcaaaaaattaaaaatagaactaccatatgatccacaatcccacctctgggtacatattcaaaagaattgaaagcagggtgttgaagatatatttgcacactctttatagcagcactgttcacaatagccaagagatgaaagtaacccaaaggttcatgaagcaatgaataaacaaaatatattatgtacatagagtaaaatactgtgcagctttaaagagaaaggaaatcttatactatgctacaacatgaatggaactttagggcattatagtaagtaaaataagccagttttttttaaaggacaaataaacactatacgattctacttaagtatttaatgttgtcaaatttataaatatagaatgtagaatagtggttaccctgagctgggggaaaggggcaaaggggaattgttattttaatgggtatagtttcagttctgcaaaatgaaaaggttctggaaatctgtttcacaatgttgtaaatataattactctgaaattgtacacttaaaaatggttaagatgacaaatagagttgtgatgtcttcttttgttattatatagaaaaactttttcatatgataatagtctttgtttttaagctgactttgctgatattaatataatccttccatttttctttaaaatgctatatgctttcacataattttgctttacgttgatgtatttatacataaggtgggtttcttatagataccacgttgtgtgtcttttttatctaagttgatagacttgccttttgttagggtatttaaataatttatatttaatgtaattattgatatagttgagtgtgttgatttttgttttctatttgctccatctgttgttggttctcattattcctctgtttctaccttcttttgtactaattattatattttattatttttcatctcaactgttggcttattagccacattgcttttaaaatttttaatgattgctctagggtttataataaacaaaatgttagcattttctaccatcaaatatttttacactattcatgtatacttcaatttctttcttcccatcctttgaactatatcttcatacattttactctacatttgttataactcagtgctttgaaagtcaattatttttgtctttgacagtcaatgatttttaaagagtttaacagtgaaaaaaaatggctttcatctttttccattagatttcatactccttctgcctgaagaatttcttttaatagaccttgtactgcgggtctcaggcaagaaattctctcagcctttgttggtttgaaaaactgcttattacacctttgtttttgaaagatattttcactaggtatagaagtctgggttgacagttctcattgtttgtcacagcatttttaagatgcccattcaattgtcttgtcttgtataattttggattagtctggtgtatttcttacctttgttcctctctgtgcaatgcttcaaccatcccacttcaggctgcctttaagatgttttcttttcccttaatctttagtttttagctggttgacagtgacgcatctaagtgtagtgtatgaggttgcttttattgtcactgttgttg

SEQ ID NO: 347 - DNA, 6758 bp, Homo sapiens
agagtgggccattgttctgactagtctggggctccccaaagaactggtatctgtctcacctgactcagaacaatgataaggctgtagatctttttggaagtctatgaaaacaggcacaatgaaggcagcatgttagagatataattccacaggaagatgccaggtaaaacaaaagagaaaaagcaggaacaagctgattaggaaatttgtgatgactaaaagtatatacacaagcccaaataagatactccaaagatgtttgataggttctagatctctagatatactgctcaatgaaagtgtccccctgaacaaagccagtctgcaaagactgggtgagatgattttttttaaatgtcaagtctcagcaacaacaaaaatgacaagacatgcacagaagcaagaaaatataacacaatcaaagaaaaaaaagccacagaaatcagtcctagagaaaactgatctatgagctgcctgamaataattataaaataactatcataaaaatgcccagtgagatataagaaaacacagacaactaaatgaatcaggaaaatgatgcatgaacaaaatgggcatatcaacagagatggaaatgacaaagataaacaaacagaaattttggagcttaaaaatacagtaagtaaagtgaataattcactaaaaatattcaatagcagactagatcaggcagaagaaaatatcaatgaacttgaagacagatcatcaagtcagaggaacaacagcaacaaaaaagaatgaaaaaagtgaagacagcctaagggacttaggagtcagtaccaaggaaatcaatatatacgttatagatgtatcagaagaaaaagggagaaaaatgaaaagaaagcatatttgaaaaaataatagctgaagaattctcaatttcaaagagagaaattgatatacaaattcaagaagttcaaaagactctagccataataaatctaaagagactcacactaagacatattatcatcaaactgtcaaaatcaaagacaaagaattgtgaaatctgccaaggaaaagtgactcatcacacataagagatataacataagattgtcacaggatttctgaacagacactttgcaggtcagagggaagtagggtgacatattccaggtgctgaaagaagaaaacaccctgccaaccaagaatatggcatccagaaaaactttcctagaagaatgaaggagaaatttagactttcccaaataaacaaaagctgagggagttcattactaccagacctgctctgcaaaatgctaaagagaaaccttcaggtgaaacaaaaagatgctagacagtaacacaaaaccactcataaataacttcttcagtaaaaataatacatcgacaaatatggtaacctgtattaatactggtgcacaaattcactttcaaattttataaataagaatttaaaggatgaaaacatctaaaactaactataaatctatataatgaatatacaatatataaaaaaatttgtgatcacaataacataaaatgggggaggtagagctgtataggggtagagcttttgtatgcaattgaaattaccatcagtttaaactgaactgttataacattaagatgttttatgtaattgcaatggtaactatattctatagaatatattaaaaagaaaaagaaaataggaagggaatcaaagcatgtccttgtaaaaaagtcaatgaaagcaaaagaaaggcagaaagagtgaaaaggaggaataaaaagttataagacataaaaaaaatgaaaatagtaatagtcctgccatatcagtaattacattaaatataaatggattaaactccctaatcaaatcatagattggtttgcaagaactaactttacaattaaagacacacagctgacggtgaagggagaaaaaaaacttccatgcagtgaccaaaatagaggagggtggctgtattactgtcagacaaaataaaatttaagtcaaaaactgttacaagagtaaaagaagggcattatacagttaaaaaagtaaattcgccaggcagacacaacaattataaatatcaatacataaaaataagagctcctaaatatatgcagcaaacagacataattgaagaaagaaataaatagctaaaatggtagaagactttaatacccccacttacaataatgtataaaataacaagacagaatgtaaataaaaatgtagagaatttgagcaacactgtagaccaattggacctaataaatatactcagaataatccatccaaccaaagcagaaacagaatatacattcttttcaagtacacatttgacattctctgggattaactacatgttatgcaacaaacaagtctcaacaatgtttaaaagtctgatattacacaaagtattgtttctgatgacgatggaaagaacctagaagccaatagcaaaaagaaaatagaaaatccacacatatgtggaaattaaactacatgcaattaagcaaagggccaaagaagaagaagaaaaaagaaaacaccgtgaaacaaataaaaacaaaaatacagcatatgaaaatgcatgggatgcagcaaaagtgatggtaagagaaatgtttatagttataaatgcaaaccttaaaaaagaagaaagaaaacaaaaatactcaaattaacaactttacaagtcaagaaggtagagaaaaaagaacaaactataccaaaagctaacacagaaagaaaagaataaagattaaaaacaaaaacaatttaaaaaatagcagaactaaaagttggttctttgaaaagatcaacagaattgacaatttcttagctacattaagaaaaatacaagactcaaataacacaaatcagtggtgaaagggggtattataactgatgccacagaaatacaaaaggatcataagggactactacaaattgtatgacaacaaattgagtaacctaggataccttgataaattccaaaaaatgcacaatatactgaatcatgaatacatgacccttataaatcaagactaaatcataaagaaatagaaaatatcaacagaccaataattagtaaggagaataaactagtaatcagaaacctcccaacaaagaaaagcttaggaccaaatggctttactggagaattctaccaaccattaaaaggataattaagaccaatcttcctcaaacttttaaaacaaatgttaaagaggaggaaactctttcaatctcattcataaggtcagcattatccttataccaaaaccagacaaagacactattaaaaaaacttagaccaatatccctgatgaatttcgatgcaagaatcctcagcaaaatactatcaaacaattcaacagcatacttaaatgattatatgctgtaatcaagatgcatttattctttgaatgcaagtgtaattcaacacataaaattcaatcaatgtaatacaccacattaacagaatgagagacaaaaaccacataattatatcaactgatgcagaaaaaaatctgacacagttcaacaccttttgtgataaaaacactcaacaaactaggaaaagaaggaaacaactttaacacatcatatgctcactgatgaaaatctacaagttctttataaaagatcaggaacaagacaataatctgcattgttaccacttctattatacgtagtattggaagttctaatcagagcaaattaggcaagaaaaataaataaaaggcatccaaagtggaaaggaagtaaaataatctctttttacagatgatataaccttagaattagaaaatcctaaaaatttcacataccaagaaaaagcgtgttaaaattaataagtaaattcagcaagttgactgatacaaaatcaacacagaaagctcagttgtgtgtctgtgtgtctcatacactaacaatgaacaatctgaaaaggagattaagaaaacaatttcatttacaatagcatcaggaaaaaaaataaatacttaggaacaaacttaaccaaggggttggaattcctgtatactgaaaactacaaatattgccaaaagaaaataaaggagacacaaataagtgatatgtttttaatatgtccacccaaagtgatcttcagattcaatgaaatccctatcaaagttataatggcatttttctgcaggaatgtaaaaatttatcctaaaattcatatagaatctctaggtaccctgagggccaaacaattttgagaaaaaaaaaagaacaaaattggaggactcacacttccagattacaagaatatttacaaattacatatttacaaaaaaaattacaaagccacaataatcaaaacaacgtgggatttgcataaaggcagatatatagaccagtggaatagtattgagagtccagaaataaacccttaggtatatcatcaaatgacatttgacaaagtgctggtaccactcaatgggaatgggacaatttgttcaacaaatagagcaaagaaaactaaacatccatgtgcaaaagaataaatctggacccttatattacactatagacaaaattaattcaaaatggattaaagatctaaatgaaagatctaaaactataaaactcctaggagaaaacagaggaaaaatttcatgctaatttggcaacattttgtgatgtgacaccaaaagcagagtcaataaaagcaaaaattagacagatggaaatccatcatagtttataacttttggtcattaaagaacagtcaacagagtgaaaaggcaatctataaaatgggggaaaaacagaaaatatgtgcaaatcacagatatctgataggggattcatatccagaataaataaagaactcctatatctcaacaacaaaaaatctaatccaatcaaaaaatgggccaagggagtgaagatacatttctccaaagatgttatacaaatggccaggaagcatatgaaaagatgttcaatgtcactaatcatcagagaaatgcaaatcaaaaccacagtgcaatatcacttcacattcattagaatggcttctgtcatgaacaacagaaaataacaagtgttgatgagtgtgtagagaaattgagacctttatataattttggcagaaattcaaaatggtgcaaccactataaaaaatgatatggaggtcctcaaaaaattaaaaatagaactaccatatgatccacaatcccacctctgggtacatattcaaaagaattgaaagcagggtgttgaagatatatttgcacactctttatagcagcactgttcacaatagccaagagatgaaagtaacccaaaggttcatgaagcaatgaataaacaaaatatattatgtacatagagtaaaatactgtgcagctttaaagagaaaggaaatcttatactatgctacaacatgaatggaactttagggcattatagtaagtaaaataagccagttttttttaaaggacaaataaacactatacgattctacttaagtatttaatgttgtcaaatttataaatatagaatgtagaatagtggttaccctgagctgggggaaaggggcaaaggggaattgttattttaatgggtatagtttcagttctgcaaaatgaaaaggttctggaaatctgtttcacaatgttgtaaatataattactctgaaattgtacacttaaaaatggttaagatgacaaatagagttgtgatgtcttcttttgttattatatagaaaaactttttcatatgataatagtctttgtttttaagctgactttgctgatattaatataatccttccatttttctttaaaatgctatatgctttcacataattttgctttacgttgatgtatttatacataaggtgggtttcttatagataccacgttgtgtgtcttttttatctaagttgatagacttgccttttgttagggtatttaaataatttatatttaatgtaattattgatatagttgagtgtgttgatttttgttttctatttgctccatctgttgttggttctcattattcctctgtttctaccttcttttgtactaattattatattttattatttttcatctcaactgttggcttattagccacattgcttttaaaatttttaatgattgctctagggtttataataaacaaaatgttagcattttctaccatcaaatatttttacactattcatgtatacttcaatttctttcttcccatcctttgaactatatcttcatacattttactctacatttgttataactcagtgctttgaaagtcaattatttttgtctttgacagtcaatgatttttaaagagtttaacagtgaaaaaaaatggctttcatctttttccattagatttcatactccttctgcctgaagaatttcttttaatagaccttgtactgcgggtctcaggcaagaaattctctcagcctttgttggtttgaaaaactgcttattacacctttgtttttgaaagatattttcactaggtatagaagtctgggttgacagttctcattgtttgtcacagcatttttaagatgcccattcaattgtcttgtcttgtataattttggattagtctggtgtatttcttacctttgttcctctctgtgcaatgcttcaaccatcccacttcaggctgcctttaagatgttttcttttcccttaatctttagtttttagctggttgacagtgacgcatctaagtgtagtgtatgaggttgcttttattgtcactgttgttg

SEQ ID NO: 348 - DNA, 501 bp, Homo sapiens
gaccatgttatgacattttagtgcttgctaagcagtaaatactgacttactttcctgctacactcttcagagcagaaagagaaatctacaaaaagggcaatgtagttgggatccaccacagccttgagactgggccatgtttctacagcttacccacattttacccccactttctctgagaaacaatgcaaactggagaacaaggtcagagaagttatcttggatggtagaagagaagaaaggagaagaarggataagcagaaaatcaaaaagggcataaaaaaattactggggaaaataattcttagtcactcaccatttcttatgtttgtgaaaacagaaacgaggagcaagtgttgttgtaagaattgttcttgcccctccccctccaccacccacatctgtcaagctatccctgtttcactgtttcctctgcactctctattaacttctttgtcctcctcttttcttttcctacagcaaagactttttgtcatgttt

SEQ ID NO: 349 - DNA, 501 bp, Homo sapiens
tgacttactttcctgctacactcttcagagcagaaagagaaatctacaaaaagggcaatgtagttgggatccaccacagccttgagactgggccatgtttctacagcttacccacattttacccccactttctctgagaaacaatgcaaactggagaacaaggtcagagaagttatcttggatggtagaagagaagaaaggagaagaaaggataagcagaaaatcaaaaagggcataaaaaaattactggrgaaaataattcttagtcactcaccatttcttatgtttgtgaaaacagaaacgaggagcaagtgttgttgtaagaattgttcttgcccctccccctccaccacccacatctgtcaagctatccctgtttcactgtttcctctgcactctctattaacttctttgtcctcctcttttcttttcctacagcaaagactttttgtcatgttttgtttctttttctattgtttctttcccttttctaatccttga

SEQ ID NO: 350 - DNA, 1148 bp, Homo sapiens
tatgagatttaatgttaagaaataaaatgtaggatctaaaacgtaatctatagcataatctcaaaaatggtttagaaatgacataataatacagacatttgtgggtggtaggattatgcatatttttatatatttttaaatatatttttcaaaagcttcctataaagaatgtaattctttcccaattccaaatctagcttaaacataattttacaaaaattattctctcagaatgtaaactagtaccacctctatggaaaacattatggagatttcctaaagagttaaaagtagatctaccatttgatccagcaatcttaatactgggtatctacccggaggaaaagaagtcattgtatgaaaaagacacttgtacacatatgtttacaggaccacaattcacaaatgcaaagatgcagaaccaacctaagtggccastgactaatgagaggataaagaagatgtggcatatatatatcagggactactactcagccattacaaggaacaaaataatgtcttttgcaacaacttggatagagctggaggccattattctaagtaaagtaattcaggaattggaaaaccaaaaaccgtatgttctctcttataagtgggaactaagttaggaataagcaaaggcacacagagggacatattggactttagagactcacgaggaggagggtaataggggactagggattaaaagaaaaactagacattaggtacaaggtaccctacttaagtgcactaaaatctcagaattcaccactacgtaattcaactaagtaacaagaaaccacttgtaccccaaaagctactgaaataaaaattattctctcaaaaattttaagccctaaacttcagttcctattgtttatatttactaagaaaaacaacagaaaacactgttttaaaaatggtggatttttttaaggttaaaggtatataagacagctgcctaaggaaacgcagatacccctgtaccttgttgttgttgttgtttttcacttttttaaaaaacatagagatgggatctccttatgctgcccaggcttgtctcaaactcctgagctcaagcaatcctctgacctcagactctcaaagttttgggactacaggcgacagtcaccatgccagccaat

SEQ ID NO: 351 - DNA, 1148 bp, Homo sapiens
tatgagatttaatgttaagaaataaaatgtaggatctaaaacgtaatctatagcataatctcaaaaatggtttagaaatgacataataatacagacatttgtgggtggtaggattatgcatatttttatatatttttaaatatatttttcaaaagcttcctataaagaatgtaattctttcccaattccaaatctagcttaaacataattttacaaaaattattctctcagaatgtaaactagtaccacctctatggaaaacattatggagatttcctaaagagttaaaagtagatctaccatttgatccagcaatcttaatactgggtatctacccggaggaaaagaagtcattgtatgaaaaagacacttgtacacatatgtttacaggaccacaattcacaaatgcaaagatgcagaaccaacctaagtggccactgactaatgagaggataaagaagatgtggcatatatayatcagggactactactcagccattacaaggaacaaaataatgtcttttgcaacaacttggatagagctggaggccattattctaagtaaagtaattcaggaattggaaaaccaaaaaccgtatgttctctcttataagtgggaactaagttaggaataagcaaaggcacacagagggacatattggactttagagactcacgaggaggagggtaataggggactagggattaaaagaaaaactagacattaggtacaaggtaccctacttaagtgcactaaaatctcagaattcaccactacgtaattcaactaagtaacaagaaaccacttgtaccccaaaagctactgaaataaaaattattctctcaaaaattttaagccctaaacttcagttcctattgtttatatttactaagaaaaacaacagaaaacactgttttaaaaatggtggatttttttaaggttaaaggtatataagacagctgcctaaggaaacgcagatacccctgtaccttgttgttgttgttgtttttcacttttttaaaaaacatagagatgggatctccttatgctgcccaggcttgtctcaaactcctgagctcaagcaatcctctgacctcagactctcaaagttttgggactacaggcgacagtcaccatgccagccaat

SEQ ID NO: 352 - DNA, 1148 bp, Homo sapiens; identical to SEQ ID NO: 351

SEQ ID NO: 353 - DNA, 1148 bp, Homo sapiens
tatgagatttaatgttaagaaataaaatgtaggatctaaaacgtaatctatagcataatctcaaaaatggtttagaaatgacataataatacagacatttgtgggtggtaggattatgcatatttttatatatttttaaatatatttttcaaaagcttcctataaagaatgtaattctttcccaattccaaatctagcttaaacataattttacaaaaattattctctcagaatgtaaactagtaccacctctatggaaaacattatggagatttcctaaagagttaaaagtagatctaccatttgatccagcaatcttaatactgggtatctacccggaggaaaagaagtcattgtatgaaaaagacacttgtacacatatgtttacaggaccacaattcacaaatgcaaagatgcagaaccaacctaagtggccactgactaatgagaggataaagaagatgtggcatatatatatcagggactactrctcagccattacaaggaacaaaataatgtcttttgcaacaacttggatagagctggaggccattattctaagtaaagtaattcaggaattggaaaaccaaaaaccgtatgttctctcttataagtgggaactaagttaggaataagcaaaggcacacagagggacatattggactttagagactcacgaggaggagggtaataggggactagggattaaaagaaaaactagacattaggtacaaggtaccctacttaagtgcactaaaatctcagaattcaccactacgtaattcaactaagtaacaagaaaccacttgtaccccaaaagctactgaaataaaaattattctctcaaaaattttaagccctaaacttcagttcctattgtttatatttactaagaaaaacaacagaaaacactgttttaaaaatggtggatttttttaaggttaaaggtatataagacagctgcctaaggaaacgcagatacccctgtaccttgttgttgttgttgtttttcacttttttaaaaaacatagagatgggatctccttatgctgcccaggcttgtctcaaactcctgagctcaagcaatcctctgacctcagactctcaaagttttgggactacaggcgacagtcaccatgccagccaat

SEQ ID NO: 354 - DNA, 611 bp, Homo sapiens
caaaacctcaaccttccagataagtctaagggtgagaacttcacacaagatgaataagaaccaatttcttccagggcgatgttgaacctggaaatgaaagccaatctctcttggaaggcctggtttgtagaaatgtcagtctttgtttcaagctgtgggagaatgagaagcaagactttagggaaagaggaataaaatagatgtgcagaaataacagagtgagaaagtcttcagggtgtcgctagccctaattgcaggcatccctgaatcctagaccttggattgcaagagactccttaatatcttcccatgtccacatttgcttcacatagtttgaatgtggcttctattatatacagatacaagattcaaatccaacctctaygatgactggtcttgtgaataagcagaagaggcactaacaatatgacgtgagggattcagggaagagcactttcttgagcacatatcttccctggtctgccagctgtagtttatgaaattccacaatgaggatgaaatggaatcaccatttacagagtactctccagatgtctaaccctaagctaggtaccttcaaaatattatctagtttagataatcaacccttt

SEQ ID NO: 355 - DNA, 601 bp, Homo sapiens
ttctctagtccaaagggttgattatctaaactagataatattttgaaggtacctagcttagggttagacatctggagagtactctgtaaatggtgattccatttcatcctcattgtggaatttcataaactacagctggcagaccagggaagatatgtgctcaagaaagtgctcttccctgaatccctcacgtcatattgttagtgcctcttctgcttattcacaagaccagtcatcatagaggttggatttgaatcttgtatctgtatataatagaagccacattcaaactatgtgaagyaaatgtggacatgggaagatattaaggagtctcttgcaatccaaggtctaggattcagggatgcctgcaattagggctagcgacaccctgaagactttctcactctgttatttctgcacatctattttattcctctttccctaaagtcttgcttctcattctcccacagcttgaaacaaagactgacatttctacaaaccaggccttccaagagagattggctttcatttccaggttcaacatcgccctggaagaaattggttcttattcatcttgtgtgaagttctcacccttagactt

SEQ ID NO: 356 - DNA, 527 bp, Homo sapiens
gctctagaatatggcattccagaagtgggatgctacaaatagtctcattgagagtcaacttgcacaatgtatcgtcctacccttacatcaatttctgaaacaacttctctttgcacttcccctatagttacatgcataataaattctgacaactcttatgaagtcatggaataactttcttcttatgtttcctatcaatgtcattagccctttatcttgtttgagtttccatcagcaatgttttcaagtcccaagatcattcatgtatccacaagcaatgatacgccagatttggacaaataatactgaatactatcttattttcactgccatgatcaaggcagtgtggattgctgccaagtccaagagaagtgaggtcagcagctgcaagccacctccgtcatttagaaaagcttcatgatgtagtgtgtcgtttcgatgtgacactgtctcacagagttaaaatgatgtgmaaggaactgttcaatggaaatttagaaatttctctttttctcaattttagtgta

SEQ ID NO: 357 - DNA, 601 bp, Homo sapiens
gaacaagattttcctgcttttaaaaatactacattaaagctgaaaatttaggccaaaattttcaagtggtaatagttacaggcaattcatctttctggtcagaaaagggtgttactgcagctatttctgcctgaaactgggtggcactactacttttttttttttttttttaactgagcagacattttccttacactaaaattgagaaaaagagaaatttctaaatttccattgaacagttccttgcacatcattttaactctgtgagacagtgtcacatcgaaacgacacactacatcaygaagcttttctaaatgacggaggtggcttgcagctgctgacctcacttctcttggacttggcagcaatccacactgccttgatcatggcagtgaaaataagatagtattcagtattatttgtccaaatctggcgtatcattgcttgtggatacatgaatgatcttgggacttgaaaacattgctgatggaaactcaaacaagataaagggctaatgacattgataggaaacataagaagaaagttattccatgacttcataagagttgtcagaatttattatgcatgtaactacagggga

SEQ ID NO: 358 - DNA, 1001 bp, Homo sapiens
gcttaatacctgagtgatggaatattctgttcaacaaacccctctgacataggtttgcctatataataaacctgttcatgtactcctgaacctaaaagtttaaaaaagattatgtagaaaacccaaaggaatctataaaaagtctactagagctagagtgattttaacaagatttcaatacacaaattcaaatgtctttctatatattaatgacaatcaacaataaaattttaaaacattattaaagtataatgaaaatatcaactgtttagggagaaatgtaacaagaatggtgaaggacctatacactaaaaagcttcaatatgttgttgagattaactgaagaaggtctaaatagatttttttttcatgtctcggaagacttaatatgtgaagataccaattcttccccaaatgatcaacaggtgaaatgcaatcccaatcaaaatcccagcaattattttaagggggaaattggcaatctgattctaaaattcatayggaaaaaaacaatggagttagaataactaaaacaagtccgaaaaagaaaaagaaatggaggactaatgctacctgatttcaagtcttatcgtataaatctacatcaataaaggacaagttggtattgggttaaagatagataaatacatcagtggaatagaatattgaatccagaataaatccacacatatatggataaaaataccagacaattcagtggagatggttttgtttttacaacaaatgttactggaacaaattgatatatgtattagtcagatatggctgccataacaaagaaccacaaacaggtggtttaaataatggaaataaatttcctcagaattctggagtatggaagcccaagatcaagttgctgggaggattcgtttcttctgagtgtctctttttttgatgacagatgactatcttttaccaatgtcttcacttggttttccctctgtgtgtgcctaggtcctattctccaattcctataagga

SEQ ID NO: 359 - DNA, 1001 bp, Homo sapiens
ctaaaagtttaaaaaagattatgtagaaaacccaaaggaatctataaaaagtctactagagctagagtgattttaacaagatttcaatacacaaattcaaatgtctttctatatattaatgacaatcaacaataaaattttaaaacattattaaagtataatgaaaatatcaactgtttagggagaaatgtaacaagaatggtgaaggacctatacactaaaaagcttcaatatgttgttgagattaactgaagaaggtctaaatagatttttttttcatgtctcggaagacttaatatgtgaagataccaattcttccccaaatgatcaacaggtgaaatgcaatcccaatcaaaatcccagcaattattttaagggggaaattggcaatctgattctaaaattcatatggaaaaaaacaatggagttagaataactaaaacaagtccgaaaaagaaaaagaaatggaggactaatgctacctgatttcaagtcttatcrtataaatctacatcaataaaggacaagttggtattgggttaaagatagataaatacatcagtggaatagaatattgaatccagaataaatccacacatatatggataaaaataccagacaattcagtggagatggttttgtttttacaacaaatgttactggaacaaattgatatatgtattagtcagatatggctgccataacaaagaaccacaaacaggtggtttaaataatggaaataaatttcctcagaattctggagtatggaagcccaagatcaagttgctgggaggattcgtttcttctgagtgtctctttttttgatgacagatgactatcttttaccaatgtcttcacttggttttccctctgtgtgtgcctaggtcctattctccaattcctataaggaaaccagtcatattggattagggcccactctaatggccccattttacttgcattatctctttaaagacactatctccagatgtagccacact

SEQ ID NO: 360 - DNA, 1058 bp, Homo sapiens
catgattagctatgctactttccactgctcttagtatactgagaggcagcataagtaaaactaaaatatctgaagatagcaatagactatttaaagtagaagaagtatgctatttttgttttgttttcatttcgaaggaaatatgcaaaggtttattgagtatttcagcttctcttacagtaggttttttttggattctttctgtgtttgtctatgttgataaaacattgaaatgccatatagctcaaaggtcattcacttaagaaatctaagtactgataacatcttagccccgattcttcataggcattgttaagcctattataattttggtwcagagagaaggtaaactatattccagacaggcatataaagcaatttctcctataattggagttcacgaaaaattcacatatttctttttaatagtaactctcacagcaagaacatatgtttgtaaataatacatcacagaatcttattggcagacaaggaaattcctaaaatattttttactgccacatcaattaagatatataaaataccttatatagaagatgtttgcacccaggccaaacaaatcaaacaagaatagaagcactgacagtcttatttcaaaattggtttaacttgtatttacaggatattgtagtaccttataaagttgattgctgattggccgtcttttacagaattctgtcagattgttattatttcttgtaaagattgattcaaacaaataaaaattgtcaggattggatatgtcctatagtgaggtgtagttatgtcacatgagatttttaattacaaagaaatggaaaataaaatgagaatagaattgagactcccctgtcacctcacaaatatgttgaaatacaatgaaatttccaaagatgttaaagcatataaagttgaataattcttattatgtattaaacttacagaaatttaatttctttactttataagaggtagtgaaaatataaaattaattatgaagacagagtagtcttagtcagacatggccctataaagcatattcccattcgttacatcaa

SEQ ID NO: 361 - DNA, 1058 bp, Homo sapiens
catgattagctatgctactttccactgctcttagtatactgagaggcagcataagtaaaactaaaatatctgaagatagcaatagactatttaaagtagaagaagtatgctatttttgttttgttttcatttcgaaggaaatatgcaaaggtttattgagtatttcagcttctcttacagtaggttttttttggattctttctgtgtttgtctatgttgataaaacattgaaatgccayatagctcaaaggtcattcacttaagaaatctaagtactgataacatcttagccccgattcttcataggcattgttaagcctattataattttggtacagagagaaggtaaactatattccagacaggcatataaagcaatttctcctataattggagttcacgaaaaattcacatatttctttttaatagtaactctcacagcaagaacatatgtttgtaaataatacatcacagaatcttattggcagacaaggaaattcctaaaatattttttactgccacatcaattaagatatataaaataccttatatagaagatgtttgcacccaggccaaacaaatcaaacaagaatagaagcactgacagtcttatttcaaaattggtttaacttgtatttacaggatattgtagtaccttataaagttgattgctgattggccgtcttttacagaattctgtcagattgttattatttcttgtaaagattgattcaaacaaataaaaattgtcaggattggatatgtcctatagtgaggtgtagttatgtcacatgagatttttaattacaaagaaatggaaaataaaatgagaatagaattgagactcccctgtcacctcacaaatatgttgaaatacaatgaaatttccaaagatgttaaagcatataaagttgaataattcttattatgtattaaacttacagaaatttaatttctttactttataagaggtagtgaaaatataaaattaattatgaagacagagtagtcttagtcagacatggccctataaagcatattcccattcgttacatcaa

SEQ ID NO: 362 - DNA, 956 bp, Homo sapiens
aaaacaaggaacaaacaaacaaaaatgttacaaccgaacaacagacttttgagtcatgtttcaggccaagaggtgatgagttactgtagttgcttgagctggttggtgaaatattacctggcaacaaaactgaaatagaaggtggcttagtaaaatgcagattcagaatgagtgccttaaggttaaggcatataagaccaaactgattttctttttcacgaggtcttcaggtaaggccattgtagaagataccttgtttgcgaacttcagtaaattacttcacttgtctcatattttcattttcaggatggaggcttgagattgaattgtagtgcaattaggtaaatttttacccattttaaatataatattaaaatattaattataaattaccttatttgaatctggaataatatttattgcagggcatataatctaagctgtaaacgtcctgtyagaagacaacatattcatcttgctaaggtataagctatatgactggcactgtgctcaactcagagtcattgaatgaacagtatttatttaatctatgaatgagagcacttcaagtatacagaaagatatctcaaaagattcagccttacattgctcataacttcaatgacttagatgaaaacctcctgaacatttttatcagttgtataggtaccccaaatcataagggaatgtttatcaattagatgatgaaatggggatgcaactacatcatggcaggctaaagcaatagaatgactttgacaagaggaaattacatagaggcacctgagtctcctaaaccaatttcaaaggtatgagaggggggtgatataaataaatagttgatagatgaaaaaactcagaagttatagttgacagcaattttaatataatatgaaaaatgtggttggacttttagggaaaaaaacctaataaaatctaatggaaattagtggtcc

SEQ ID NO: 363 - DNA, 956 bp, Homo sapiens
caaccgaacaacagacttttgagtcatgtttcaggccaagaggtgatgagttactgtagttgcttgagctggttggtgaaatattacctggcaacaaaactgaaatagaaggtggcttagtaaaatgcagattcagaatgagtgccttaaggttaaggcatataagaccaaactgattttctttttcacgaggtcttcaggtaaggccattgtagaagataccttgtttgcgaacttcagtaaattacttcacttgtctcatattttcattttcaggatggaggcttgagattgaattgtagtgcaattaggtaaatttttacccattttaaatataatattaaaatattaattataaattaccttatttgaatctggaataatatttattgcagggcatataatctaagctgtaaacgtcctgtcagaagacaacatattcatcttgctaaggtrtaagctatatgactggcactgtgctcaactcagagtcattgaatgaacagtatttatttaatctatgaatgagagcacttcaagtatacagaaagatatctcaaaagattcagccttacattgctcataacttcaatgacttagatgaaaacctcctgaacatttttatcagttgtataggtaccccaaatcataagggaatgtttatcaattagatgatgaaatggggatgcaactacatcatggcaggctaaagcaatagaatgactttgacaagaggaaattacatagaggcacctgagtctcctaaaccaatttcaaaggtatgagaggggggtgatataaataaatagttgatagatgaaaaaactcagaagttatagttgacagcaattttaatataatatgaaaaatgtggttggacttttagggaaaaaaacctaataaaatctaatggaaattagtggtccactcatttctccacctaggatgttaaaaat

SEQ ID NO: 364 - DNA, 601 bp, Homo sapiens
gtaaaacacatagatcgctgtatccttgttcagtaagctacaacatactcgtatctcctgaaatcctgggcttaaatcgaggtctcaaaggctttgttttgttttgttgtatggttgtatggtgagtgtgtgtgtgtgtgtgtgtgtgtgtgtttattctcctgaaattctcctcctcacttgacttaagctaaaagataaacgtcctcttcctttcagccacagatggtgatggataaattgaatgtcattcacattattcccttaaaataaactctctccctcccctctcccgtctcawccttgtccctttctttatataatgggtaatgcgttaatgtcagcagaatagttttggggccataatggcaagtatcacgtggatggtttagcattgtttttagaatgctgtgaatttgggtatatgtgagttttggggaaagttttgcaactatatgtttgttaattaaatgaggactataaagtaatataaaattatgtttctggaacatattttggaagctataaagtcatctgtatttattatccacagacataatgtcattgttcaggtcctgcaaccttcttataatcaacatac

SEQ ID NO: 365 - DNA, 601 bp, Homo sapiens
agtaagctacaacatactcgtatctcctgaaatcctgggcttaaatcgaggtctcaaaggctttgttttgttttgttgtatggttgtatggtgagtgtgtgtgtgtgtgtgtgtgtgtgtgtttattctcctgaaattctcctcctcacttgacttaagctaaaagataaacgtcctcttcctttcagccacagatggtgatggataaattgaatgtcattcacattattcccttaaaataaactctctccctcccctctcccgtctcatccttgtccctttctttatataatgggtaatkcgttaatgtcagcagaatagttttggggccataatggcaagtatcacgtggatggtttagcattgtttttagaatgctgtgaatttgggtatatgtgagttttggggaaagttttgcaactatatgtttgttaattaaatgaggactataaagtaatataaaattatgtttctggaacatattttggaagctataaagtcatctgtatttattatccacagacataatgtcattgttcaggtcctgcaaccttcttataatcaacatacgtgggcccagggattttatgtatcttcgcct

SEQ ID NO: 366 - DNA, 1079 bp, Homo sapiens
gaatttatggtctgatggagaagggaatcattaaagttctatgtagtgagatatccccaaggggtgtattaggcttaccaccactggaatctggatagatgaagacagagtggcagggaagtcgtattaaggttctgtttctgctgggagccacaggtcctcaggaagcaacaagtactgggcagattgatactgtagctrggctctagctctatacctctagaataaaggttacaaactagcaacttgaaagctaaacctggcccacagatatgttttatttggctcttacactgttttaaaaaatattaccaacatttaaaactgggaagttttatgaaaaaacccagacttctggattctgttgaaaaaaaaaatcagaagatctggcaatactgagctgacattcctatatgacaacaattggctggatctatgcagcttctctccaaaaagcaaagaatgtgttcttgcttaacacagtccccaccactccctcatattctccaatcctggacctgagcgtcatttgctatgtatcgccatttgccatgaagttttacactctacagaaatataatttttttgtagaagactatgctttaatcaagatcaggataatataaagtgagatctgaaagtggaaaaaagataaatgtccaacaatgatagactggattaagaaaatgtggcacatatacaccgtggagtactatgcagccaaaaaaaacgatgagttcatgtcctttgtagggacatggatgaagctggaaaccaccattctcagcaaactatcgcaaggacaaaaaaccaaacgccgcatgttctcactcataggtgggaattgaacaatgagaacacttgggcacaggaaggggaacatcacacaccgggccctgttgtggggtggggggaggagggagggatagcatttggagatatacctaatgttaaatgactagtttctgggtgcagcacaccatcatggcacatgtatacatatgtaactaacctgcacattgtgcacatgtaccctaaaacttaaagtataatttttaaaaaaagatattttcttatct

SEQ ID NO: 367 - DNA, 501 bp, Homo sapiens
ataaattttctcttccctcaagaatttatggtctgatggagaagggaatcattaaagttctatgtagtgagatatccccaaggggtgtattaggcttaccaccactggaatctggatagatgaagacagagtggcagggaagtcgtattaaggttctgtttctgctgggagccacaggtcctcaggaagcaacaagtactgggcagattgatactgtagctgggctctagctctatacctctagaataaakgttacaaactagcaacttgaaagctaaacctggcccacagatatgttttatttggctcttacactgttttaaaaaatattaccaacatttaaaactgggaagttttatgaaaaaacccagacttctggattctgttgaaaaaaaaaatcagaagatctggcaatactgagctgacattcctatatgacaacaattggctggatctatgcagcttctctccaaaaagcaaagaatgtgttcttgcttaaca

SEQ ID NO: 368 - DNA, 1001 bp, Homo sapiens
tgaagaagccgcctggcttcttgtttcttctcatagcaaaatgcaatgagaaagagataatttgagaaaagaaccgtttaaacaaaaagaaaccaagacataatgattttggaaattctcagtttattcagactgcaaaagatattaaaataaagaaactcagtaacagggatagataatctaaagaaaaagcctaggacacggctgtagtaaccttctgtttttatacctcagcaatttgctaatgcctcaaaaagatcaaaagtactcaaatataaagggctctttgaagagattagatttcctcaatcaaaccaaagagcatcgaggaagcttaaggttactgtccctcacatatctcagcagaaggcaaaaatagaagactgattatctaagaaagatctctgaaagagtctcatattatggagtgaacccctgtggcatacatgggagacccacttggttcttgagaattttatatcaggagaaacactgtcagtytgtattgaaaggaacagagaaaatacgaaattaaagaagactattaaacctccaaaattctggcaggaaagaagcttacacagctactcagttgcaaagatctgccacttttcatatacatgaaaggactcagaggaggaagccacaggtttagaaggaaaagctaaaagcaacatcgtattagtcttggatctaggaacctaatttctctagcagaatctagaaatggcttgggacaagtgattgtttttttacctaggattttctccctcttgaaaacaggactgtctgtaactattatcctatgcctgccctaccatcatatttcagaaacaggtaacttatgttttcactttcaaagattcacaataaagagaaattgtacctcagaatggattataccagagctttcctcatgcataaattaaataatttaggttatgtgatttgaagcttttgagtgggtgaggtgacattttggatgctgagttggtgccgta

SEQ ID NO: 369 - DNA, 1001 bp, Homo sapiens
tcttctcatagcaaaatgcaatgagaaagagataatttgagaaaagaaccgtttaaacaaaaagaaaccaagacataatgattttggaaattctcagtttattcagactgcaaaagatattaaaataaagaaactcagtaacagggatagataatctaaagaaaaagcctaggacacggctgtagtaaccttctgtttttatacctcagcaatttgctaatgcctcaaaaagatcaaaagtactcaaatataaagggctctttgaagagattagatttcctcaatcaaaccaaagagcatcgaggaagcttaaggttactgtccctcacatatctcagcagaaggcaaaaatagaagactgattatctaagaaagatctctgaaagagtctcatattatggagtgaacccctgtggcatacatgggagacccacttggttcttgagaattttatatcaggagaaacactgtcagtctgtattgaaaggaacagagaaaatrcgaaattaaagaagactattaaacctccaaaattctggcaggaaagaagcttacacagctactcagttgcaaagatctgccacttttcatatacatgaaaggactcagaggaggaagccacaggtttagaaggaaaagctaaaagcaacatcgtattagtcttggatctaggaacctaatttctctagcagaatctagaaatggcttgggacaagtgattgtttttttacctaggattttctccctcttgaaaacaggactgtctgtaactattatcctatgcctgccctaccatcatatttcagaaacaggtaacttatgttttcactttcaaagattcacaataaagagaaattgtacctcagaatggattataccagagctttcctcatgcataaattaaataatttaggttatgtgatttgaagcttttgagtgggtgaggtgacattttggatgctgagttggtgccgtagtgagtccagaattctgcggaactt

SEQ ID NO: 370 - DNA, 601 bp, Homo sapiens
ctctagactcctcctgtattttaatttagccacttttttagggcctacaattttagatctccacagggctcttgaaacttcttgaacctcatcagtaacatgtccattagtggcatgacccaagagttctagaacatctattcagcaagtgtgtatctggtaagtgaatattccttctatgtgttcccttttgcatcaaactacacactgtcattcctcctttatctccaaaagcttgaaaattcctcacttgtatctcattctttctctcttagaaaactgatcacctctgatgaattaraacggaatgaccaagctttgggagaggcaaaagaatctcggtgttaaagactcagagtttaagaagcaacaaaaagattatacagatgtgaatatgtgaccttcctccaccagggcatgttgccttggagtaagataatctaagcacacacttcatagcctgagaacaattttggaagtctttgctttatggatatttacataaagcaaatatggatatttacctaaaggctggaccaaggcctaattcctctagagccccttgatcatgaacaccattcctgtcatgattcttaaggtc

SEQ ID NO: 371 - DNA, 601 bp, Homo sapiens
acaagctccagccatggacgcaattccttctagaagcaaaatttatctctagactcctcctgtattttaatttagccacttttttagggcctacaattttagatctccacagggctcttgaaacttcttgaacctcatcagtaacatgtccattagtggcatgacccaagagttctagaacatctattcagcaagtgtgtatctggtaagtgaatattccttctatgtgttcccttttgcatcaaactacacactgtcattcctcctttatctccaaaagcttgaaaattcctcacttgtrtctcattctttctctcttagaaaactgatcacctctgatgaattagaacggaatgaccaagctttgggagaggcaaaagaatctcggtgttaaagactcagagtttaagaagcaacaaaaagattatacagatgtgaatatgtgaccttcctccaccagggcatgttgccttggagtaagataatctaagcacacacttcatagcctgagaacaattttggaagtctttgctttatggatatttacataaagcaaatatggatatttacctaaaggctggaccaaggcctaattcctcta

SEQ ID NO: 372 - DNA, 701 bp, Homo sapiens
gaagatgcactctaatgttttttcccagaagctctgtaggtttagcttttacctttctgggtttgttttgttttgttttttgagatggagtcccactcgtgtcacccaggctggagtacaatggtgcaatctcggttcactgcaacctccacctcccgggttcaagcaattcccctgtctccacctctcgagtagctgggatgggaggcgcctgccaccatacctggctaattttcatatttttagtaaagatagggtttcaccatgttagccaggctggtctcgaactcctgacctcaagtgatccacccgcctcagcttcccaaagtgctgggattacaggcgtgagccactgcgcccagccctagctttttggtctatgattcctcccaaattaatttctgtgaaccattaccttaagatgttgagatttaatgtccagaatctcatttgttcacctttgaaaattaagaaaccctggcacagtgttgactggagccwcttaccttaatagaaaataaagctcacatatatccataatgaaaagcagagaccagcacaaccatagtcacctgacagttttaaaatccaaggccaggatcttctcaactcaggcccactcacttactccacaacatacttcttctttcctcagcatctactacttgtgctgggaccttggtcttcccattgttcatgtc

SEQ ID NO: 373 - DNA, 701 bp, Homo sapiens
agatggagtcccactcgtgtcacccaggctggagtacaatggtgcaatctcggttcactgcaacctccacctcccgggttcaagcaattcccctgtctccacctctcgagtagctgggatgggaggcgcctgccaccatacctggctaattttcatatttttagtaaagatagggtttcaccatgttagccaggctggtctcgaactcctgacctcaagtgatccacccgcctcagcttcccaaagtgctgggattacaggcgtgagccactgcgcccagccctagctttttggtctatgattcctcccaaattaatttctgtgaaccattaccttaagatgttgagatttaatgtccagaatctcatttgttcacctttgaaaattaagaaaccctggcacagtgttgactggagccacttaccttaatagaaaataaagctcacatatatccataatgaaaagcagagaccagcacaaccatagtcacctgacagtttwaaaatccaaggccaggatcttctcaactcaggcccactcacttactccacaacatacttcttctttcctcagcatctactacttgtgctgggaccttggtcttcccattgttcatgtcattcttttcctcacagttcccattcttttctccctgaaataaagaaatttcaaaatataccatgtttcatgaaaaagacaaa

SEQ ID NO: 374 - DNA, 701 bp, Homo sapiens
gatttccaccctcaggtgatggggatggttgaacatccaacacctgaaacaggacagacgatattgacagtacttgttagttgcatataatcacagaccagtggaaacagatgaaccacacagggccacagcggggtttcactggggaacagagtgaacaatcaggaggtgtgggaggcaggtttagtagtttaaagaggttgaggtgtccccctggatcccatgggaggatcacattggctcatttgaattatcatacggactggcagggaactgaaatcttctactcagggataagcagaaactgtccctggtttccttgataaaaagggttgtttgataggggaccttatccatgggaggaaagtgaggagggaaatttgtggctaagccattcaaggccctcccagttttactagatgtcaaggcagcacacgtaatattgggacttaattttagccacataactaataaatttgtaagtatgtgcaacggctcacrcttgcttccagaatggcacctaaaaaacagatttacctctccccaaattcagatatggaattaaatgtaatgtcaggaaaattgtctaagagttggaaatgggaaaaaaatgttcttttggtggagttatggactccagaggttatcagattctattgaataacgtacttttgattgtatttgtaacaattaggctattt

SEQ ID NO: 375 - DNA, 1001 bp, Homo sapiens
gcatataatcacagaccagtggaaacagatgaaccacacagggccacagcggggtttcactggggaacagagtgaacaatcaggaggtgtgggaggcaggtttagtagtttaaagaggttgaggtgtccccctggatcccatgggaggatcacattggctcatttgaattatcatacggactggcagggaactgaaatcttctactcagggataagcagaaactgtccctggtttccttgataaaaagggttgtttgataggggaccttatccatgggaggaaagtgaggagggaaatttgtggctaagccattcaaggccctcccagttttactagatgtcaaggcagcacacgtaatattgggacttaattttagccacataactaataaatttgtaagtatgtgcaacggctcacacttgcttccagaatggcacctaaaaaacagatttacctctccccaaattcagatatggaattaaatgtaatgtcaggaaaaytgtctaagagttggaaatgggaaaaaaatgttcttttggtggagttatggactccagaggttatcagattctattgaataacgtacttttgattgtatttgtaacaattaggctatttgtgaactcggtaggggtagaaatcgagttgtagaaaatggatggtaatgcaagtgatttttgaccatatcaatgcaaatgaattctgttggtagaaatattcatttccacactgtagatgaccctaaacatatgtcattacattatattttattgccttatagactattaaccaattttgaatcatacagtagcaaatttatttcagcattcttgtgtgtatgtgtttatatatacacgtgcatatgtatttaagatatataattgtatattcttcaaattcttctttgaacaggtttgaacctcttattagtttcctcattaaggaatttaataagacctttaatgcatgtttgtattttcatgagagtcattattttacc

SEQ ID NO: 376 - DNA, 695 bp, Homo sapiens
tgctccttcattagtgcaatggaacagcaaatcaggatactttcacagttctcttaagtgagcctagaagtggggagctgcttgttcacaaacttgaagcctgaatatgttaatattctttcagtggccggacgcggtggctcatgcctgtaatcccaacactttgggaggccgaggtaggcagatcaacctgaagtcaggagttcgaggccagcctggccaacatggtgaaaccccacctgttggtctgtactaaaaatagaaaaattagctgggcatggtggcgcatgcctgtaatcccagctactcaggaggctgtggcagaagaatcgcctgcacctgggaggcagaggttgctttgagttgatatcgtgtcactgcactccagcctgggcaacagagtgagatcctttcagaaacctgctgtctgtatttggatacaattaaaaaaaaaaaaaagatgagacaggcaggtgcgaaagaaataaaagtcamaactgatccagttgggaaactcagaattgacagttacgtgtcctttcatttattgatattttgagattcacaggggtttaaactttatttttccaagactgaatagttcccacctcccttccatatataaaatttgagtagctggggagatttaaaagaggctccccataaactcagaagttaaaagagacaagggtccc

SEQ ID NO: 377 - DNA, 601 bp, Homo sapiens
aaccccacctgttggtctgtactaaaaatagaaaaattagctgggcatggtggcgcatgcctgtaatcccagctactcaggaggctgtggcagaagaatcgcctgcacctgggaggcagaggttgctttgagttgatatcgtgtcactgcactccagcctgggcaacagagtgagatcctttcagaaacctgctgtctgtatttggatacaattaaaaaaaaaaaaaagatgagacaggcaggtgcgaaagaaataaaagtcacaactgatccagttgggaaactcagaattgacagttasgtgtcctttcatttattgatattttgagattcacaggggtttaaactttattcttccaagactgaatagttcccacctcccttccatatataaaatttgagtagctggggagatttaaaagaggctccccataaactcagaagttaaaagagacaagggtcccagtaaatacaaaatgattggggttgaggaggcagattttctgtcctcagtgaagtttgttggttggttggttggttggttggttaattggttggtttttgagtcagggtctcactttgtcacccaagctggagtgca

SEQ ID NO: 378 - DNA, 663 bp, Homo sapiens
tgtagcaacaggagggatgagacccaaaggtctgaaaagccagtattttaagaagtcttggaaaatgtggaggttgaaaaatctaacaggagtgcttgcttcagcagcaatttagagtagattagcatggcctctgcgccaggatgacatgcacattcctaaaagtgttccgtgttttaaaaaaaagagagagacagaatctaaggggatgtgtacatttgctagagctactataacaaagtaccagaggcagggtcacttcaacaacagaaatttatttctcacagttctggaggctagacgtccaagattaaggtgttgactgggttgaattcagcccataacaggaaataaggagttaaataaagcacttgcttctattgtttgtacctaaacttaacagaayacagtaagtaacaagtcattgggatgcagaaaagaaaaaagagagtgaaggaaggagagaaggtgaagggagaatggaagagaggaagggagggaggaaagaaaagtttgatgaatgattgcagtctaaactggttcaaacaagagatcttgtttaattaaggaattcatcccatctctgcctattaggaggaggaaaaagtctaaaatagaagatggtgaaagttggatgaccccaggcattaaggccattcatct

SEQ ID NO: 379 - DNA, 662 bp, Homo sapiens
ttaagaagtcttggaaaatgtggaggttgaaaaatctaacaggagtgcttgcttcagcagcaatttagagtagattagcatggcctctgcgccaggatgacatgcacattcctaaaagtgttccgtgttttaaaaaaaagagagagacagaatctaaggggatgtgtacatttgctagagctactataacaaagtaccagaggcagggtcacttcaacaacagaaatttatttctcacagttctggaggctagacgtccaagattaaggtgttgactgggttgaattcagcccataacaggaaataaggagttaaataaagcacttgcttctattgtttgtacctaaacttaacagaacacagtaagtaacaagtcattgggatgcagaaaagaaaaaagagagtgaaggaaggagaraaggtgaagggagaatggaagagaggaagggagggaggaaagaaaagtttgatgaatgattgcagtctaaactggttcaaacaagagatcttgtttaattaaggaattcatcccatctctgcctattaggaggaggaaaaagtctaaaatagaagatggtgaaagttggatgaccccaggcattaaggccattcatctttaactgttatgcttggatcatgcaaatgtgtctggtagctacaag

SEQ ID NO: 380 - DNA, 615 bp, Homo sapiens
ttccatacattccttccacaccattgcccttaacctttcaaattcctgcttaaaactaatcccatttttatggctgacctcaccctgtatcaaaaactccgacatccctttacgacagagagcacaaactagtggtccaaaatgtcatgggggtcttctcagagttgttttttcaatcaggaaatttcacataaaaatatggatttctgatttctcttttaaaaacagaaaaacgagccaccagtgggagcactgcaggtatctgtgtgagaccygtacttcacaactcctgctttccctccataaagtagcttgcattttccacattgactttgcagttctttggtatctgtattggttttaagataatttctactatatcacatatctcctcacagtacaaagatatcattttctttcccttttctttttaaaaaatttgtatttttaatttttgtgggtacacagtagatatttatggggcatatgaggtattttataggcatataatatgtactagggtaagtggggtattcatcacctcaagcatttatcctttctttgtgtaaaatatagcattttctgaacactatgaatacttaagtacaaggatca

SEQ ID NO: 381 - DNA, 994 bp, Homo sapiens
tcaaagtgtaacaaatttcctttcctcataaactagcagacattctatcccctcattattgtaacacatttctaatatctttctcaaattgtcttcctgtattacaatgcactcaccttggcttagaatgtctgagacaagaaaatctattcaccattcccacagatgactccctcactctcctcccaagtcttccatacattccttccacaccattgcccttaacctttcaaattcctgcttaaaactaatcccatttttatggctgacctcaccctgtatcaaaaactccgacatccctttacgacagagagcacaaactagtggtccaaaatgtcatgggggtcttctcagagttgttttttcaatcaggaaatttcacataaaaatatggatttctgatttctcttttaaaaacagaaaaacgagccaccagtgggagcactgcaggtatctgtgtgagacctgtacttcacaactcctgctttccctccataaagyagcttgcattttccacattgactttgcagttctttggtatctgtattggttttaagataatttctactatatcacatatctcctcacagtacaaagatatcattttctttcccttttctttttaaaaaatttgtatttttaatttttgtgggtacacagtagatatttatggggcatatgaggtattttataggcatataatatgtactagggtaagtggggtattcatcacctcaagcatttatcctttctttgtgtaaaatatagcattttctgaacactatgaatacttaagtacaaggatcaagtcataggatttggaattgatttttaaaatatgttgaccaaagtgctcttatcatcaaacttaacatcactaatgaaggatgaacatcccaaatctgaaaatccaaaatccaaaatgctccataatctaaaacttgttgagcaccaacatgatgcttaaaggaaatgctcctggagcatttcagat

SEQ ID NO: 382 - DNA, 1001 bp, Homo sapiens
ctatgagaaatatttttaaagtggttaggaacaattcatagcactgacatgttatcagtaaaaatagaagaaaataaattaatattatgaaatattaattatatttcattaattatgtaatatgaattatgttttagctcaaatatttcccaagggacaattaagtaaatgaaaaatacacacagattaaaataataaatagagaaggagatattaatgaggtacaaaaagaaaaaatacatgtaatcacatgaaatgctattatttgaaagattaacaaaacttgtaaactacctgctaacttgatcaaagaaaaaaatcgagaaaccatatgcgcaattaatagtaagagggaaataaacattgaaacagaagacatttgaaataccatataagactgggtttcagagctctatgtacgtaaattgataatgtcctggagaagtgcagatgaccaaaatggacacctttcaacttagaaatcataaacagattcatttycttaaagttaatgaaaagaattaacagaccctcctcaaaaaagacatatatgcggcctacaatcatatgaaaaaaagttcaacattactgttcattagagaaatgcaaatcaaaaccacaatgagataccatctcacaccagtcagaatggctattattaagaagtcaaaaaataaaagatgctggcgaggttgtggagaaaaaagaatgcttttatacacttggtgggaatgtaaattagttcagtcattgtggaagactttgatgattcctagaagacctaaatacagaactactatttgacccaacaatcccattactgggtatatactcaaatgactataaatcattctattataaagacacatgcatggatatgttcattacagcactatgcacaatagcaaagacttggaatcaacatgaatgtccatcaatgatagactagataaagaaaatgtggtacacatataccatggaatactatgcagccataaaaa

SEQ ID NO: 383 - DNA, 1001 bp, Homo sapiens
tcagtaaaaatagaagaaaataaattaatattatgaaatattaattatatttcattaattatgtaatatgaattatgttttagctcaaatatttcccaagggacaattaagtaaatgaaaaatacacacagattaaaataataaatagagaaggagatattaatgaggtacaaaaagaaaaaatacatgtaatcacatgaaatgctattatttgaaagattaacaaaacttgtaaactacctgctaacttgatcaaagaaaaaaatcgagaaaccatatgcgcaattaatagtaagagggaaataaacattgaaacagaagacatttgaaataccatataagactgggtttcagagctctatgtacgtaaattgataatgtcctggagaagtgcagatgaccaaaatggacacctttcaacttagaaatcataaacagattcatttccttaaagttaatgaaaagaattaacagaccctcctcaaaaaagacatatatgcrgcctacaatcatatgaaaaaaagttcaacattactgttcattagagaaatgcaaatcaaaaccacaatgagataccatctcacaccagtcagaatggctattattaagaagtcaaaaaataaaagatgctggcgaggttgtggagaaaaaagaatgcttttatacacttggtgggaatgtaaattagttcagtcattgtggaagactttgatgattcctagaagacctaaatacagaactactatttgacccaacaatcccattactgggtatatactcaaatgactataaatcattctattataaagacacatgcatggatatgttcattacagcactatgcacaatagcaaagacttggaatcaacatgaatgtccatcaatgatagactagataaagaaaatgtggtacacatataccatggaatactatgcagccataaaaatgaaggagatcatgccctttgcagggacacgaatagaggtggaggccattatcc

SEQ ID NO: 384 - DNA, 501 bp, Homo sapiens
agttgcttgaaagcaaagttctcgcagtagctctctatctagaaggaggcattttatttatgtaaggaagtcacctaaaagaaaattcatttgttatggtgtggctttaagagttacttacttttaatggaatcccccagataataataaattctgaaaaaaaaaaatcagaatcatggcatgttaaaactggatacattcctagaaatagatggaaactgctcttgcaaaaagcttagcacatgttaaarcattttagaaacaatttgccaaagtttatttagtctagtgatttcgacaggttaaatggaccctttgagatcttttttcctcaagtacaaaggctcacttgcttaatgaacacagtcccagaaaagcagggggctgaaccttggctctaccatcttacctaagattctagagttagcaaagggtttccacaagcccaaattattatgtttaatcttttcaattatctgtgaagcattaggttggtgcaaa

SEQ ID NO: 385 - DNA, 501 bp, Homo sapiens
gaggcattttatttatgtaaggaagtcacctaaaagaaaattcatttgttatggtgtggctttaagagttacttacttttaatggaatcccccagataataataaattctgaaaaaaaaaaatcagaatcatggcatgttaaaactggatacattcctagaaatagatggaaactgctcttgcaaaaagcttagcacatgttaaagcattttagaaacaatttgccaaagtttatttagtctagtgatttygacaggttaaatggaccctttgagatcttttttcctcaagtacaaaggctcacttgcttaatgaacacagtcccagaaaagcagggggctgaaccttggctctaccatcttacctaagattctagagttagcaaagggtttccacaagcccaaattattatgtttaatcttttcaattatctgtgaagcattaggttggtgcaaaagtaactgcaggttttgacattaaaactggcaaaaactgcaataa

SEQ ID NO: 386 - DNA, 703 bp, Homo sapiens
gacaccagttagcatattgtcgcgggggagaggggtgggaaaggcgagagaacagcatgtggtccagaggccatacccagatggaggctgcagtcagctccccagtcaaaggcaaagcccaagtcaaagccatgcttccctcttgcccacctgctccaatgccacccacagagagtgcgccacagctcacaggatgcaggtctggttgaatcttaacaataactttgtaagggaggtgtcattagctccattctcctggcaggaggatgaggctcaaggcagctaaaggcttttgctgaacatcaagtggtgagccaggactcaawgccagatcttcttgtttccctgttaggtgtatgtagcacaactggtatctgcagactatgctgctggaagggctagccgtcactgttatcacagcgactgctgcctgagatatgccaggtactgctgcaagaagtttacaaatataagctcacttgatcttcataacatactacctaggtacaatcattatatttatttgacagatacagagacagaggggacacagaaaggattagtaacttgccccaaaccacacagccagcaaggtgtaagtgagcacctgcagtctagatgagacaccactcaaaacgtcatttttctggcagccccgtgcagttaccacagtggtcaccccagtggtcagctaaaggccaag

SEQ ID NO: 387 - DNA, 704 bp, Homo sapiens
gcatattgtcgcgggggagaggggtgggaaaggcgagagaacagcatgtggtccagaggccatacccagatggaggctgcagtcagctccccagtcaaaggcaaagcccaagtcaaagccatgcttccctcttgcccacctgctccaatgccacccacagagagtgcgccacagctcacaggatgcaggtctggttgaatcttaacaataactttgtaagggaggtgtcattagctccattctcctggcaggaggatgaggctcaaggcagctaaaggcttttgctgaacatcaagtggtgagccaggactcaatgccagatcttcttgtttccctgttaggtgtwtgtagcacaactggtatctgcagactatgctgctggaagggctagccgtcactgttatcacagcgactgctgcctgagatatgccaggtactgctgcaagaagtttacaaatataagctcacttgatcttcataacatactacctaggtacaatcattatatttatttgacagatacagagacagaggggacacagaaaggattagtaacttgccccaaaccacacagccagcaaggtgtaagtgagcacctgcagtctagatgagacaccactcaaaacgtcatttttctggcagccccgtgcagttaccacagtggtcaccccagtggtcagctaaaggccaagcccaccgtttct

SEQ ID NO: 388 - DNA, 975 bp, Homo sapiens
gacttaagacaagggggtcttaatttgattatttttttctgttttatatgatttctatgaaaactacaacaaaataaagttaattctatttaagtgactttttaatgaattgcctttgttagaaaaaaaattaagtgtttttgtctcactctgtcacccaggctggagcacagtggtgtgatcatggcttactgcagccatgacctcccgggctcaggtgatcctcccacctcagcttcccaaatagatgggactacagttgtgtgccacaacgcctggctaatttttgtatttttttgtagagacagggtctcaccaggttgcccaggctgatcttgaactccttggctcaagcgatccacccacctcagcctccctgagtgctgggattacaggcatgagccagcgcacccagccagaattacatttttttaaatggtactgtcctagaaaatccaggatgtgcagtgatcaygtatgaatgcatggacctgcacacacaggagtgaacaaaagacccacccctgccaggtcaccactcatatctcaccccagcccacgctagctcacactcctccccacacaccactgacctcatcattgctaggtacccacttgacttctcaacaggttcaagacaattggccttcctcgtctcttctagaaacaccctcttttctgggctttgtgtaacacctggtctttctcccctctctggccacttctcagcttttctttttctttctttcttttttttttttttttttttgccacttcctcttcctctacatcaagcttgtccaacccacagcccaggacagctttgaatgcagcctaacacaaattcgtaagctttcttaaaacattatgagatgtgtgtgtgtgtgtgtgtgtgtgtgtgtgtgtgtgtgtgtgtgtgtgtttagctcatcagctatcgttattgttagtgtattttatgtgtggcccaagaca

SEQ ID NO: 389 - DNA, 976 bp, Homo sapiens
gactttttaatgaattgcctttgttagaaaaaaaattaagtgtttttgtctcactctgtcacccaggctggagcacagtggtgtgatcatggcttactgcagccatgacctcccgggctcaggtgatcctcccacctcagcttcccaaatagatgggactacagttgtgtgccacaacgcctggctaatttttgtatttttttgtagagacagggtctcaccaggttgcccaggctgatcttgaactccttggctcaagcgatccacccacctcagcctccctgagtgctgggattacaggcatgagccagcgcacccagccagaattacatttttttaaatggtactgtcctagaaaatccaggatgtgcagtgatcacgtatgaatgcatggacctgcacacacaggagtgaacaaaagacccacccctgccaggtcaccactcatatctcaccccagcccacgctagctcacrctcctccccacacaccactgacctcatcattgctaggtacccacttgacttctcaacaggttcaagacaattggccttcctcgtctcttctagaaacaccctcttttctgggctttgtgtaacacctggtctttctcccctctctggccacttctcagcttttctttttctttctttcttttttttttttttttttttgccacttcctcttcctctacatcaagcttgtccaacccacagcccaggacagctttgaatgcagcctaacacaaattcgtaagctttcttaaaacattatgagatgtgtgtgtgtgtgtgtgtgtgtgtgtgtgtgtgtgtgtgtgtgtgtgtttagctcatcagctatcgttattgttagtgtattttatgtgtggcccaagacatttcttcttccagtgtggcccagggaagccaaaagattggacacccctgctctacaacatctcaatataggcctttttcatgtttcattctagatt

SEQ ID NO: 390 - DNA, 801 bp, Homo sapiens
atccagacggtgcccatactccctgctctgtctagatggtgtccacattccctgctccgtctagactgtgcccatattcgctgctggctgcaaatgcgaggagttgacagcagcctcccctttacaaggcaggaggtgccactgttcgccattgtctccacctagggcttcacttgctttctatctgcagacatcagagggacccacatctctctgttctgacacgctgtgtgttgatggcagagtttaattatccacatgcaatcttactttccttattcccaagtccgtggggctgcctcatcaaagcattgtaagaactgataaccatcttctagaagtatcatagtgatattaagaacacacatcacagatcatagtaaatggctttaattttttarcgaaatctcactactgcaaatgcattgttgtcctagctaatgaatgcatagagtattgcctgcaaaataataattgagattctatttttaagaagcttagaacagtacatggtgcatagcaaagactctgtgtatgtgaagccagattttaaaatatggtaacaagtgtctgaaaatatgtggctcaatttgtctcccggttacttttccctctccccctttaaaatgtagaggaaggagaagaagagataagaggtttgtgagtgaagacaagggccctttaaggcctgggaagactaacgccatagggatctccctctgccttaaaaggcacaggaatcttagtggggaaaaagaagtggtgataaatagccagtccgtgtgcctggaatatcaaagt

SEQ ID NO: 391 - DNA, 801 bp, Homo sapiens
ccctgctccgtctagactgtgcccatattcgctgctggctgcaaatgcgaggagttgacagcagcctcccctttacaaggcaggaggtgccactgttcgccattgtctccacctagggcttcacttgctttctatctgcagacatcagagggacccacatctctctgttctgacacgctgtgtgttgatggcagagtttaattatccacatgcaatcttactttccttattcccaagtccgtggggctgcctcatcaaagcattgtaagaactgataaccatcttctagaagtatcatagtgatattaagaacacacatcacagatcatagtaaatggctttaattttttagcgaaatctcactactgcaaatgcattgttgtcctagctaatgaatgcayagagtattgcctgcaaaataataattgagattctatttttaagaagcttagaacagtacatggtgcatagcaaagactctgtgtatgtgaagccagattttaaaatatggtaacaagtgtctgaaaatatgtggctcaatttgtctcccggttacttttccctctccccctttaaaatgtagaggaaggagaagaagagataagaggtttgtgagtgaagacaagggccctttaaggcctgggaagactaacgccatagggatctccctctgccttaaaaggcacaggaatcttagtggggaaaaagaagtggtgataaatagccagtccgtgtgcctggaatatcaaagtcagtgcgtgccagggatcacactgcgggtcacgtgcactctgggtctct

SEQ ID NO: 392 - DNA, 601 bp, Homo sapiens
ttggcctggggctgattcctccaaagcaatgtgtctcttcgcagagtctcttagagctgcaaggcagtatgggatcatcagagaggatgctaggaagcttcagaaatggaggtcctggtagaaagggtcctttggcgtggcctctgaagagtccaaatgtgggacaagaccctccgaaagcggtggcctggggagccacaggtggggcagccagcacggaagagggtggctttgctaccattgggaaaacttatcctccacatcctcatgaggcaaacacctttcctaccttaccgctccycagtggcctccctgttgccttcttattcaagactaagaccctctagaatgttctttatcctgagtccagctgattgtctatactaatatcagtacggggtgtagatgaggacaaccagtgtgcctggctgccaggcaccccctccccaaaccccaggagtttctggaacattccaactctgcttgagggtatccatgcagcatctactactgtgagcaggtggtctgatctgtggaaaacttctatgattcacctgagggtaactgccctttgtgatttgaaagaatgatgctaacagaa

SEQ ID NO: 393 - DNA, 601 bp, Homo sapiens
gcagagtctcttagagctgcaaggcagtatgggatcatcagagaggatgctaggaagcttcagaaatggaggtcctggtagaaagggtcctttggcgtggcctctgaagagtccaaatgtgggacaagaccctccgaaagcggtggcctggggagccacaggtggggcagccagcacggaagagggtggctttgctaccattgggaaaacttatcctccacatcctcatgaggcaaacacctttcctaccttaccgctcctcagtggcctccctgttgccttcttattcaagactaagacyctctagaatgttctttatcctgagtccagctgattgtctatactaatatcagtacggggtgtagatgaggacaaccagtgtgcctggctgccaggcaccccctccccaaaccccaggagtttctggaacattccaactctgcttgagggtatccatgcagcatctactactgtgagcaggtggtctgatctgtggaaaacttctatgattcacctgagggtaactgccctttgtgatttgaaagaatgatgctaacagaaagtgttgtcatttctgaacttttctgaactctgcagcgag

SEQ ID NO: 394 - DNA, 1001 bp, Homo sapiens
agatttggatggggacacaaaaccaaaccatatcataggttaaattgtgtctcccaccccaaaaatgtgtatgttgaagtcctaaccttcagtactcagaatgtgacattatttggaaatagggtcattgcagatggagttagttaagatgaggtcattaggatgagtccctaatccaatatgactggtgctcttacaaaaaggggaagtttggacacagagccatgcacatgggtgggaagaatcccaaatgaacggataggcagagggttggagagatgcatcaacaaggaacaccaaagattgccagcaacccccagaagctgggggagaggcctggaacagattctccctcacagcctgagaggaaccaagctggctgacaccttgatctcaggttaccggccttgagaactgagagaccctgggtttctgttgtttaagcctctcagggtgcagcactttattatggaagcctgagctgactaatacaggtgtctytatatctcactgagggaaagtgacaggaaagtaagaaccatttatgtccaagagtccagaggagtcaaccagattctgggggaaaagaaggtacaatgctggcctctccatgcagcctagtccccaacacttgtagggcccagggcaagatctaaagcactctctcacctatgcatctatatgctgtaactcagataaacaaactattaaataatatatgtgtcttgcctctcaatctgacaattacacctttataatagcaacataggaaaataactaaaactatggtttttaggcaaccaaataccagcaaaatgtaataattcctattattagatatgtttaagtgttctgctggtgggtcagcatctttggtagagtcataaaattaaaatgtacataattaattaaatattatatgtttattccctaacatttatttctgtcatttcttttttctttttttcagacagtctcactcttttgcccaggccggagtg

SEQ ID NO: 395 - DNA, 1001 bp, Homo sapiens
ttgtgtctcccaccccaaaaatgtgtatgttgaagtcctaaccttcagtactcagaatgtgacattatttggaaatagggtcattgcagatggagttagttaagatgaggtcattaggatgagtccctaatccaatatgactggtgctcttacaaaaaggggaagtttggacacagagccatgcacatgggtgggaagaatcccaaatgaacggataggcagagggttggagagatgcatcaacaaggaacaccaaagattgccagcaacccccagaagctgggggagaggcctggaacagattctccctcacagcctgagaggaaccaagctggctgacaccttgatctcaggttaccggccttgagaactgagagaccctgggtttctgttgtttaagcctctcagggtgcagcactttattatggaagcctgagctgactaatacaggtgtctctatatctcactgagggaaagtgacaggaaagtaagaaccatttrtgtccaagagtccagaggagtcaaccagattctgggggaaaagaaggtacaatgctggcctctccatgcagcctagtccccaacacttgtagggcccagggcaagatctaaagcactctctcacctatgcatctatatgctgtaactcagataaacaaactattaaataatatatgtgtcttgcctctcaatctgacaattacacctttataatagcaacataggaaaataactaaaactatggtttttaggcaaccaaataccagcaaaatgtaataattcctattattagatatgtttaagtgttctgctggtgggtcagcatctttggtagagtcataaaattaaaatgtacataattaattaaatattatatgtttattccctaacatttatttctgtcatttcttttttctttttttcagacagtctcactcttttgcccaggccggagtgcagtggcgtgatctcagctcactgcaacctccgcctcccaggtt

SEQ ID NO: 396 - DNA, 1218 bp, Homo sapiens
gataaagaaaggtcatcctcaatttcaatttactttatatattctttgagaggtaaccgtgtcttatctccccccaaaattccttttaaaaggaaatttccaaagatgctctattctgtgaataaagcattgtgccacagccgagaggatccagcaatgaacatgagattgcccttgattcataaggtctacaagctagtaaggatagagaacactttaaaataaaaaaaaatagtttttggtatatttatattgtgtatttggtataattgagttttctacattctcatatatgtatttcatattttgaagaatatgcagaaaataatcaagcttccaaataaacatttttttttaagaactgcacaagtgagaatttaggagaacagaagatcagagggctgcacrggctaaactagacaatgagcccatgcaagtaagttaagaggagaagcgggtaagtatgcacctgctttgtctaggtgaccagcaagcatttagcaatagtcttttcaaaacaacagctccttatattgtcaaatctcaagaagtaatatttatggttaaaaaaatctcagacccaacagaaaatccatgagggagatggttttggaaacgcagaattttcagctatgatatccttttataaacaagcagatactttccccaaatataattcaatgcctcagtctacctcctgctgaaaccactaacaccaccactaaagctcgactatatgggaaaatttaggtgtcactttcaaaatatgtcctagcataaaggcaattaaaaaatgtaaagcaccaaagatgcaagagagacataaatgaataaaatatctggcacgaaagttttcaaaagcttgggaatctgattcaaaaaaaaataaaatcagccaagcagtgttagtaagttagccaatcaggtttcaagaaggcagaaagacaaaatcaacatcaccagcatttgacaccgctactgggggaaaaaagggggatggagttcgtttatggcctttttaaaaatgccattacttggacaagagtcataacagagaagcactgcttatttcagttctgttaactgtaaatatcagagccaacacccagaaaaagttcaccattagccaattggttttgcctggccaattggagatggtaataggcctgctatggatgacattctttctgatataagttgtttcttgctttttctccc

SEQ ID NO: 397 - DNA, 1218 bp, Homo sapiens
gataaagaaaggtcatcctcaatttcaatttactttatatattctttgagaggtaaccgtgtcttatctccccccaaaattccttttaaaaggaaatttccaaagatgctctattctgtgaataaagcattgtgccacagccgagaggatccagcaatgaacatgagattgcccttgattcataaggtctacaagctagtaaggatagagaacactttaaaataaaaaaaaatagtttttggtatatttatattgtgtatttggtataattgagttttctacattctcatatatgtatttcatattttgaagaatatgcagaaaataatcaagcttccaaataaacatttttttttaagaactgcacaagtgagaatttaggagaacagaagatcagagggctgcacgggctaaactagacaatgagcccatgcaagtaagttaagaggagaagcgggtaagtatgcacctgctttgtctaggwgaccagcaagcatttagcaatagtcttttcaaaacaacagctccttatattgtcaaatctcaagaagtaatatttatggttaaaaaaatctcagacccaacagaaaatccatgagggagatggttttggaaacgcagaattttcagctatgatatccttttataaacaagcagatactttccccaaatataattcaatgcctcagtctacctcctgctgaaaccactaacaccaccactaaagctcgactatatgggaaaatttaggtgtcactttcaaaatatgtcctagcataaaggcaattaaaaaatgtaaagcaccaaagatgcaagagagacataaatgaataaaatatctggcacgaaagttttcaaaagcttgggaatctgattcaaaaaaaaataaaatcagccaagcagtgttagtaagttagccaatcaggtttcaagaaggcagaaagacaaaatcaacatcaccagcatttgacaccgctactgggggaaaaaagggggatggagttcgtttatggcctttttaaaaatgccattacttggacaagagtcataacagagaagcactgcttatttcagttctgttaactgtaaatatcagagccaacacccagaaaaagttcaccattagccaattggttttgcctggccaattggagatggtaataggcctgctatggatgacattctttctgatataagttgtttcttgctttttctccc

SEQ ID NO: 398 - DNA, 1072 bp, Homo sapiens
cacttaaaagctctggaaacctacgagattatctttaaaatcgtggggaccaaatggctggccaaggacttgtttctgtacaggtgcgattgcttctctgctgtgttcctttttattacccaagtaaccggtatttcagctcacaagatgagaaaatgacaaacaggcaaaataagcgtagggctgtgtgtgcaacagttwatcataaagccatcaccaggagacgtcactgggcgccttctggagtctatccgtcctaactttgctttctttctttttttttttaaatttaagttctagggtacatatgcacaacgtgcaggtttgtcacacatgtatacatgtgccatgttggtgtgctgcacccattaactcgtcatttacattaggtgtatctcctagtgctatccctccccactcccccgaccccatgacaggccccagtgtgtgatgttccccttcctgtgtccaagtgttctcattgttcaatccccacctatgagtgagaacatgccatgtttggttttttgtccttgcgatagtttgctgagaatgatggtttccagcttcatccatgtccctacaaaggacatgaactcatccttttttatggctacatagtattccatggtgtatatgtgccacattttcttaatccagtctatcatcgatggacatttgggttggttccaagtctttgctattgtgactagtgttgcaataaatatacgtgtggatgtgtctttatagcagtttgatttataatcctttgggtatatacccagtaacgggatggctgggtcaaatggtatttctagttctagatccttgaggaatcgccacactgacttccacaatggttgaactagttaacagtcccaccaacagtgtgaaagtgttcctatttctccacatcctctccagcaccccattttgactttgctataagggaactttagcatctgaacgtgcggacagcttcattgctggcttgttacgtaacagtgttttgtgaccatctcatgtcatacccacacatcgaaaccagcagtttaaatggccagctgtttgc

SEQ ID NO: 399 - DNA, 1072 bp, Homo sapiens
agattatctttaaaatcgtggggaccaaatggctggccaaggacttgtttctgtacaggtgcgattgcttctctgctgtgttcctttttattacccaagtaaccggtatttcagctcacaagatgagaaaatgacaaacaggcaaaataagcgtagggctgtgtgtgcaacagtttatcataaagccatcaccaggagacrtcactgggcgccttctggagtctatccgtcctaactttgctttctttctttttttttttaaatttaagttctagggtacatatgcacaacgtgcaggtttgtcacacatgtatacatgtgccatgttggtgtgctgcacccattaactcgtcatttacattaggtgtatctcctagtgctatccctccccactcccccgaccccatgacaggccccagtgtgtgatgttccccttcctgtgtccaagtgttctcattgttcaatccccacctatgagtgagaacatgccatgtttggttttttgtccttgcgatagtttgctgagaatgatggtttccagcttcatccatgtccctacaaaggacatgaactcatccttttttatggctacatagtattccatggtgtatatgtgccacattttcttaatccagtctatcatcgatggacatttgggttggttccaagtctttgctattgtgactagtgttgcaataaatatacgtgtggatgtgtctttatagcagtttgatttataatcctttgggtatatacccagtaacgggatggctgggtcaaatggtatttctagttctagatccttgaggaatcgccacactgacttccacaatggttgaactagttaacagtcccaccaacagtgtgaaagtgttcctatttctccacatcctctccagcaccccattttgactttgctataagggaactttagcatctgaacgtgcggacagcttcattgctggcttgttacgtaacagtgttttgtgaccatctcatgtcatacccacacatcgaaaccagcagtttaaatggccagctgtttgcttgtgaaaactcccctcggctggct

SEQ ID NO: 400 - DNA, 948 bp, Homo sapiens
aaattttctttgctgaagtgtcttttcaaatttttgccttttaaaaaaattgagttgtcttaatattgagtcgtaaggttctttatatattctggctatatgtcctttgtcagatatatgtcttgcaaatattttctcccagtctgtggcttaccttttccatttttaaactgtgttttataaaaaaaagaagtttttttagatcaaagtccattttaatcattttttcttttatagttcatgctttttgtgtctcatttaagaaatctttccctactccaatgtcacaaatatattctctgagaagcttaacagtttttgcaactaaatttaggtctatgatccgttttgacttaatttttccatatggtgtcatgtaacagttgagatttttttcctatgcaggcagatattcaatggttcaagtaccatttattgaaatggctatcttttctccactgaatgaccttggcacttttatcaaacatcaactggccacayacaggtgagtctacttctggacacttaccctgttccattcatctgtatatctctatccttacaccaacacgcatagtcttgaatactagggcaagttaattttaagatgtctcctggatatgtaaaaattatatctgagttgaactacagtttatttatatatccaggcagcaaataaatgtgagaatctggaggtgagggaagagatcagagataccaccttggaaaccatcaatttagagatgattcttaaggcaggggactaagggacactctgtaggacacagacatagagaagggaaggggctgcggcctgaacaccccacctgcatgctcactcacatactttcgtcggcctgtgttaacgaagtgctgggtctccccagcctctctcatctgtaagcagtgccaacaacgtccaacacagttccatccaatttggatctg

SEQ ID NO: 401 - DNA, 920 bp, Homo sapiens
aatttttgccttttaaaaaaattgagttgtcttaatattgagtcgtaaggttctttatatattctggctatatgtcctttgtcagatatatgtcttgcaaatattttctcccagtctgtggcttaccttttccatttttaaactgtgttttataaaaaaaagaagtttttttagatcaaagtccattttaatcattttttcttttatagttcatgctttttgtgtctcatttaagaaatctttccctactccaatgtcacaaatatattctctgagaagcttaacagtttttgcaactaaatttaggtctatgatccgttttgacttaatttttccatatggtgtcatgtaacagttgagatttttttcctatgcaggcagatattcaatggttcaagtaccatttattgaaatggctatcttttctccactgaatgaccttggcacttttatcaaacatcaactggccacacacaggtgagtctacttctggacacttaycctgttccattcatctgtatatctctatccttacaccaacacgcatagtcttgaatactagggcaagttaattttaagatgtctcctggatatgtaaaaattatatctgagttgaactacagtttatttatatatccaggcagcaaataaatgtgagaatctggaggtgagggaagagatcagagataccaccttggaaaccatcaatttagagatgattcttaaggcaggggactaagggacactctgtaggacacagacatagagaagggaaggggctgcggcctgaacaccccacctgcatgctcactcacatactttcgtcggcctgtgttaacgaagtgctgggtctccccagcctctctcatctgtaagcagtgccaacaacgtccaacacagttccatccaatttggatctg

SEQ ID NO: 402 - DNA, 701 bp, Homo sapiens
tgtgctgcttccattccataggcacctgatcctaagtgttaaccaatcccagaactctccccttatttcttgctgcatgttttgaattgatgtgataaacaatgtgattcgagcgtcttaactcagcctatgagcctctctattctgtgactgctggaataggctgcttggccatgttcttggaagctaccaccatatcarggtaatttcccacacaacattccagcccctgctttcccctctggccttatctagggccattccccaactcaggtgaatgcagactccaaatgtactgagctgtgtgcaggggccaggtgcaaatgctttctgtgcatctgcacatgctgttctacctgggaagtcctttcctcctttcacctatttttaccttaaacctcagacatcatctaccctggaaagtccttcctgacctcacgcatctaagtaggtcccccccataatccctatccatgccttctatagtacttaacatggtgacctttaattgttcatttacttagctctctgctctcccacactgtgaactccttacaaacagggaatgtcatctctgaatgaatctttcatctccatgtaacacatgcctccaaccctacctagcacacaatctggcatataacaggcactcaataaaccttcaatgaatgccttgatcaagtacaaggaacataagcaaa

SEQ ID NO: 403 - DNA, 701 bp, Homo sapiens
ttaaccaatcccagaactctccccttatttcttgctgcatgttttgaattgatgtgataaacaatgtgattcgagcgtcttaactcagcctatgagcctctctattctgtgactgctggaataggctgcttggccatgttcttggaagctaccaccatatcagggtaatttcccacacaacattccagcccctgctttccyctctggccttatctagggccattccccaactcaggtgaatgcagactccaaatgtactgagctgtgtgcaggggccaggtgcaaatgctttctgtgcatctgcacatgctgttctacctgggaagtcctttcctcctttcacctatttttaccttaaacctcagacatcatctaccctggaaagtccttcctgacctcacgcatctaagtaggtcccccccataatccctatccatgccttctatagtacttaacatggtgacctttaattgttcatttacttagctctctgctctcccacactgtgaactccttacaaacagggaatgtcatctctgaatgaatctttcatctccatgtaacacatgcctccaaccctacctagcacacaatctggcatataacaggcactcaataaaccttcaatgaatgccttgatcaagtacaaggaacataagcaaatttcctgtggaaaaaaagaattgtattaagttctttgg

SEQ ID NO: 404 - DNA, 601 bp, Homo sapiens
atgttcacttacacatctttctttcacttaattgaatcctttatttttgtcttagaatcttctgaatattgaaaacagagaactatactggaagaacatagtgtattaagactcatggagagggagatgtgatactgtgtcactgaggtcgttccagtcataggagaaatgttaccactggattgaggtctggtacattttaaaagatgatttaattctatgatatgtgttcaacttgcactaggatagtttttactttcacctttgttccatgcaccgcgcaaatacctgggaacccttrttgcccaactcaagagccagagtcctctgtcatcattttgcctctctcctaagtgacaggactgagtgcagacttggtgtttgtgggtgaggcatgtggactgacaggcaggcttcagtttatttagcgagtgtgagccctggcaggaagattctctttctctgcttgccaggttgaggaggcctcattaagcagtttgaacttgtggttttggcgtgtctagtcctggtgcaggtggcttggtatcctcacaggcatttctttggcctcacccttggggtgactgttcacttgtgtttg

SEQ ID NO: 405 - DNA, 601 bp, Homo sapiens
tcttctgaatattgaaaacagagaactatactggaagaacatagtgtattaagactcatggagagggagatgtgatactgtgtcactgaggtcgttccagtcataggagaaatgttaccactggattgaggtctggtacattttaaaagatgatttaattctatgatatgtgttcaacttgcactaggatagtttttactttcacctttgttccatgcaccgcgcaaatacctgggaacccttgttgcccaactcaagagccagagtcctctgtcatcattttgcctctctcctaagtgasaggactgagtgcagacttggtgtttgtgggtgaggcatgtggactgacaggcaggcttcagtttatttagcgagtgtgagccctggcaggaagattctctttctctgcttgccaggttgaggaggcctcattaagcagtttgaacttgtggttttggcgtgtctagtcctggtgcaggtggcttggtatcctcacaggcatttctttggcctcacccttggggtgactgttcacttgtgtttgagcggctgggactcagtaggttcactggagtaggtatttctttagagccactggcgg

SEQ ID NO: 406 - DNA, 701 bp, Homo sapiens
cagctccttggcaagcctgctccttccccagcaaatggaaacaccattctgaacacctgggcattgtctctgatgtcccttttcatctccctactctcacacaatccagctgcctctctgccttccacggatattaagaacgtccaccatctcctgagtccaagcccttctcactcacctctttcttgaactaatttcttyctgtttttttccagtcctcccttctgttcatgtctctcctctgcacacttccattttctggttcagaaaatgtcaccgtcccagtcacacttgccttatggctgttgtgtcataaatacagttgacacttgaacaacatgggtttgaactgcatggattcacttatacacatattttttcaatacaaatatatttaaaaattttggagatttgcaacaatttgaaaaaacttgcagatgaacagcatagcatagaaatattgaaaaattaagaaaaaggtatgtcatgaatgcataaaacatatgcagatactagtctattttaacctttactgccataaaatatacacaaatctattataaaaggttaaagtttatcaaagcttatgcacacaaacacttatagaccatatagggagccattcagtagagagaaatgtaagcgaacgtaaaggtgtgctatttaatcacaactgcatacacactgtaccactgcactaa

SEQ ID NO: 407 - DNA, 701 bp, Homo sapiens
gggcattgtctctgatgtcccttttcatctccctactctcacacaatccagctgcctctctgccttccacggatattaagaacgtccaccatctcctgagtccaagcccttctcactcacctctttcttgaactaatttctttctgtttttttccagtcctcccttctgttcatgtctctcctctgcacacttccattttstggttcagaaaatgtcaccgtcccagtcacacttgccttatggctgttgtgtcataaatacagttgacacttgaacaacatgggtttgaactgcatggattcacttatacacatattttttcaatacaaatatatttaaaaattttggagatttgcaacaatttgaaaaaacttgcagatgaacagcatagcatagaaatattgaaaaattaagaaaaaggtatgtcatgaatgcataaaacatatgcagatactagtctattttaacctttactgccataaaatatacacaaatctattataaaaggttaaagtttatcaaagcttatgcacacaaacacttatagaccatatagggagccattcagtagagagaaatgtaagcgaacgtaaaggtgtgctatttaatcacaactgcatacacactgtaccactgcactaatttcagagccacctcctgttgtgattgtggtgagcccaagtgttgtgaggatctgctt

SEQ ID NO: 408 - DNA, 501 bp, Homo sapiens
caggtagggtaagcaaatgaacacaaattcaaactcggaattcaaaaccagcctctgtgtattcctgaggaccatactgtctgctaagtgtagagaaaggcacatcctggttcaacagcagagaaagcaaacaggaggcactttctgtgagtcatctccaccacagggccctctcttttgtgatccagcgatacttgttcacagtcaaagcccaggaagagtggaaagattaacctttgtgagccaaaccrtgtgacacttgattacttgacagaactaatccttctgtcctgatgacagaaattcaactacacaggtacatgcaagctaatatctgttgtaatgcctcccagtttctctggagaattccttagtttcctggacatctctgaaatgcaaagttttggcaacgagtctctgaattaacctctgaaaatctcacccagccaagatggccttcttgagaagactgaagaacatggttggtttcaggctgagctg

SEQ ID NO: 409 - DNA, 604 bp, Homo sapiens
cactttctgtgagtcatctccaccacagggccctctcttttgtgatccagcgatacttgttcacagtcaaagcccaggaagagtggaaagattaacctttgtgagccaaaccgtgtgacacttgattacttgacagaactaatccttctgtcctgatgacagaamttcaactacacaggtacatgcaagctaatatctgttgtaatgcctcccagtttctctggagaattccttagtttcctggacatctctgaaatgcaaagttttggcaacgagtctctgaattaacctctgaaaatctcacccagccaagatggccttcttgagaagactgaagaacatggttggtttcaggctgagctggaagtggtttacctcccaggagaggttccccacagtggtgtttaaggcatggggtggaccaacaccaggaagactcagacatcacaccacccaccttcaactcagtcacatccacctacattttctgaaaacaaaaggcagtctccccaaaaagcactgagactcttgtgtaggtaatctgagcagacaccaacttcccagggcttccttttatccaggagagcttggctgttctttttaa

SEQ ID NO: 410 - DNA, 701 bp, Homo sapiens
ctccttccgccatggttgtaagtttcctgacgcctcccagtcatgcttcccgtacagcctgcagaactgcgagtcaatgaaatcccttttctccacaaattacccagtctcaggtagttccttacagcagcgtgggaacagactcaagagctgaagcaagcaaggccgttagcaaggagcgggctggggagagcactccaggcagagggaacagccagggccagggccttgagacagacgtgagccaggatatctgaggaacagcagagaagccagtgtggccgcagctaaatgaggaacaatgtgtgagttccctggggcggccaaaacaaacaccacggacgggggccttcaaccacagacaccgatttcctcacagctctggaggcgaaaagtccaagaaaactgcacggagtatctatgaggccctgatggagacctgacctggtccacacccatggcctggcaagctagatggggtgaattttcacctgccacagycgcaagtcaaagccaccggcttctctcttctccctcccattgctcctgacagccagggttaatattttgcctcatgtaaacagggaggcatccacccgagaatctcccctcagcccacataagctctgcagagagggctgtgttgctccagttcccacctggacatgagcactttgaagggcagcttccctcccggggtc

SEQ ID NO: 411 - DNA, 612 bp, Homo sapiens
gggctggggagagcactccaggcagagggaacagccagggccagggccttgagacagacgtgagccaggatatctgaggaacagcagagaagccagtgtggccgcagctaaatgaggaacaatgtgtgagttccctggggcggccaaaacaaacaccacggacgggggccttcaaccacagacaccgatttcctcacagctctggaggcgaaaagtccaagaaaactgcacggagtatctatgaggccctgatggagacctgacctggtccacacccatggcctggcaagctagatggggtgaattttcacctgccacagtcgcaagtcaaagccaccggcttctctcttctccctcccattgctcctgacagccagggttaatattttgcctcatgtaaacagggaggcayccacccgagaatctcccctcagcccacataagctctgcagagagggctgtgttgctccagttcccacctggacatgagcactttgaagggcagcttccctcccggggtctggctgagctcagggtaggcgtcagtctgcatggattggatggaggaaggctgtgcgtggcaggagatgacactgcccttgggctgtgtgg

SEQ ID NO: 412 - DNA, 1001 bp, Homo sapiens
ttggggaaggaagcactggggggaaggaagcactgggcttgggacagggctgggcgctgcctcttcactggaccatgacaaggttgttacctcaccaaggagaggtgcaaaaagcttaggggcttggatttctagatttcagtgccaactatgccacttactggctttatccttggggaatttatctactctgtgaccctcagtttttttatcttaattattaatacatacctcataatgtgactgtgaggattcacttaataatatatggaaaaccatagaatagtgcccagcatctaggaagtgccacagcccccttcagaagctagtgaaacctgcagaccacttttcagagtgatattattatttttttctaggtttactgagttataattgaaaaaataaaaatggaatatagatgtacaacatgaagctctgatgcatatatccattgtgaaatgatgaccacaatcaagctaattaatgttatctatcacttcwcatagttcaacctttttttgtggtgagagtactgaagatctactctcttagcaattttcaaatctaaaatacattattattaacacagtcactgtgccgtacgttagctctgaggaccttattcattttatacctaaaagtctgtatcctttaaccaacctctcctaatttcccactgtcatccctactgccacctctggtaaccagccttctgctctgtttctgagtccaaccttcttagattccacatatgagtgagatcatgctgtgcagtgtttgtttttctgtgtctggcttgctttcacttagcataatgtcctccaggtccacccatgttgttgcaaatggcagaatcttcttcttgttaaagactgaataatatccctgtgtgtgcgtgcatgtgtgtgtgtgtttgtgtgtgtgtgtgtatcacattttcttcatccattcatccatcaatggacactaagcactaaggttgattccgtatcttggctatt

SEQ ID NO: 413 - DNA, 2480 bp, Homo sapiens
aacattacttggggaaggaagcactggggggaaggaagcactgggcttgggacagggctgggcgctgcctcttcactggaccatgacaaggttgttacctcaccaaggagaggtgcaaaaagcttaggggcttggatttctagatttcagtgccaactatgccacttactggctttatccttggggaatttatctactctgtgaccctcagtttttttatcttaattattaatacatacctcataatgtgactgtgaggattcacttaataatatatggaaaaccatagaatagtgcccagcatctaggaagtgccacagcccccttcagaagctagtgaaacctgcagaccacttttcagagtgatattattatttttttctaggtttactgagttataattgaaaaaataaaaatggaatatagatgtacaacatgaagctctgatgcatatatccattgtgaaatgatgaccacaatcaagctaattaatgttatctatcacttcacatagttcaacctttttttgtggtgagagtactgaagatctactctcttagcaattttcaaatctaaaatacattattattaacacagtcactgtgccrtacgttagctctgaggaccttattcattttatacctaaaagtctgtatcctttaaccaacctctcctaatttcccactgtcatccctactgccacctctggtaaccagccttctgctctgtttctgagtccaaccttcttagattccacatatgagtgagatcatgctgtgcagtgtttgtttttctgtgtctggcttgctttcacttagcataatgtcctccaggtccacccatgttgttgcaaatggcagaatcttcttcttgttaaagactgaataatatccctgtgtgtgcgtgcatgtgtgtgtgtgtttgtgtgtgtgtgtgtatcacattttcttcatccattcatccatcaatggacactaagcactaaggttgattccgtatcttggctattgtgaataatgctgcaataaacatatgagtccagatacctcttcaagatactgatttcatttcctttaaatatatgcccagaagtgggattgctggatcatatggtagttctatatttagtatcttgaggaatttccatactgtttttcataatgattgtagcaatctatattcccatcaacagtgtacaagggttccattttctacatggccttaccaacgtttgttatcacttatctttttgataatagatattctagcaggtgtgaggtggtatctcattgtggttttaatttgcattttcctgatgattagtggtgtagagcatcttttcatattcccattggtaattcgtatatcttcctttgagaaatatttattcagatcttttgcccattgttagctgagttatatgtgagttggttttggtttgttgttgttttttgtttttgctattgagctgagttccttgtatattttggatattaaatccttctcagctgtatggttgacagatacattcttgcattctgtaagttgcatctgtaggttgcaacagagtctctttactctgttgattgcttgctttactgtgtgaaagcttttttagcttgatgtaattgtgtttgtctatttttgcttttgttgcttgtacttttagtgtcatatccaaaaagttattgcccagaccagtgtcatcccctatgttttcttctagtaattttaaagtttcaggtcttatgtctatgtctttaatccattttgagttaatttttgtgtagggtttaagataagaatccaattttatttttattttttgtatatggatatccaatttccccaacaccatttattgaaaattctatcctttctttgttgtgtattaacatcagaataatatttttaaatacataaaattcagaagatgacaaaggaaaccaattacattgaaatgcatacagagttataattctgaaagagcaatatatgtgcctctttgtaaacacatcatatatcaaactgcagtgaccgttctaacaactattgcaatttcaaagtcatgttgagtaggaggagtactttgagattctgaaacaacgttcttgtgctatgaaatatccatgattttgattggtgatggtatcccaggtcttgttaatgctgctgtaatctgttgcttccattccatagttgaataaaatgcttgatatctgttggaaattagtaaaaataaaaacgtatttttttccatccaagttcattctcagaccctgaagagtcacttctctggattctgcagcaaagttcccagctggggcagcaagatttaggcaattgaaaagaacatacaccttgttctcagtggcaaaccacatggaaagctttaaatgtcagagaagaattctgccattttgctgacttttttgtagttctcctaataaacaagtgttaagtgacaagcttttcagagg

SEQ ID NO: 414 - DNA, 601 bp, Homo sapiens
ccccccccccccccgcagatctcaggtgggcatttttgaacttaactagataacaaaacacagctaagacaagtccttttctccagcaaagatggcaatgctctaataactctgagcatattaaagattctccaagactctagcctctgctgcaaaaacacatacaaatacctactactactgctgctgtgatgatgatgatgacagcaatagtgagaatattttaaatatgccaggcacggtggcaactgctttccaaatattatcatatttaatctgatcattgccctatgaggtaggragtattctgattcccattttataaataaggaacccgaggcttagagagcatcggtgacttgttcaaggtcacccacagctgtcaagtgacagaacttcgataaaaatccagactcctttaatggagtatggagggaggtcagaaaacataggaagtaagggattgtgattgacaatgtgtccttgcaaagggacaggttaagagacacaagggcagctgtctgaggtgtgccattcaccagcttcaggagagaagtggcaggctacctccagctatccagccctatccagccaaggaagc

SEQ ID NO: 415 - DNA, 601 bp, Homo sapiens
caaaacacagctaagacaagtccttttctccagcaaagatggcaatgctctaataactctgagcatattaaagattctccaagactctagcctctgctgcaaaaacacatacaaatacctactactactgctgctgtgatgatgatgatgacagcaatagtgagaatattttaaatatgccaggcacggtggcaactgctttccaaatattatcatatttaatctgatcattgccctatgaggtagggagtattctgattcccattttataaataaggaacccgaggcttagagagcatcrgtgacttgttcaaggtcacccacagctgtcaagtgacagaacttcgataaaaatccagactcctttaatggagtatggagggaggtcagaaaacataggaagtaagggattgtgattgacaatgtgtccttgcaaagggacaggttaagagacacaagggcagctgtctgaggtgtgccattcaccagcttcaggagagaagtggcaggctacctccagctatccagccctatccagccaaggaagcttgggagacatgttagttcccgccttcatttccatcagcaacctcaaagccac

SEQ ID NO: 416 - DNA, 5823 bp, Homo sapiens
tatttcaggctttcttctttctatggataagaaagctcctcaggtggcaacaaaggccatttctttggaagcaggcatggcatgtgacgaaaaaaagacatctcagaaaagagccaagaataagactggagagccactgtcagagaacagaaactgggcttaatcaaggaacatctcttgttcccagagtaggaggctggcaatattttctcactgaaatttcagaattgttatggaccagtgactgctctatgtgttcaatttgttcccttttcaaatggaagcatttattgcagacgacctgcctctgtcccaccattgtgtattaggtttgtagagygtagacaacttgcctttttagtttgtaggtttctgtatcaagagaagatgtgtgtgggcctaacctagattacaggatcctggacttcaagtctgatataatgactggatgagactttgactgtcctagaattgggatgaacatattttgccggtgggagggcgtgagtaattgcggttagagggcagactgtccctcacacctattccttttcatggtgccttcccaaactgcctctggaggtggccacacaaatggctttggccattgtgaccatgggaaacttgatgcagaggctggaaaaagcacttgcatgtttctgtctcctctcttgttcctctacaatcacaagaaatgtctaggcaggtctgagcaggcccaggctcatctgccatggaagaagaatggcacatggaagagggtcacattgtcccaaccaagacgatcctagaccagccaggccccagttcatggttcaagacacatgaacatagttgcacgaaccaagattagttgtgtatggcccagactagcagcagcacccatccaacctacagactctgagaaataaatactagttgtcttaagcttccaagtttcagtgtgagcattaggtagtaacagttaatgaataagacagataatcattttatctgtctggatacttatacaatgatttctattttttattgatacataatattttacatattgctggggtacatgtgacattttgctacatacatagaatgtgtaatgatccagtcaggatatctgaggtgtccatcactttgagaatttctcacttctgtgtgttgggaacaattcaagtcgtctcttctagttattttaaaatatacaatacattgttaactgtagtcttttttattgaatgacaggacttgtaccttttatctaactgtatgtttgtatctattaagctagttctctttatccctgccccctcctacccactcactcttcccaacctctaacatgtatcatcctattctatatctccatgagatcaacttctttagctcccacatatgagcaaaaacatatgatgtttgtctttctgtgcccggtttatttcacttatgacctccatttccatccatgttactataaatgacaggatttcattctttttgtggccaaacagtatttcattgtgtatatatactacattttctttatccattcatccattgatgaacacttacgttgattccatatctttgctattgtgaatggtgctgcaataaacatgcacgtgcagttatccctttgatacactgatttattttcctttggataaatacccagtagtgagattgctggatcatacggtagttctacttttagtttttgagacatttccatacttttccagtgtttgtattaatttacattcccatcaacaatgtataagatttccctttcctccacatcctcaccagcatctgctattttttgtctttttaataatagtcattctaactggggtgagaggatatctcgctatggttttgatttgcatttccctgatatttaatgatattgagcatttcttcatataacctattggccatttgtgtgtcttttttttttttttttttttttttgagaattgtctactcatttttggctttttaaaagatttattttttgttgttgttgagtttagtgcatatcctggatattagtctcttatctgatgaagagtttgccaatattttctcccattcaacaggttgtctcttcattctgttgactgtttcctttgctgtgcagaagcactttatatacagtcccatttgtctattttttagtagtctatgcatttaaggtctcagccacaaaatctttgcctagaccagtcctaaagtgtttcccctatattttcttctagtagttttattgtttcatgtcttatatttaagtctataatccattgtgagttgatttttgtatatggtgagataggggccttgtttcattcctctgcatatagatatttaattttctcagcaccatttattgaaggtgtccttccctattgtatgttcttggtgcctttgtcaaaattcagttggctataaatatgtgaatttatttctgggttctctatgtggttccattagtctatgtgtctatttttataccaatatcatgctgttttgattaccatagccttgtaatatattttgaagtcaggtagtgtgatgcctccagctttgttctttttgctcaggattgctgtgcatactctggctttttggttacatacaaatttcaggatttttgtatttctgtgaaaaatggcattagtattttgataggaattgcactggatctgtatattgtcctggacaacatggtcattttaacaatattaattcttctaatctatgagtatgagacgtcttcccacttgtttgtgtcctcttcaatttctttcattggtgtttcataatctcccttctacaggcctttcacctccttggttaaattaattcctaggtatttttttgtagctactgtaaatgggactgccttctttctcagctagttcatttttggtgcatagaaaccctatttttgtatgttcattttctatcctgcaacattaccaaatttgcttatcagctttaagtgtgtattttgctttgcttgtagagtcttctggtttctctaaatgtaagacgatgtcatctgcaaacggggacaatttgacttcctcttaaaaatctgtatgccttttattcctttctcttgcctgattgctctggctctacctccagtactatactgaataaaagtggtaaaagtgagcatccttccttgtcttgctctagttcttagaggaaatactttcagtttttccccactcagtatgatgttagctgtgggtcatatatagcctttattatgttaagatatgtttcttctgtacctggtttgttgacagctttttatcataaaaggatgtagaattttatcaaatgttttttctgcatctgttgagataatcatatggtttttgtcattccttctactgttgtgatgtatcatgtttattgatttgtgtatgttaaaccatccttgtgtccttggtataaattatacttggtcatggtgtattatctttttggcatcctgtcgaattgtttgctagctttttgttttgttctttttgagaatttttatgtctaggttccttagaaacactggcctgtagttctctttttgtgtgtgtgtccttgtctagtttggtgtcagggaaatggtggtcttgtagaatgagttgttttttctttgatttttttgcaagagtttgaggagaatgggtattagttcttctttatgtggttggtcaaattggcagtgaattcattcagtcatgagcttttctttttttgggagggttctcattactgagttaatcacactgctcattactgatctgttcagattttctatttcttctggaatctcagtagttgtatgtttccagcaatttatccatttcctctaggttttctagtttggtagtatatagctattcataatagtctctgatgatcttttgtatttctgtgatatcagttgtaatgtctttttcatttcctattttatttgggtcttttcttgtttagtctagcaaggggtttatctattttatctttttgaagaaccaactttttgtttcattgaccctttctacgtctttagtctttatttcatttagatttgctctgaactttactatgtctttccttctaattttgggtttggtttgttcttttctagttccttgaggtgcatcattgaattgtttctttgatatctatctactcatttgatgtaggtgtttattgctatacactctcccctcctagagctccttttgttgtgtcccataggtcttggtatgttgtttctattttcatttgtttcaaacattttatttccatattaatttttatcattcaggaggagcatattatttaattcccatgtatttgtatagtttccaaagttcctcttatttctatttttactccattgtggtctgagaagatacttcatatgatttcaatttttaaaaatttgtcaagacttgttttttgtcctaacatatggtctatcctggagaatgttccatgtgctgatgagaaaaatgtgtactcagcagttgttgagtaacatgttctacaaatatctgttagatccatttggtctaaagtctagtttaaatccaatgagtttttgttaattttgtctagatgatcatgatctgagactgaggtgaagtccccaacaattatcgtgttggagtctacctctctttttaaatctagaaatatttgctttataaatccgggtggtctagtgttgggtgcatatatttagttgttatttcctcattagattgatctctttactattatataataactgtttactgcttctggcataaagtctgttttatgtaagtacagccattcctgcttgagtttagtaccatgttgacaaagggatgcatagagagttggtaaagcatgatttctgggtgtctgtgtgaaggtgttttgagaagagtttagcatgagtctgtggagtgagtgggaagattctccctcaatgtcagcaggaaccatccatccactgggggcccaggtagaaaaagatgaagaaatggtgaattctctctctctcctggagctgggtcacccttcttctgcccttgaacaggacatcacaactccaggctctccagcctttggactccaagactgacaccagtgcccctccccaattaccccaggccctcaggcctttggcctaggattgagacttacaccatcagcttccctggttctgaggcttctggacttgcactgggccatactaccagcatcccagggtctccagcttgcagagagcctgttgtgggacttttcagcctccataatcaagtaagccaatttccctggtatctatatagatatacaatcatgttttgcttaccagcctgaaaaatgtatcgctagatgagtctgtcattgcataaacatcatagtgtacttacacaaacctagattctatagcctactacacacctagtctataaacatgtacagcatgttactgtactgaatattgtaggcaactgtaacacaatggtgaatatttgcatatttaaacatatcttatcattaaaaagatacagtaaacataaggtataaaagacaaaaaccggcacacctatatagggcacttaccataaatgcagcttgcaggactagaagtcactcagggtgagtcagtgagcgaacgtgaaggcctaggttattactgtccactacggtagactttatcaacactgtacacaggctacactaaatttattttttaaaaatttgctctccaataataaattaatcttcgcatcctttttttgttgttcactgtgg

SEQ ID NO: 417 - DNA, 5823 bp, Homo sapiens
tatttcaggctttcttctttctatggataagaaagctcctcaggtggcaacaaaggccatttctttggaagcaggcatggcatgtgacgaaaaaaagacatctcagaaaagagccaagaataagactggagagccactgtcagagaacagaaactgggcttaatcaaggaacatctcttgttcccagagtaggaggctggcaatattttctcactgaaatttcagaattgttatggaccagtgactgctctatgtgttcaatttgttcccttttcaaatggaagcatttattgcagacgacctgcctctgtcccaccattgtgtattaggtttgtagagtgtagacaacttgcctttttagtttgtaggtttctgtatcaagagaagatgtgtgtrggcctaacctagattacaggatcctggacttcaagtctgatataatgactggatgagactttgactgtcctagaattgggatgaacatattttgccggtgggagggcgtgagtaattgcggttagagggcagactgtccctcacacctattccttttcatggtgccttcccaaactgcctctggaggtggccacacaaatggctttggccattgtgaccatgggaaacttgatgcagaggctggaaaaagcacttgcatgtttctgtctcctctcttgttcctctacaatcacaagaaatgtctaggcaggtctgagcaggcccaggctcatctgccatggaagaagaatggcacatggaagagggtcacattgtcccaaccaagacgatcctagaccagccaggccccagttcatggttcaagacacatgaacatagttgcacgaaccaagattagttgtgtatggcccagactagcagcagcacccatccaacctacagactctgagaaataaatactagttgtcttaagcttccaagtttcagtgtgagcattaggtagtaacagttaatgaataagacagataatcattttatctgtctggatacttatacaatgatttctattttttattgatacataatattttacatattgctggggtacatgtgacattttgctacatacatagaatgtgtaatgatccagtcaggatatctgaggtgtccatcactttgagaatttctcacttctgtgtgttgggaacaattcaagtcgtctcttctagttattttaaaatatacaatacattgttaactgtagtcttttttattgaatgacaggacttgtaccttttatctaactgtatgtttgtatctattaagctagttctctttatccctgccccctcctacccactcactcttcccaacctctaacatgtatcatcctattctatatctccatgagatcaacttctttagctcccacatatgagcaaaaacatatgatgtttgtctttctgtgcccggtttatttcacttatgacctccatttccatccatgttactataaatgacaggatttcattctttttgtggccaaacagtatttcattgtgtatatatactacattttctttatccattcatccattgatgaacacttacgttgattccatatctttgctattgtgaatggtgctgcaataaacatgcacgtgcagttatccctttgatacactgatttattttcctttggataaatacccagtagtgagattgctggatcatacggtagttctacttttagtttttgagacatttccatacttttccagtgtttgtattaatttacattcccatcaacaatgtataagatttccctttcctccacatcctcaccagcatctgctattttttgtctttttaataatagtcattctaactggggtgagaggatatctcgctatggttttgatttgcatttccctgatatttaatgatattgagcatttcttcatataacctattggccatttgtgtgtcttttttttttttttttttttttttgagaattgtctactcatttttggctttttaaaagatttattttttgttgttgttgagtttagtgcatatcctggatattagtctcttatctgatgaagagtttgccaatattttctcccattcaacaggttgtctcttcattctgttgactgtttcctttgctgtgcagaagcactttatatacagtcccatttgtctattttttagtagtctatgcatttaaggtctcagccacaaaatctttgcctagaccagtcctaaagtgtttcccctatattttcttctagtagttttattgtttcatgtcttatatttaagtctataatccattgtgagttgatttttgtatatggtgagataggggccttgtttcattcctctgcatatagatatttaattttctcagcaccatttattgaaggtgtccttccctattgtatgttcttggtgcctttgtcaaaattcagttggctataaatatgtgaatttatttctgggttctctatgtggttccattagtctatgtgtctatttttataccaatatcatgctgttttgattaccatagccttgtaatatattttgaagtcaggtagtgtgatgcctccagctttgttctttttgctcaggattgctgtgcatactctggctttttggttacatacaaatttcaggatttttgtatttctgtgaaaaatggcattagtattttgataggaattgcactggatctgtatattgtcctggacaacatggtcattttaacaatattaattcttctaatctatgagtatgagacgtcttcccacttgtttgtgtcctcttcaatttctttcattggtgtttcataatctcccttctacaggcctttcacctccttggttaaattaattcctaggtatttttttgtagctactgtaaatgggactgccttctttctcagctagttcatttttggtgcatagaaaccctatttttgtatgttcattttctatcctgcaacattaccaaatttgcttatcagctttaagtgtgtattttgctttgcttgtagagtcttctggtttctctaaatgtaagacgatgtcatctgcaaacggggacaatttgacttcctcttaaaaatctgtatgccttttattcctttctcttgcctgattgctctggctctacctccagtactatactgaataaaagtggtaaaagtgagcatccttccttgtcttgctctagttcttagaggaaatactttcagtttttccccactcagtatgatgttagctgtgggtcatatatagcctttattatgttaagatatgtttcttctgtacctggtttgttgacagctttttatcataaaaggatgtagaattttatcaaatgttttttctgcatctgttgagataatcatatggtttttgtcattccttctactgttgtgatgtatcatgtttattgatttgtgtatgttaaaccatccttgtgtccttggtataaattatacttggtcatggtgtattatctttttggcatcctgtcgaattgtttgctagctttttgttttgttctttttgagaatttttatgtctaggttccttagaaacactggcctgtagttctctttttgtgtgtgtgtccttgtctagtttggtgtcagggaaatggtggtcttgtagaatgagttgttttttctttgatttttttgcaagagtttgaggagaatgggtattagttcttctttatgtggttggtcaaattggcagtgaattcattcagtcatgagcttttctttttttgggagggttctcattactgagttaatcacactgctcattactgatctgttcagattttctatttcttctggaatctcagtagttgtatgtttccagcaatttatccatttcctctaggttttctagtttggtagtatatagctattcataatagtctctgatgatcttttgtatttctgtgatatcagttgtaatgtctttttcatttcctattttatttgggtcttttcttgtttagtctagcaaggggtttatctattttatctttttgaagaaccaactttttgtttcattgaccctttctacgtctttagtctttatttcatttagatttgctctgaactttactatgtctttccttctaattttgggtttggtttgttcttttctagttccttgaggtgcatcattgaattgtttctttgatatctatctactcatttgatgtaggtgtttattgctatacactctcccctcctagagctccttttgttgtgtcccataggtcttggtatgttgtttctattttcatttgtttcaaacattttatttccatattaatttttatcattcaggaggagcatattatttaattcccatgtatttgtatagtttccaaagttcctcttatttctatttttactccattgtggtctgagaagatacttcatatgatttcaatttttaaaaatttgtcaagacttgttttttgtcctaacatatggtctatcctggagaatgttccatgtgctgatgagaaaaatgtgtactcagcagttgttgagtaacatgttctacaaatatctgttagatccatttggtctaaagtctagtttaaatccaatgagtttttgttaattttgtctagatgatcatgatctgagactgaggtgaagtccccaacaattatcgtgttggagtctacctctctttttaaatctagaaatatttgctttataaatccgggtggtctagtgttgggtgcatatatttagttgttatttcctcattagattgatctctttactattatataataactgtttactgcttctggcataaagtctgttttatgtaagtacagccattcctgcttgagtttagtaccatgttgacaaagggatgcatagagagttggtaaagcatgatttctgggtgtctgtgtgaaggtgttttgagaagagtttagcatgagtctgtggagtgagtgggaagattctccctcaatgtcagcaggaaccatccatccactgggggcccaggtagaaaaagatgaagaaatggtgaattctctctctctcctggagctgggtcacccttcttctgcccttgaacaggacatcacaactccaggctctccagcctttggactccaagactgacaccagtgcccctccccaattaccccaggccctcaggcctttggcctaggattgagacttacaccatcagcttccctggttctgaggcttctggacttgcactgggccatactaccagcatcccagggtctccagcttgcagagagcctgttgtgggacttttcagcctccataatcaagtaagccaatttccctggtatctatatagatatacaatcatgttttgcttaccagcctgaaaaatgtatcgctagatgagtctgtcattgcataaacatcatagtgtacttacacaaacctagattctatagcctactacacacctagtctataaacatgtacagcatgttactgtactgaatattgtaggcaactgtaacacaatggtgaatatttgcatatttaaacatatcttatcattaaaaagatacagtaaacataaggtataaaagacaaaaaccggcacacctatatagggcacttaccataaatgcagcttgcaggactagaagtcactcagggtgagtcagtgagcgaacgtgaaggcctaggttattactgtccactacggtagactttatcaacactgtacacaggctacactaaatttattttttaaaaatttgctctccaataataaattaatcttcgcatcctttttttgttgttcactgtgg

SEQ ID NO: 418 - DNA, 707 bp, Homo sapiens
aacggtgtcagctggagtgaactcctgtgtgtgcaaggcctgggtctcctggtcagactactttctatgggaaaggcatagtgtatagtctatatactatacataggggtgctgggaggaactggggttttcacagccagctttggttttcattaggtttgtttagtttccattgcttcaggggtgttagttttgtgttcmcaactagattataaactcctcttgcattcctgatggcagtgacttgaaggcatttatttgaagaataatagacatacagaaaggggcgcatgtcataaaggtacagctggacgacttttcacaaagtgagcacatttgtatgatcgatgttgagaccaagagcattcagtggacaactcctttccagttactccaccccactcccagtgaccatcattctgacttctaactgtgtagacatgttttgcttgttttgtactttacaaacatatctactctattttaggtggctagacaatgtgttttacaatgctggccatgacagtgtttgaaagaataaaatggaatcaaatagaatgggcagtatcagagtgtgttgcctgcctaagaaatgttttgtgacattttggctttgggtctatttacacattaaatctaagagcaccagaatgtggtgtcaaaatgtgtttggggatgaagatattctaaagtcctgtagtaagcaa

SEQ ID NO: 419 - DNA, 712 bp, Homo sapiens
cagactactttctatgggaaaggcatagtgtatagtctatatactatacataggggtgctgggaggaactggggttttcacagccagctttggttttcattaggtttgtttagtttccattgcttcaggggtgttagttttgtgttcccaactagattataaactcctcttgcattcctgatggcagtgacttgaaggcatttatttgaagaataatagacatacagaaaggggcrcatgtcataaaggtacagctggacgacttttcacaaagtgagcacatttgtatgatcgatgttgagaccaagagcattcagtggacaactcctttccagttactccaccccactcccagtgaccatcattctgacttctaactgtgtagacatgttttgcttgttttgtactttacaaacatatctactctattttaggtggctagacaatgtgttttacaatgctggccatgacagtgtttgaaagaataaaatggaatcaaatagaatgggcagtatcagagtgtgttgcctgcctaagaaatgttttgtgacattttggctttgggtctatttacacattaaatctaagagcaccagaatgtggtgtcaaaatgtgtttggggatgaagatattctaaagtcctgtagtaagcaatgcaaaacgttctggaggtgtttattaaacatttgtttgtagaatggagaggaagaca

SEQ ID NO: 420 - DNA, 1210 bp, Homo sapiens
aaagcagcactgctctgcattcagccttgctacgtctccttcagatgggcgcactagatactgagtgatgatcatgccttgtctaggatctcaccaagacagttcatgaaagagacagtgcagctcatggaggagatggtgcagctcacagagaggatggtgccatcatggaaagcatggggcagtcatggagatgacggrgtagctcatggagaatataatgccatcatggaaggcatagtgcagtcatggagatgatggtgcagctcatggagaagatggtgccatcatggaaggcatggtgcaatcatggagtagacagtgcagctgggccaagattctccctgactaagctcttctcaggcacctctgagccgtcgtcttaactaggcctccagcttggcttgtgaaaactgcagactctcagcacaaatgatttgcctcctacattaagagacttaaataaacacttgcatggctgtgtttatttaaacagctcaaggctgtgtccctgggatgacaatgactccagcccctaaaattcctgcttgtgaaagctcattgctgacagaaggatctaccatttgttccagccaacacctggtggcaggcagataggccctgagccccatttaagagcagttcctttagaaagcttgcaattgtaaatcttttctctgcccatttgagatgtaaatcttctaccacctagaactgtcttctcaaggacctgtgagctgactcactgaaatgcaaacattcagggagataactccactcctgtccccatgcgacggcgaggccctgactttggtgggcaccttgctcttatttgcaccaccacctcctgtcctaaagacatgagacgtttgtctctcctctggataagtgcctattaaccaacccaggtgtcctggtcacatgaaccagtccagcctagcacctggcactgcctttccctcagcacactccagtctgtaaaagtctccttatggttgttttggcaaagttgagcttagttaatgctagaccccttctctactgcaatagttactgctgaataaagtctatccttaccactttaactagtgttgggctttgtttctctttcataagctcatggagaagacaatgcagttccatcaagtttctggctcttacactgctaacagtcagctctggggtccctgagagggacagactcacacca

SEQ ID NO: 421 - DNA, 1194 bp, Homo sapiens
gcattcagccttgctacgtctccttcagatgggcgcactagatactgagtgatgatcatgccttgtctaggatctcaccaagacagttcatgaaagagacagtgcagctcatggaggagatggtgcagctcacagagaggatggtgccatcatggaaagcatggggcagtcatggagatgacggagtagctcatggagaakataatgccatcatggaaggcatagtgcagtcatggagatgatggtgcagctcatggagaagatggtgccatcatggaaggcatggtgcaatcatggagtagacagtgcagctgggccaagattctccctgactaagctcttctcaggcacctctgagccgtcgtcttaactaggcctccagcttggcttgtgaaaactgcagactctcagcacaaatgatttgcctcctacattaagagacttaaataaacacttgcatggctgtgtttatttaaacagctcaaggctgtgtccctgggatgacaatgactccagcccctaaaattcctgcttgtgaaagctcattgctgacagaaggatctaccatttgttccagccaacacctggtggcaggcagataggccctgagccccatttaagagcagttcctttagaaagcttgcaattgtaaatcttttctctgcccatttgagatgtaaatcttctaccacctagaactgtcttctcaaggacctgtgagctgactcactgaaatgcaaacattcagggagataactccactcctgtccccatgcgacggcgaggccctgactttggtgggcaccttgctcttatttgcaccaccacctcctgtcctaaagacatgagacgtttgtctctcctctggataagtgcctattaaccaacccaggtgtcctggtcacatgaaccagtccagcctagcacctggcactgcctttccctcagcacactccagtctgtaaaagtctccttatggttgttttggcaaagttgagcttagttaatgctagaccccttctctactgcaatagttactgctgaataaagtctatccttaccactttaactagtgttgggctttgtttctctttcataagctcatggagaagacaatgcagttccatcaagtttctggctcttacactgctaacagtcagctctggggtccctgagagggacagactcacacca

SEQ ID NO: 422 - DNA, 1194 bp, Homo sapiens; identical to SEQ ID NO: 421

SEQ ID NO: 423 - DNA, 1118 bp, Homo sapiens
accaagacagttcatgaaagagacagtgcagctcatggaggagatggtgcagctcacagagaggatggtgccatcatggaaagcatggggcagtcatggagatgacggagtagctcatggagaagataatgccatcatggaaggcatagtgcagtcatggagatgatggtgcagctcatggagaagatggtgccatcatgraaggcatggtgcaatcatggagtagacagtgcagctgggccaagattctccctgactaagctcttctcaggcacctctgagccgtcgtcttaactaggcctccagcttggcttgtgaaaactgcagactctcagcacaaatgatttgcctcctacattaagagacttaaataaacacttgcatggctgtgtttatttaaacagctcaaggctgtgtccctgggatgacaatgactccagcccctaaaattcctgcttgtgaaagctcattgctgacagaaggatctaccatttgttccagccaacacctggtggcaggcagataggccctgagccccatttaagagcagttcctttagaaagcttgcaattgtaaatcttttctctgcccatttgagatgtaaatcttctaccacctagaactgtcttctcaaggacctgtgagctgactcactgaaatgcaaacattcagggagataactccactcctgtccccatgcgacggcgaggccctgactttggtgggcaccttgctcttatttgcaccaccacctcctgtcctaaagacatgagacgtttgtctctcctctggataagtgcctattaaccaacccaggtgtcctggtcacatgaaccagtccagcctagcacctggcactgcctttccctcagcacactccagtctgtaaaagtctccttatggttgttttggcaaagttgagcttagttaatgctagaccccttctctactgcaatagttactgctgaataaagtctatccttaccactttaactagtgttgggctttgtttctctttcataagctcatggagaagacaatgcagttccatcaagtttctggctcttacactgctaacagtcagctctggggtccctgagagggacagactcacacca

SEQ ID NO: 424 - DNA, 601 bp, Homo sapiens
gtaggggcactgtctatactggctgcactctggccagtgctgtcccaacgctgacccctctggaagctaatctggcttataatgaggatgctttctttagaggggactctccatgcacagcagaaaatcccaatggagtggttcttccctatgtccccaagggactgggaatattctttcagtaacaatggcccattgggggaagaaggatgaaagtggggtgagagacgtgaaatttggagaggtccctcaaagattgtgatgtgcctctcttgttccaatcacaggacaggggtataayggctttcctttgaaacacggggatgaatttaactattcacttcccaggtagattcatcagggtctagagcttcagctaacagcatgaggaagattccaaatgtgcccccatcagcataggaactgggtatgttgagtctatggtctcataaaaccagaagaaggacaagggattgtggctccaggcttgggagcaccttttccttaccatgggctacagtatttatttagggtaaaggaaggaaactcctgaggtgctatggggtgccagcaatttggagcatcagtaattcaatgtccc

SEQ ID NO: 425 - DNA, 601 bp, Homo sapiens
acgctgacccctctggaagctaatctggcttataatgaggatgctttctttagaggggactctccatgcacagcagaaaatcccaatggagtggttcttccctatgtccccaagggactgggaatattctttcagtaacaatggcccattgggggaagaaggatgaaagtggggtgagagacgtgaaatttggagaggtccctcaaagattgtgatgtgcctctcttgttccaatcacaggacaggggtataacggctttcctttgaaacacggggatgaatttaactattcacttcccargtagattcatcagggtctagagcttcagctaacagcatgaggaagattccaaatgtgcccccatcagcataggaactgggtatgttgagtctatggtctcataaaaccagaagaaggacaagggattgtggctccaggcttgggagcaccttttccttaccatgggctacagtatttatttagggtaaaggaaggaaactcctgaggtgctatggggtgccagcaatttggagcatcagtaattcaatgtcccttcagccatgtgtattcaactcctgctgtgggtgtggacttggtgca

SEQ ID NO: 426 - DNA, 701 bp, Homo sapiens
ttcctgggcatcgtcatattctgtaaaacaaggaagctcagcccagtgtgttctaacatgacctcctttctacatccttaggtgttgttatgcgtgaatcacgtccccccaaaagacatgttcatgtcctaacccccaggacctcagaatgtgtgatctggtttggaaataaggtcatcacagatgaaattagctaagacaaggtcatattggaatagggttggcccttaatccactgtgactggtgtccttttaagaagaggacacagacacaggaggggagagggccatgggatgatgcaggtggagactggagtgctacagctgcaagcaaatacatttctgtgctgtgaagccacccatttggtggtactacgttaaaacagctctaggaaattaatacagatgttgcctgtatttttgtttctcatattactactcattgttttaatgatgactgttttattcattaagttgaaagctcctaaagcagagggaccrtatttttatgtcccaactctccttaaggccttgcctatgatagcacatctcttcaatagaattgtcctaactttaacagagacaacttgggttatttaatatggagaacaaagggttaagctggtgccagatgggtttcattttctctaaatctggaaccaaaggcagcaagtctatggggtggacggagttcttagctc

SEQ ID NO: 427 - DNA, 701 bp, Homo sapiens
caaggaagctcagcccagtgtgttctaacatgacctcctttctacatccttaggtgttgttatgcgtgaatcacgtccccccaaaagacatgttcatgtcctaacccccaggacctcagaatgtgtgatctggtttggaaataaggtcatcacagatgaaattagctaagacaaggtcatattggaatagggttggcccttaatccactgtgactggtgtccttttaagaagaggacacagacacaggaggggagagggccatgggatgatgcaggtggagactggagtgctacagctgcaagcaaatacatttctgtgctgtgaagccacccatttggtggtactacgttaaaacagctctaggaaattaatacagatgttgcctgtatttttgtttctcatattactactcattgttttaatgatgactgttttattcattaagttgaaagctcctaaagcagagggaccatatttttatgtcccaactctccttaagsccttgcctatgatagcacatctcttcaatagaattgtcctaactttaacagagacaacttgggttatttaatatggagaacaaagggttaagctggtgccagatgggtttcattttctctaaatctggaaccaaaggcagcaagtctatggggtggacggagttcttagctcaaccctttggtgaggtaagaagaaggat